European Patent Application EP 4 674 971 A1, published January 7, 2026. Title: Novel methods for acyl group transfer and polyketide synthesis. Applicant: kez.biosolutions GmbH. Application EP. The sequence listing filed with the application follows.

SEQUENCE LISTING (165 sequences)

SEQ ID NO: 1 - protein, 2504 aa, Mus musculus
MEEVVIAGMSGKLPESENLQEFWANLIGGVDMVTDDDRRWKAGLYGLPKRSGKLKDLSKFDASFFGVHPKQAHTMDPQLRLLLEVSYEAIVDGGINPASLRGTNTGVWVGVSGSEASEALSRDPETLLGYSMVGCQRAMMANRLSFFFDFKGPSIALDTACSSSLLALQNAYQAIRSGECPAALVGGINLLLKPNTSVQFMKLGMLSPDGTCRSFDDSGSGYCRSEAVVAVLLTKKSLARRVYATILNAGTNTDGSKEQGVTFPSGEVQEQLICSLYQPAGLAPESLEYIEAHGTGTKVGDPQELNGITRSLCAFRQAPLLIGSTKSNMGHPEPASGLAALTKVLLSLEHGVWAPNLHFHNPNPEIPALLDGRLQVVDRPLPVRGGNVGINSFGFGGSNVHVILQPNTRQAPAPTAHAALPHLLHASGRTLEAVQDLLEQGRQHSQDLAFVSMLNDIAATPTAAMPFRGYTVLGVEGRVQEVQQVSTNKRPLWFICSGMGTQWRGMGLSLMRLDSFRESILRSDEAVKPLGVKVSDLLLSTDERTFDDIVHAFVSLTAIQIALIDLLTSVGLKPDGIIGHSLGEVACGYADGCLSQREAVLAAYWRGQCIKDAHLPPGSMAAVGLSWEECKQRCPAGVVPACHNSEDTVTISGPQAAVNEFVEQLKQEGVFAKEVRTGGLAFHSYFMEGIAPTLLQALKKVIREPRPRSARWLSTSIPEAQWQSSLARTSSAEYNVNNLVSPVLFQEALWHIPEHAVVLEIAPHALLQAVLKRGVKSSCTIIPLMKRDHKDNLEFFLTNLGKVHLTGINVNPNALFPPVEFPAPRGTPLISPHIKWDHSQTWDVPVAEDFPNGSSSSSATVYSIDASPESPDHYLVDHCIDGRVIFPGTGYLCLVWKTLARSLGLSLEETPVVFENVSFHQATILPKTGTVALEVRLLEASHAFEVSDTGNLIVSGKVYLWEDPNSKLFDHPEVPTPPESASVSRLTQGEVYKELRLRGYDYGPQFQGICEATLEGEQGKLLWKDNWVTFMDTMLQVSILGSSQQSLQLPTRVTAIYIDPATHRQKVYRLKEDTQVADVTTSRCLGITVSGGIHISRLQTTATSRRQQEQLVPTLEKFVFTPHMEAECLSESTALQKELQLCKGLARALQTKATQQGLKAAMLGQEDPPQHGLPRLLAAACQLQLNGNLQLELGEALAQERLLLPEDPLISGLLNSQALKACVDTALENLSTLKMKVAEVLAGEGHLYSRIPALLNTQPMLQLEYTATDRHPQALKDVQTKLQQHDVAQGQWNPSDPAPSSLGALDLLVCNCALATLGDPALALDNMVAALKEGGFLLVHTVLKGHALGETLACLPSEVQPAPSLLSQEEWESLFSRKALHLVGLKRSFYGTALFLCRRAIPQEKPIFLSVEDTSFQWVDSLKSTLATSSSQPVWLTAMDCPTSGVVGLVNCLRKEPGGHRIRCILLSNLSNTSHAPKLDPGSPELQQVLKHDLVMNVYRDGAWGAFRHFQLEQDKPKEQTAHAFVNVLTRGDLASIRWVSSPLKHTQPSSSGAQLCTVYYASLNFRDIMLATGKLSPDAIPGKWASRDCMLGMEFSGRDRCGRRVMGLVPAEGLATSVLLSSDFLWDVPSSWTLEEAASVPVVYTTAYYSLVVRGRIQRGETVLIHSGSGGVGQAAISIALSLGCRVFTTVGSAEKRAYLQARFPQLDDTSFANSRDTSFEQHVLLHTGGKGVDLVLNSLAEEKLQASVRCLAQHGRFLEIGKFDLSNNHPLGMAIFLKNVTFHGILLDALFEEANDSWREVAALLKAGIRDGVVKPLKCTVFPKAQVEDAFRYMAQGKHIGKVLVQVREEEPEAVLPGAQPTLISAISKTFCPAHKSYIITGGLGGFGLELARWLVLRGAQRLVLTSRSGIRTGYQAKHIREWRRQGIQVLVSTSNVSSLEGARALIAEATKLGPVGGVFNLAMVLRDAMLENQTPELFQDVNKPKYNGTLNLDRATREACPELDYFVAFSSVSCGRGNAGQTNYGFANSTMERICEQRRHDGLPGLAVQWGAIGDVGIVLEAMGTNDTVIGGTLPQRISSCMEVLDLFLNQPHAVLSSFVLAEKKAVAHGDGDTQRDLVKAVAHILGIRDLAGINLDSTLADLGLDSLMGVEVRQILEREHDLVLPMREVRQLTLRKLQEMSSKTDSATDTTAPKSRSDTSLKQNQLNLSTLLVNPEGPTLTQLNSVQSSERPLFLVHPIEGSTTVFHSLAAKLSVPTYGLQCTQAAPLDSIPNLAAYYIDCIKQVQPEGPYRIAGYSFGACVAFEMCSQLQAQQGPAPTHNNLFLFDGSHTYVLAYTQSYRAKMTPGCEAEAEAEALCFFIKQFLDVEHSKVLEALLPLKSLEDRVAASVDLITKSHHSLDRRELSFAAVSFYHKLRAADQYKPKAKYHGNVTLLRAKTGGTYGEDLGADYNLSQVCDGKVSVHIIEGDHRTLLEGSGLESIINIIHSSLAEPRVSVREG

SEQ ID NO: 2 - protein, 2505 aa, Rattus norvegicus
MEEVVIAGMSGKLPESENLQEFWANLIGGVDMVTDDDRRWKAGLYGLPKRSGKLKDLSKFDASFFGVHPKQAHTMDPQLRLLLEVSYEAIVDGGINPASLRGTNTGVWVGVSGSEASEALSRDPETLLGYSMVGCQRAMMANRLSFFFDFKGPSIALDTACSSSLLALQNAYQAIRSGECPAAIVGGINLLLKPNTSVQFMKLGMLSPDGTCRSFDDSGNGYCRAEAVVAVLLTKKSLARRVYATILNAGTNTDGCKEQGVTFPSGEAQEQLIRSLYQPGGVAPESLEYIEAHGTGTKVGDPQELNGITRSLCAFRQSPLLIGSTKSNMGHPEPASGLAALTKVLLSLENGVWAPNLHFHNPNPEIPALLDGRLQVVDRPLPVRGGIVGINSFGFGGANVHVILQPNTQQAPAPAPHAALPHLLHASGRTMEAVQGLLEQGRQHSQDLAFVSMLNDIAATPTAAMPFRGYTVLGVEGHVQEVQQVPASQRPLWFICSGMGTQWRGMGLSLMRLDSFRESILRSDEALKPLGVKVSDLLLSTDEHTFDDIVHSFVSLTAIQIALIDLLTSMGLKPDGIIGHSLGEVACGYADGCLSQREAVLAAYWRGQCIKDANLPAGSMAAVGLSWEECKQRCPPGVVPACHNSEDTVTISGPQAAVNEFVEQLKQEGVFAKEVRTGGLAFHSYFMEGIAPTLLQALKKVIREPRPRSARWLSTSIPEAQWQSSLARTSSAEYNVNNLVSPVLFQEALWHVPEHAVVLEIAPHALLQAVLKRGVKPSCTIIPLMKRDHKDNLEFFLTNLGKVHLTGIDINPNALFPPVEFPVPRGTPLISPHIKWDHSQTWDIPVAEDFPNGSSSSSATVYNIDASSESSDHYLVDHCIDGRVLFPGTGYLYLVWKTLARSLSLSLEETPVVFENVTFHQATILPRTGTVPLEVRLLEASHAFEVSDSGNLIVSGKVYQWEDPDSKLFDHPEVPIPAESESVSRLTQGEVYKELRLRGYDYGPHFQGVYEATLEGEQGKLLWKDNWVTFMDTMLQISILGFSKQSLQLPTRVTAIYIDPATHLQKVYMLEGDTQVADVTTSRCLGVTVSGGVYISRLQTTATSRRQQEQLVPTLEKFVFTPHVEPECLSESAILQKELQLCKGLAKALQTKATQQGLKMTVPGLEDLPQHGLPRLLAAACQLQLNGNLQLELGEVLARERLLLPEDPLISGLLNSQALKACIDTALENLSTLKMKVVEVLAGEGHLYSHISALLNTQPMLQLEYTATDRHPQALKDVQTKLQQHDVAQGQWDPSGPAPTNLGALDLVVCNCALATLGDPALALDNMVAALKDGGFLLMHTVLKGHALGETLACLPSEVQPGPSFLSQEEWESLFSRKALHLVGLKKSFYGTALFLCRRLSPQDKPIFLPVEDTSFQWVDSLKSILATSSSQPVWLTAMNCPTSGVVGLVNCLRKEPGGHRIRCILLSNLSSTSHVPKLDPGSSELQKVLESDLVMNVYRDGAWGAFRHFQLEQDKPEEQTAHAFVNVLTRGDLASIRWVSSPLKHMQPPSSSGAQLCTVYYASLNFRDIMLATGKLSPDAIPGKWASRDCMLGMEFSGRDKCGRRVMGLVPAEGLATSVLLSPDFLWDVPSSWTLEEAASVPVVYTTAYYSLVVRGRIQHGETVLIHSGSGGVGQAAISIALSLGCRVFTTVGSAEKRAYLQARFPQLDDTSFANSRDTSFEQHVLLHTGGKGVDLVLNSLAEEKLQASVRCLAQHGRFLEIGKFDLSNNHPLGMAIFLKNVTFHGILLDALFEGANDSWREVAELLKAGIRDGVVKPLKCTVFPKAQVEDAFRYMAQGKHIGKVLVQVREEEPEAMLPGAQPTLISAISKTFCPEHKSYIITGGLGGFGLELARWLVLRGAQRLVLTSRSGIRTGYQAKHVREWRRQGIHVLVSTSNVSSLEGARALIAEATKLGPVGGVFNLAMVLRDAMLENQTPELFQDVNKPKYNGTLNLDRATREACPELDYFVAFSSVSCGRGNAGQSNYGFANSTMERICEQRRHDGLPGLAVQWGAIGDVGIILEAMGTNDTVVGGTLPQRISSCMEVLDLFLNQPHAVLSSFVLAEKKAVAHGDGEAQRDLVKAVAHILGIRDLAGINLDSSLADLGLDSLMGVEVRQILEREHDLVLPIREVRQLTLRKLQEMSSKAGSDTELAAPKSKNDTSLKQAQLNLSILLVNPEGPTLTRLNSVQSSERPLFLVHPIEGSITVFHSLAAKLSVPTYGLQCTQAAPLDSIPNLAAYYIDCIKQVQPEGPYRVAGYSFGACVAFEMCSQLQAQQGPAPAHNNLFLFDGSHTYVLAYTQSYRAKLTPGCEAEAEAEAICFFIKQFVDAEHSKVLEALLPLKSLEDRVAAAVDLITRSHQSLDRRDLSFAAVSFYYKLRAADQYKPKAKYHGNVILLRAKTGGTYGEDLGADYNLSQVCDGKVSVHIIEGDHRTLLEGRGLESIINIIHSSLAEPRVSVREG

SEQ ID NO: 3 - protein, 2503 aa, Cricetulus griseus
MEEVVIAGMSGKLPESENLQEFWANLIGGVDMVTDDDRRWKAGLYGLPKRSGKLKDLSKFDASFFGVHPKQAHTMDPQLRLLLEVSYEAIVDGGINPASLRGTNTGVWVGVSGSEASEALSRDPETLLGYSMVGCQRAMMANRLSFFFDFKGPSIALDSACSSSLLALQSAYQAIRNGECPAALVGGINVLLKPNTSVQFMKLGMLSPEGTCKSFDDSGNGYCRSEAVVAVLLTKKSLARRVYATILNAGTNTDGCKEQGVTFPSGEAQEQLIQSLYRPAGLAPESLEYIEAHGTGTKVGDPQELNGIVRSLCASRQGPLLIGSTKSNMGHPEPASGLAALTKVLLSLENGVWAPNLHFHNPNPEIPALLDGRLQVVDRPLPVRGGNVGINSFGFGGANVHVILQPNTQQAPAPAPHAALPHLLHASGRTAEAVQGLLEQGRKHSQDMAFVSMLNDIAATPTAAMPFRGYTVLGVEGDVQEVQQVPASKRPLWFICSGMGTQWRGMGLSLMRLDSFRESILRSDEAVKPLGIKVSDLLLSTDESTFDDIVHAFVGLTAIQIALIDLLTSVGLKPDGIIGHSLGEVACGYADGCLSQREAVLAAYWRGQCIKDAHLPPGSMAAVGLSWEECKQRCPSGVVPACHNSEDTVTISGPQAAVSEFVEQLKQEGVFAKEVRTGGLAFHSYFMEGIAPMLLQALKKVIREPRPRSARWLSTSIPEAQWQSSLARTSSAEYNVNNLVSPVLFQEALWHVPEHAVLLEIAPHALLQAVLKRGVKSSCTIIPLMKRDHKDNLEFFLTNLGKVHLTGIDVNPNALFPPVDFPAPRGTPLISPHIKWDHSQTWDVPAAEDFPNGSCSSSATVYSIDASPESPDHYLVDHCIDGRVLFPATGYLYLVWKTLARNLSLSLEETPVVFEDVTIHQATILPKTGTVPLEVRLLEASRAFEVSENGNLIVSGKVYQWEDPDSKLFDHPHVLNPPESTPVSRLTQTEVYKELRLRGYDYGPHFQGIVEASLEGEQGKLLWKGNWVTFLDTMLQVSILGVSQQSLRLPVRVTAIHIDPATHLQKVYTLEGENQVADVTTSLCLDSTVSGGVRISRLHTTAAPRRQQEQLVPTLEKFIFTPHVEDGCLSENTTLQRELQLCKDLAQALQTKATQQGLKMTVPGLEGPPQHGLSRLLAAACQLQLNGNLQLELGEALAQERVLLPEDPLISGLLNSQALKACVDTALENLPSLKMKVVEVLSGEGRLYSRIPSLLNTQPMLQLEYTATDLHPEALKDVQAKLQQHDIAQGQWNPEDPAPSNLGALDLVVCSCAVATLGNPALALSNMVAALKEGGFLLMHTVLRGHSLGETLACLPSAVQPGPSLSQEEWESLFSKKGLHLVGLKKSFYGTALFLCRRATLQDNPLFLPVEDTSYQWVDSLKRILAESSSQPVWLTATDCPTSGVVGLVNCLRKEPGGHRIRCILLSNLSTSSHTPKMGPGSSELQKVLKNDLVMNVYRDGAWGAFRHFLLEQDKPEEQTAHAFVNVLTRGDLASIRWVCSPLKHAQPTSPGTQLCTVYYASLNFRDIMLATGKLPPDAIPGKWASRDCMLGMEFSGRDKCGRRVMGLVPAEGLATSVLLSPDFLWEVPSSWTLEEAASVPVVYTTAYYSLVVRGRVQRGETVLIHSGSGGVGQAAISIALSLGCRVFTTVGSAEKRAYLQARFPQLDDTSFANSRDTSFEQHVLLHTGGKGVNLVLNSLAEEKLQASVRCLAQHGRFLEIGKFDLSNNHPLGMAIFLKNVTFHGILLDALFEEANDSWREVAALLQAGIRDGVVKPLKCTVFPKDQVEDAFRFMAQGKHIGKVLVQVREEEPEAVLPGAQPTLIPAISKTFCPAHKSYIITGGLGGFGLELARWLVLRGAQRLVLTSRSGIRTGYQAKQVQEWRRQGIHVLVSTSNASSLEGARALITEATKLGPVGGVFNLAMVLRDAMLENQTPELFQDVNKPKYNGTLNLDRTTREACPELDYFVAFSSVSCGRGNAGQTNYGFANSAMERICEQRRHDGLPGLAVQWGAIGDVGIVLEAMGTNDTVIGGTLPQRIASCMEVLDLFLNQPYAVLSSFVLAEKKAVAQGDGEAQRDLVKAVAHILGIRDLAGVNLDSSLADLGLDSLMGVEVRQILEHEHDLVLPMREVRQLTLRKLEELSSKAGSASETTAPKSKNDTALKQTQLNLSTLLVNPEGPTLTRLNSVQSSERPLFLVHPIEGSTTVFHSLAAKLSVPTYGLQCTQAAPLDSIPDLAAYYIDCIKQVQPEGPYRVAGYSFGACVAFEMCSQLQAQQGPTPTHNSLFLFDGSHTYVLAYTQSYRARMTPGCEAEAEAEAICYFIKQFTDAEHNKVLEALLSLKSLEDRVTAAVDLITKSHHSLDRRELSFAALSFYQKLRAADQYKPKAKYHGNVTLLRAKTGGTYGEDLGADYNLSQVCDGKVSVHIIEGDHRTLLEGSGLESIINIIHSSLAEPRVSVREG

SEQ ID NO: 4 - protein, 2511 aa, Homo sapiens
MEEVVIAGMSGKLPESENLQEFWDNLIGGVDMVTDDDRRWKAGLYGLPRRSGKLKDLSRFDASFFGVHPKQAHTMDPQLRLLLEVTYEAIVDGGINPDSLRGTHTGVWVGVSGSETSEALSRDPETLVGYSMVGCQRAMMANRLSFFFDFRGPSIALDTACSSSLMALQNAYQAIHSGQCPAAIVGGINVLLKPNTSVQFLRLGMLSPEGTCKAFDTAGNGYCRSEGVVAVLLTKKSLARRVYATILNAGTNTDGFKEQGVTFPSGDIQEQLIRSLYQSAGVAPESFEYIEAHGTGTKVGDPQELNGITRALCATRQEPLLIGSTKSNMGHPEPASGLAALAKVLLSLEHGLWAPNLHFHSPNPEIPALLDGRLQVVDQPLPVRGGNVGINSFGFGGSNVHIILRPNTQPPPAPAPHATLPRLLRASGRTPEAVQKLLEQGLRHSQDLAFLSMLNDIAAVPATAMPFRGYAVLGGERGGPEVQQVPAGERPLWFICSGMGTQWRGMGLSLMRLDRFRDSILRSDEAVKPFGLKVSQLLLSTDESTFDDIVHSFVSLTAIQIGLIDLLSCMGLRPDGIVGHSLGEVACGYADGCLSQEEAVLAAYWRGQCIKEAHLPPGAMAAVGLSWEECKQRCPPGVVPACHNSKDTVTISGPQAPVFEFVEQLRKEGVFAKEVRTGGMAFHSYFMEAIAPPLLQELKKVIREPKPRSARWLSTSIPEAQWHSSLARTSSAEYNVNNLVSPVLFQEALWHVPEHAVVLEIAPHALLQAVLKRGLKPSCTIIPLMKKDHRDNLEFFLAGIGRLHLSGIDANPNALFPPVEFPAPRGTPLISPLIKWDHSLAWDVPAAEDFPNGSGSPSAAIYNIDTSSESPDHYLVDHTLDGRVLFPATGYLSIVWKTLARALGLGVEQLPVVFEDVVLHQATILPKTGTVSLEVRLLEASRAFEVSENGNLVVSGKVYQWDDPDPRLFDHPESPTPNPTEPLFLAQAEVYKELRLRGYDYGPHFQGILEASLEGDSGRLLWKDNWVSFMDTMLQMSILGSAKHGLYLPTRVTAIHIDPATHRQKLYTLQDKAQVADVVVSRWLRVTVAGGVHISGLHTESAPRRQQEQQVPILEKFCFTPHTEEGCLSERAALQEELQLCKGLVQALQTKVTQQGLKMVVPGLDGAQIPRDPSQQELPRLLSAACRLQLNGNLQLELAQVLAQERPKLPEDPLLSGLLDSPALKACLDTAVENMPSLKMKVVEVLAGHGHLYSRIPGLLSPHPLLQLSYTATDRHPQALEAAQAELQQHDVAQGQWDPADPAPSALGSADLLVCNCAVAALGDPASALSNMVAALREGGFLLLHTLLRGHPLGDIVAFLTSTEPQYGQGILSQDAWESLFSRVSLRLVGLKKSFYGSTLFLCRRPTPQDSPIFLPVDDTSFRWVESLKGILADEDSSRPVWLKAINCATSGVVGLVNCLRREPGGNRLRCVLLSNLSSTSHVPEVDPGSAELQKVLQGDLVMNVYRDGAWGAFRHFLLEEDKPEEPTAHAFVSTLTRGDLSSIRWVCSSLRHAQPTCPGAQLCTVYYASLNFRDIMLATGKLSPDAIPGKWTSQDSLLGMEFSGRDASGKRVMGLVPAKGLATSVLLSPDFLWDVPSNWTLEEAASVPVVYSTAYYALVVRGRVRPGETLLIHSGSGGVGQAAIAIALSLGCRVFTTVGSAEKRAYLQARFPQLDSTSFANSRDTSFEQHVLWHTGGKGVDLVLNSLAEEKLQASVRCLATHGRFLEIGKFDLSQNHPLGMAIFLKNVTFHGVLLDAFFNESSADWREVWALVQAGIRDGVVRPLKCTVFHGAQVEDAFRYMAQGKHIGKVVVQVLAEEPEAVLKGAKPKLMSAISKTFCPAHKSYIIAGGLGGFGLELAQWLIQRGVQKLVLTSRSGIRTGYQAKQVRRWRRQGVQVQVSTSNISSLEGARGLIAEAAQLGPVGGVFNLAVVLRDGLLENQTPEFFQDVCKPKYSGTLNLDRVTREACPELDYFVVFSSVSCGRGNAGQSNYGFANSAMERICEKRRHEGLPGLAVQWGAIGDVGILVETMSTNDTIVSGTLPQRMASCLEVLDLFLNQPHMVLSSFVLAEKAAAYRDRDSQRDLVEAVAHILGIRDLAAVNLDSSLADLGLDSLMSVEVRQTLERELNLVLSVREVRQLTLRKLQELSSKADEASELACPTPKEDGLAQQQTQLNLRSLLVNPEGPTLMRLNSVQSSERPLFLVHPIEGSTTVFHSLASRLSIPTYGLQCTRAAPLDSIHSLAAYYIDCIRQVQPEGPYRVAGYSYGACVAFEMCSQLQAQQSPAPTHNSLFLFDGSPTYVLAYTQSYRAKLTPGCEAEAETEAICFFVQQFTDMEHNRVLEALLPLKGLEERVAAAVDLIIKSHQGLDRQELSFAARSFYYKLRAAEQYTPKAKYHGNVMLLRAKTGGAYGEDLGADYNLSQVCDGKVSVHVIEGDHRTLLEGSGLESIISIIHSSLAEPRVSVREG

SEQ ID NO: 5 - protein, 2510 aa, Macaca mulatta
MEEVVIAGMSGKLPESENLQEFWDNLIGGVDMVTDDDRRWKAGLYGLPRRSGKLKDLSRFDASFFGVHPKQAHTMDPQLRLLLEVTYEAIVDAGINPASLRGTHTGVWVGVSGSEASEALSRDPETLVGYSMVGCQRAMMANRLSFFFDFKGPSIALDTACSSSMVALQSAYQAISSGQCPAAIVGGINVLLKPNTSVQFLRLGMLSPEGTCKAFDAEGNGYCRSEGVVAVLLTKKSLARRVYATILNAGTNTDGCKEQGVTFPSGEAQEQLIRSLYQSAGVAPESFEYIEAHGTGTKVGDPQELNGIARALCATRQEPLLVGSTKSNMGHPEPVSGLAALAKVLLSLEHGLWAPNLHFHSPHPEIPALLDGRLQVVAQPLPVRGGNVGINSFGFGGSNVHVILRPHTQPPPAPAPHASLPRLLRASGRTPEAVQELLEQGLQHSQELAFLSMLNDIAAIPTTAMPFRGYAVLGGEHSGPEVQQVPAGERPLWFICSGMGTQWRGMGLSLMRLDRFRDSILRSDEAVKPFGLKVSQLLLSMDESTFDDIVHAFVSLTAIQIGLIDLLSCMGLRPDGIIGHSLGEVACGYADGCLSQEEAVLAAYWRGQCIKEAHLPPGAMAAVGLSWEECKQRCPPGVVPACHNSKDTVTISGPQASVFEFMEQLRKEGVFAKEVRTGGMAFHSYFMEAIAPPLLQALKKVIREPKPRSARWLSTSIPEAQWHSSLARTSSAEYNVNNLVSPVLFQEALCHVPEHAVVLEVAPHALLQAVLKRGLKPGCTIIPLMKKDHRDNLEFFLTGIGRLHLSGIDANPNALFPPVEFPAPRGTPLISPLIKWDHSLAWDVPAAEDFPNGSGSPSAAVYNIDTSSESPDHYLVDHTIDGRVIFPATGYLCIVWKTLARALGLAVEQLPVVFEDVVLHQATILPKTGTVSLEVRLLEASRAFEVSQNGNLIVSGKVYQWEDPDPRLFNHPESPTPNPEEPLFLTQAEVYKELRLRGYDYGPHFHGILEASLEGESGRLLWKDNWVSFLDAMLQISILGLAKRSLPLPTRITAIHIDPATHRQKLYTLQDDAQVADVVVSRWLSITVAGGVHMSRVHTESAPRRQQDQQVPILEKFCFTPHVEEGCLSERAALQKELQLCKGLAQALQTKVTQQGLRMVVPGLDGAQVPQDPLQQGLPQLLSAACRLQLNGNLQLELAQVLAQKRPELSEDPLLSGLLDSPALRACLDTAVENMPSRKMKVVEVLAGHGHLYSRIPGLLGAQPLLQLSYTATDRHPQALEAAEAQLQQHDIAQGQWDPADPAPSTLGSTDLLVCNCAVAALGDPASALSNMVATLREGGFLLLHTLLRGHPLGETVAFLTSAEPQYGQGILSQDAWESLFSSVSLRLVGLKKSFYGSALFLCRRPAPQDSPIFLPVDDTSFRWVESLKGILADEDSSRPVWLKAVNCATSGVVGLVNCLRQEPGGHRLRCVLLSNLSSTSRVPEVDPGSAELQKVLQGDLVMNVYRDGAWGAFRHFLLEEDKPEEPTAHAFVTTLTRGDLSSIRWVCSSLRHAQPSRPGAQLCTVYYASLNFRDIMLATGKLSPEAIPGKWASQDNLLGMEFSGRDPSGKRVMGLVPAEGLATSVLLSPDFLWDVPSNWTLEEAASVPVVYCTAYYSLVVRGRVRPGETVLIHSGSGGVGQAAIAIALSLGCRVFTTVGSSEKRAYLQARFPQLDSTSFANSRDTSFEQHVLRHTGGKGVDLVLNSLAEEKLQASVRCLAQHGRFLEIGKFDLSQNHPLGMAIFLKNVTFHGILLDALLDGSAEWQEVAALLQAGIRDGVVQPLKCTVFPGAQVEDAFRYMAQGKHIGKVLVQVLAEEPEAVLKGAKPTLMSAISKTFCPAYKSYIIAGGLGGLGLELAQWLIQRGAQKLVLTSRSGVRTGYQAKQVRQWRRQGVQVLVSTSNISSLEGARGLIAEAAQLGPVGGIFNLTMVLRDAMLENQTPEFFQDVCKPKYSGTLNLDRVTREACPELDYFVVFSSVSSGRGNAGQSNYGFANSAMERICEKRRHEGLPGLAVQWGAIGDVGILADTVNIHATVIGGTLPQRVASCLEVLDLFLNQPHMVLSSFVLAEKAAAYRDRDGEQDLVKAVAHILGIRDLAAINLDSSLADLGLDSLMSVEVRQTLERELNLVLSMREVRQLTLRRLQELSLKADAANDLASPTPKEDGPAQQQTQLNLRSLLVNPEGPTLMRLNSVQSSERPLFLVHPIEGSTTVFHSLASRLSIPTYGLQCTRAAPLDSIHSLAAYYIDCIRQVQPEGPYRVAGYSYGACVAFEMCSQLQAQQNPAPTHNSLFLFDGSHTYVLAYTQSYRAKLTPGCEAEAETEAICFFVQQFTDMEHNRVLEALLPLKGLEERVAAAVDLIIKSHQGLDRQELSFAALSFYYKLRAAEQYTPKAKYHGNVMLLRAKTGGAYGEDLGADYNLSQVCDGKVSVHVIEGDHRTLLEGSGLESIVSIIHSSLAEPRVSVREG

SEQ ID NO: 6 - protein, 2513 aa, Bos taurus
MEEVVITGMSGKLPESENLEEFWANLIGGVDMVTDDDRRWKAGLYGLPRRSGKLKDLSRFDASFFGVHPKQAHNMDPQLRLLLEVTYEAIVDAGINPASIRGTNTGVWVGVSGSEASEALSRDPETLVGYSMVGCQRAMLANRLSFFFDFKGPSITLDTACSSSLLALQRAYQAIQRGECAMAIVGGVNIRLKPNTSVQFMKLGMLSPEGTCKFFDASGNGYCRAKAVMAILLTKKSLARRVYATILNAGTNTDGCKEKGVTFPSGEAQEQLISSLYKPAGLDPETLEYVEAHGTGTKVGDPQELNGIVQALCGTRQSPLRIGSTKSNMGHPEPASGLAALAKVLLSLEHGLWAPNLHFHNPNPKIPALQDGRLQVVDRPLPVLGGNVGINSFGFGGSNVHVILQPNSQPLPPPAPHAALPRLLRASGRTLEGVQGLLELGLQHSQNLAFVSMLNDIATPSPAAMPFRGYAVLGSQGGSQKVQQVLAGKRPLWFICSGMGTQWRGMGLSLMRLSRFRDSILRSDEAVKPLGLQVSQLLLSTDEAIFDDMVISFVSLTAIQIALIDLLTSMGLQPDGIIGHSLGEVACGYADGCISQEEAILSAYWRGQCIKEANIPPGAMAAVGLTWEECKQRCPPGIVPACHNCIDTVTISGPQASMLEFVQQLKQEGVFAKEVRTGGMAFHSYFMDAIAPMLLQQLKKVIREPQPRSPRWLSTSIPETQWQESLARTFSAEYNVNNLVSPVLFQEALWRVPEDAVVLEIAPHALLQAVLKRGLKSSCTIIPLMKKDHRDNLEFFLSNVGQLYLTGIDVNPNGLFPPVEFPAPRGTPLISPHIKWDHSQTWDVPTAEDFPSGSSSSSATIYKIDINPESPDHYLVDHCIDGRIIFPGTGYLCLVWKTLARALDQNMEHTPVVFEDVTLHQAVILPKTGIVLLKVRLLEASCTFEVSENGNLIASGKVYQWEDPNPKLFDNRYGPDPATPVDPTTAIHLSRGDVYKELQLQGFNYGPYFQGILEASSEGNTGQLLWKDNWVTFMDTMLQMSILAPSKRSLRLPTRITAIYIHPATHQQKLYTLQDKTQVADVVINRCLDTTVAGGIYISRIHTSVAPRHQQEQLVPILEKFCFTPHVETGCLAGNLALQEELQLCVGLAQALQTRVAQQGIKMVVPGLDGAQAPQEAPQQGLPRLLATACQLQLNGNLQMEMGQILAQERALLCDDPLLSGLLNSPALKACVTLALENMTSLKMKVVLAGDGQLYSRIPTLLNTQPLLELDYTATDRHPQALEAAQAKLQQLDITQGQWDPSDPAPSNLGGANLVVCNYALASLGDPATAVGNMVAALKEGGFLLLHTLLRGHPLGETVTFLTCPEPQQGQRHLLSQDEWERLFAGASLHLVALKKSFYGSVLFLCRRLAPLDSPIFLPVEDTSFQWVDSLKNILADSSSRAVWLMAVGCTTSGVVGLVNCLRKEPDGHRIRCVLVSNLNSTSPIPETDPKSLELQKVLQSDLVMNVYRDGAWGAFRHFPLEQDKPEEQTEHAFINVLTRGDLSSIRWVCSPLRHSQPTAPGFQLCTIYYASLNFKRNHAGHGQAVPRRHPRNWASRNCLLGMEFSGRDASGKRVMGLVPAEGLATSTLVPQSFLWDVPSNWTLEEAASVPVVYSTAYYALMVRGRMQPGETVLIHSGSGGVGQAAIAIALSLGCRVFPLVGSAEKRAYLQSRFPQLNETSFANSRDTSFEQHVLWHTAGKGADLVLNSLAEEKLQASVRCLAQHGRFLEIGKFDLSKNHPLGMAIFLKNVTFHGILLDSLFEENNTMWQEVSTLLKAGIRKGVVQPLKRTVFPRTQAEDAFRYMAQGKHIGKVVIQVREEEQEAVLHGTKPTQMVALCKTFCPAHKSYIITGGLGGFGLELAHWLVERGAQKLVLTSRSGIRTGYQARQVHEWRRQGVQVLVSTSDVSTLDGTRSLITEAAQLGPVGGIFNLAVVLRDAMLDNQTPEFFQDVNKPKYNGTLNLDRVTREACPELDYFEVFSSVSCGRGNAGQTNYGFANSTMERICEKRRHDGLPGLAVQWGAIADVGLLMELKGTKDKAIGGTLPQRITSCMEVLDLFLNQPHPVLSSFVLAEKATSRGPSGSHQDLVKAVTHILGIRDLATVNLDSSLSDLGLDSLMGVEVRQMLEREHNLLLSMREIRQLTIHKLQEISAQAGTADELTDSTPKFGSPAQSHTQLNLSTLLVNPEGPTLTRLNSVQSSERPLFLVHPIEGSTTVFHSLATKLSIPTYGLQCTGAAPLDSIQSLATYYIECIRQVQPEGNYRIAGYSYGACVAFEMCSQLQAQQNAGPTNNSLFLFDGSHTFVMAYTQSYRAKLNPGCEAEAEAEAMCFFMQQFTEAEHSRVLEALLPLGDLEARVAATVELIVQSHAGLDRHALSFAARSFYHKLRAAEEYTPRATYHGNVTLLRAKMGSAYQEGLGADYNLSQVCDGKVSVHIIEGDHRTLLEGSGLESILSIIHSSLAEPRVSVREG

SEQ ID NO: 7 - protein, 2514 aa, Capra hircus
MEEVVIAGMSGKLPESENLEEFWANLIGGVDMVTDDDRRWKAGLYGLPRRSGKLKDLSRFDASFFGVHPKQAHNMDPQLRLLLEVAYEAIVDAGINPASIRGTNTGVWVGVSGSEAAEALSRDPETLVGYSMVGCQRAMMANRLSFFFDFKGPSIALDTACSSSLLALQRAYQAIQRGECAMAIVGGINILLKPNTSLQFMKLGMLSPEGTRKSFDASGDGYCRAEAVMAVFLTKKSLARRVYATILNAGTNTDGCKKQGVTYPSGEAQEQLISSLYKPAGLDPETLEYIEAHGTGTKVGDPEELNGITQALCGTRQGPLLIGSTKSNMGHPEPASGLAALAKVLLSLEHGLWAPNLHYHNPNPKIPALQDGRLQVVDRPLPVLGGIVGINSFGFGGSNVHVILQPNSQPPPPPGPHAALPRLLRASGRTLEGVQGLLELGLQHSQNLAFVSMLNDIAAPSPAAMPFRGYAVLGSQEGSQEVQQVPTSKRPLWFICSGMGTQWRGMGLSLMRLSSFRDSILRSDEAVKPLGLRVSQLLLSADDIFDDIIVSFVSLTAFQIALIDLLTSMGLRPDGIIGHSLGEVACAYADGCISQEEAILSAYWRGQCIKEANIPPGAMAAVGLTWEECKQRCPPGIVPACHNSIDTVTISGPQASMLEFVKQLKQEGVFAKEVQTGGMAFHSYFMDAIAPTLLQQLKKVIREPQLRSPRWLSTSIPESQWHESLARTFSAEYNVNNLVSPVLFQEALWHVPENAVVLEIAPHALLQAILKRGLQPSCTIIPLMKKDHRDNLEFFLSNVGQLYLTGIDVNPNGLFPPVEFPAPRGTPLISPHIKWDHSQTWDVPAAEDFPNGSSSSSATVYKIDISPESPDHYLVDHCIDGRVLFPATGYLCLVWKTLARALDQNTEHTPVVFEDVMLHQATLLPKTGTVLLEVRLLEASCTFEVSEKGSLIVSGKVYQWEDPDPKLFDNRYGTEPATPVDPTTAIHLRCGDVYKELQLQGFNYGPNFQGILETSSEGNMGQLLWKDNWVTFMDTMLQMSILAPGQRSLRLPTRITAIYIHPATHQQKLYTLQDGTQVADVVMNRCLDTTVAGGVYISRIHTSVAPRHQQEQPVPILEKFCFTPHVESGCLAGNLALQEELQLCVGLAQALQTKVAQQGIKMVVPGLDGTQASQEAPQQGLPQLLATACQLQLNGNLQMGMGQILAQERALLCDDPLLSGLLNSPALKACVDTALENMTSLKMKVVEVLAGDGQLYSRIPALLNTQPLLELDYIATDRHPQALEAAQAKLQQLNITQGQWDPSDPAPSNLGGANLVVCNCALASLGDPATAVGNMVAALKEGGFLLLHTLLRGHPLGETVTFLTCPEPQQGQRHLLSQDEWESLFAGTSLHLVALKKSFYGSVLFLCRRLAPRDSPIFLPVEDTSFQWVDSLKNILADSSSRPVWFMAVGCTTSGVVGLVNCLRKEPDGHRIRCVLVSNLNSTSPIPEIAPKSLELQKVLQSDLVMNVYRDGAWGAFRHFLLEQDKPEEQTEHAFINVLTRGDLSSIRWVCSPLRHSQSTGPGVQLCTIYYASLNFRDIMLATGKLSPDAIPGNWASRNCMLGMEFSGRDASGKRVMGLVPAEGLATSTLVPQSFLWDVPSNWTLEEAASVPVVYSTAYYALIVRGRMQPGETVLIHSGSGGVGQAAIAIALSLGCCVFTTVGSAEKRAYLQSRFPQLNETSFANSRDTSFEQHVLWHTAGKGVDLVLNSLAEEKLQASARCLAQHGRFLEIGKFDLSNNHPLGMAIFLKNVTFHGILLDALFEENSTMWQEVSSLLKAGIREGVVQPLKRTVFPRTQVEDAFRYMAQGKHIGKVVIQVREEEQKAVLHGTKPTQMAALCKTFCPAHKSYVITGGLGGFGLELAHWLVERGAQKLVLTSRSGIRTGYQARQVREWRRQGVQVLVSTRDVSSLDGTQRLITEAAQLGPVGGVFNLAVVLRDAMLDNQTPEFFQDVNKPKYNGTLNLDRVTREACPELDYFVVFSSVSCGRGNAGQTNYGFANSTMERICEKRRHDGLPGLAVQWGAIADVGILVELKGTNDKAIGGTLPQRITSCLEVPDFFLNQPHPVLSSFALAEKAASRGPSGSQQDLVKAVAHILGIRDLATVNPDSSLSDLGLDSLMGVEVRQMLERERSLTLSMREIRQLTIRKLQEISAQAGTADELTNSTHKLSSPAQSQTQLNLSTLLVNPEGPTLTRLNSVQSSERPLFLVHPIEGSTTVFHSLAAKLSIPTYGLQCTRAAPLDSIQSLAAYYIECIRQVQPEGPYRIAGYSYGACVAFEMCSQLQAQQSAGPTNNSLFLFDGSHTFVMAYTQSYRAKMNPGCEAEAEAEAMCFFMRQFMEAEHSRVLEALLPLGDLEARVAATVELIVQRHAGLDRHALSFAARSFYHKLRAAEQYTPRATYHGNVTLLRAKMGGAYGEGLGADYNLSQVCDGKVSVHIIEGDHRTLLEGSGLESILSIIHSSLAEPRVSVREG

SEQ ID NO: 8 - protein, 2489 aa, Equus caballus
MEEVVIAGMSGRLPESENMQEFWANLIGGVDMVTDDDRRWKAGLYGLPRRSGKLKDLSKFDASFFGVHPKQAHTMDPQLRLLLEVTYEAIVDGGINPALLRGTHTGVWVGVSGSEASEALSRDPETLLGYSMVGCQRAMMANRLSFFFDLKGPSITLDTACSSSLLALHNAYQAIRSGECPAAIVGGINVLLKPNTSVQFMKLGMLSPEGACKSFDEAGNGYCRSEAVVAVLLTKKSLARRVYATILNSGTNTDGSKEQGVTFPSGDAQEQLMSSLYKPAGVAPESLEYLEAHGTGTRVGDPQELKGVVRALCATRQDPLLIGSTKSNMGHPEPASGLAALAKVLLSLEHGLWAPNLHFHSPNPEIPALRDGRLQVVDRPLPIRGGNVGINSFGFGGSNVHVILQPNSRLPLVPTPHVALPCLLRASGRTSEAVLGLLEQGRQHSQDLAFVSMLNDIAATPPSAMPFRGYAVLGGEGDAQEVQQVSTGQRPLWFICSGMGAQWRGMGLSLMRLGTFRDSILRSDKAVKPLGLQVSDLLLSADEATFDDTVPGFVSLTAIQIALIDLLTSMGLRPDGIIGHSLGEVACGYADGCVSQEEAILAAYWRGQCIKEANIPPGAMAAVGLSWEECKQRCPPGVVPACHNSKDTVTISGPQAAVSEFVEQLKQEGVFAKEVRTGGLAFHSYFMDSISHTLLQALKKVIREPRPRSVRWLSTSIPEAQWQSSLARTFSAEYNVNNLVSPVLFQEALCHVPEHAVVLEIAPHALLQAVLKRGLKPSCTIVPLMKKDHRDNLEFFLSNVGRLHLMGIDVNPNGLFPPVEFPAPRGTPLISPHIKWDHSQTWYVPSAKDFPSGSSCSSSTVYNIDASPESPDHYLVDHCIDGRTLFPATGYLCLVWRTLAHALGENLEQMPVVFEDVTLYQATILPKTGTMPLEVRLLEASHTFEVSENGTLIVSGKVYQWDNPNPKLFDNRDSLDPADPTDPTATFHLAQGDVYKELRLRGYDYGPHFQGILKANLEGNTGQLLWKDNWVTFLDTMLQMSILGSAQRSLRLPTRIAAIHIDPATHQQKVYTLQGEAQVADLVVDSCLSSTVAGGAIISRLHTSLAPRRQQEQLAPTLEKFCFTPHVEGGCLAGSATLQEELQLCKGLAQALQVKVAQQGLKMVVPGLDGAQVPRESPQQGLPRLLAAACQLQLNGNLQLELGQVLAQESPLLCDDPLLSGLLDSPALKACVDTALENVASLRMKVVEVLAGDGHLYSRIPALLTTQPMLQLDYTATDRHAQALKAAQAKLQQHHVAQGQWDPMDPAPSSLGATDLLVCNCAVATLGDPATALGNMAAVLKEGGFLLLHTLLRGYPLGEMVAFLTCPEPQRGRQGLLSQDEWESLFAGASLRLVALKKSFYGSVLFLCRRPAPQDSPIFLPVEDMSFRWVDSLKNILADLSSRPVWLTAVSCSTSGVIGMANCLRKEPGGHRIRCILVSNLSNTSPVPKMDPSSSELQKVLQGDLVMNVYRDGAWGTFRHFPLEQDQPEEQTEHAFINVLTRGDLSSIRWVCSPLRHAQHPGPGLQLCTVYYASLNFRDIMLATGKLSPDAIPGKWAARDCMLGMEFSGRDASGKRVMGLVPAEGLATSVLLSQDFLWDVPSCWTLEEAASVPVVYTTAYYSLVVRGRVRRGETVLIHSGSGGVGQAAIAIALSLGCRVFTTVGSAEKRAYLQARFPQLNDTSFANSRDTSFEQHVLRHTAGKGVDLVLNSLAEEKLQASVRCLAQHGRFLEIGKFDLSNNHPLGMAVFLKNVTFHGILLDALFDETSSDWQEVVALVRAGIQDGVVQPLKCTVFPKTQVEDAFRYMAQGKHIGKVVVQVREEEPEAVLQEVKPTRMVALSKTFFPAHKSYVVVGGLGGFGLELAQWLVLRGAQKLVLTSRSGIRTGYQAKQVREWRRQGVQVLVSTCNASSLDGARGLIAEAAQLGPVGGVFNLAMVLRDAMLENQTPELFQDVNKPKYNGTLNLDRVTRETCPELDYFVAFSSVSCGRGNAGQTNYGFANSTMERICEKRRHDGLPGLAVQWGAIGDVGIILEAMGANDTVIGGTLPQRIASCLEVLDLFLNQPHPVLSSFVLAEKKAAAHSDSSSQQDLVKAVAHILGIQDLATINLDSSLVDLGLDSLMGVEVRQTLEREHDMVLSMRDIQQLTLRKLQELSSQTCMADELAAPTPKEDGLTRQQAQLNLSTLLVNPEAPTLTRLNSVQSSERPLFLVHPIEGSITVFHSLATKLSIPTYGLQCTKAAPLDSIQSLAAYYIECIRQVQPEGPYRIAGYSYGACVAFEMCSQLQAQQSSAPAHNSLFLFDGSHAYVLAYTQSYRAKLTPGCEAEAETEAMCFFIQQFTDAEHSRVLEALLPLKGLEERVVAAVDLIVQNHAGLDRRVLSFAARSFYYKLRAAEQYMPRATYHGNVTLLRAKTGSAYSEDLGADYNLSQKHDSNCCVDFEISCQLSV

SEQ ID NO: 9 - protein, 2655 aa, Felis catus
MALPAALCEALSQEHPSSRLQRLQGLLGSRYEAAGPWGGWSPQARAPEVPGQCQRPEGPVLPVKSEGWLDQCGLPHTPEASVLASPGRRSWPPGSGSHRSQTRRWCCGVRKPGERLQPGGLAAGSDQRQAPTLLPLHRAAMEEVVIAGMSGKLPESENMEEFWANLIGGVDMVTDDDRRWKAGLYGLPKRTGKLKDLSKFDASFFGVHPKQAHTMDPQLRLLLEVTYEAILDGGINPATLRGTHTGVWVGVSGSEASEALSRDPETLVGYSMVGCQRAMMANRLSFFFDFKGPSIALDTACSSSLLALQNAYQAIRRGECPAAIVGGLNLLLKPNTSVQFMKLGMLSPDGICKAFDESGDGYCRAEAVVAVLLTKKSLARRVYATILNAGTNTDGCKEQGVTFPSGEVQEQLIRSLYEPAGLSPESLEYIEAHGTGTKVGDPQELNGIARALCPSRQEPLLIGSTKSNMGHPEPASGLAALAKVLLSLEHGLWAPNLHFRSPNTQIPALQDGRLQVVQQPLPVRGGNVCINSFGFGGSNVHVILRPNMRPPLAPTRHASLPRLLRASGRTPEAVHCLLEQGRRHSQDLAFVSMLNDIAAISPTAMPFRGYTVLGGKGGSQEVQLVAAGKRPLWFICSGMGAQWCGMGLSLMRLGSFRDSILRSDEAVKPLGLQVSELLLSTDEATFDDIIHAFVSLTAIQIALIDLLNSMGLRPDGIIGHSLGEVACGYADGCLSQEEAILAAYWRGQCIKETNIPPGTMAAVGLSWEECKQRCPPGVVPACHNSEDTVTISGPQAEVAAFVAELKREGVFAKEVRTGGMAFHSYFMDSIAPTLLQALKKVIREPRPRSARWLSTSIPEAQWQGSLARTFSAEYNVNNLVSPVLFQEALWHVPGDAVVLEIAPHALLQAVLKRGLKSSCTIVPLMKKDQRDNLEFFLSNVGKLHLLGFDVNPNGLLPPVEFPVPRGTPLISPHIKWDHSQTWDVPTAKDFPSGSSGSSASTVCNISISPESPDHYLADHCIDGRVLFPATGYLCLVWKTLARTLSQNMEQVPVAFEDVTLHQATVLPKTGTVPLEVRLLQASRTFEVSENGNLIVSGKVYQWEDPDTKLFDSRDGLDATDPMATFHLSQRDVYKELRLRGYDYGPHFQGILEANLEGNAGRLLWKNNWVTFLDAMLQTSILGLAQRSLRLPTRITSVRIDPATHQRRVYSLQGEAQAVNVLVNRCLNSTVAGGVLVSGLHASMAPRRQQEQFAPILEKFCFTPHTEEGLLAGDAALQEGLQLCRGLAQALQTKVAQQGLKMVVSGLDGAQAPQEPPKQGLPRLLAAACQLQLNGGLQLELGQLLAQQRPLLQDDPLLSGLLASPALKACVDTALENMPSLKMKVVEVLAGDGRLYSHIPALLNTQPMLQLEYTATDRHPQALEAVQAKLQQHGIAQGQWDPADHAPGSLGSADLLLCNCAVASLGDPAVAVGNMGAALKEGGFLLLHALLKGHPLGETVAFLTCPEPQRGQQSLLSQDQWESLFAGASLHLVALKKSFYGSVLFLCRRPVLWDSPVFLPVEDPSFQWVNSLKNILADSSQQPVWLTATSCPDSGVVGLVNCLRREPGGHRIRCVLVSNLSSTSSTPSLDPGSSELQKVLRGDLVMNVYRDGAWGAFRHFPLERGLPEEQTEHAFVNVLTRGDLSSIRWVCSPLRHTQLTGPGTHLCAVYYASLNFRDIMLATGKLSPDAIPGKWARHDCLLGMEFSGRDASGKRVMGLVPAEGLATSVLLSQDFLWEVPSSWTLEEAASVPVVYTTAYYSLVVRGRVQPGETVLIHSGSGGVGQAAIAIALSLGCRVFTTVGSAEKRAYLQARFPQLDDTSFANSRDTSFEQHVLRHTAGKGVDLVLNSLAEEKLQASVRCLAQHGRFLEIGKFDLSNNHLLGMAVFLKNVTFHGVLLDSLMDEGGNSWQEVAALLKAGIRDGVVQPLKCTVFPKDRVEDAFRYMAQGKHIGKVVVQVRREEPEAVLRETGPTLMAAVSKTYCPAHKSYVITGGLGGLGLELAQWLVLRGARKLVLTSRSGIRTGYQAKQVREWRRQGIQVLVSTSNASSLDGAQSLIDEATQLGPVGGVFNLAVVLRDAMLENQTPELFEDVVRPKYSGTVNLDRVTRAACPELDYFVAFSSVSCGRGNAGQTNYGFANSTMERVCEKRQHDGLPGLAIQWGAVGDVGIVLESMGSNDVVIGGTLPQRIASCLEVLDVFLNQPHPVLSSFVLAEKKATAHNDSSSRQDPMEAVAHILGIRDLATVNLDSSLADLGLDSLMGVEVRQMLEREHDLVMSMRDIRQLTLRKLQELSSKAGTANELAAPTPKEDTPAGQQAQLNLSTLLVNPEGPTLTRLNSVQSSERPLFLVHPIEGSITVFRSLASKLSIPTYGLQCTRAAPLDSIQSLAAYYIECIRQVQPEGPYRIAGYSYGACVAFEMCSQLQAAQQGPTPAHNSLFLFDGSHTYVLAYTQSYRAKLTPGCEAEAEAEAMCFFVQQFTDMEHNRVLEALLPLKSLEERVAATVDLITRSHAGLDPRELSFAARSFYHKLRAAEQYIPRATYHGNVTLLRTKTGSVYSEGLGADYNLSQVCDGKVSVHVIEGDHRTLLEGSGLETILSIIHSSLAEPRVSVREG

SEQ ID NO: 10 - protein, 2512 aa, Sus scrofa
MEEVVIAGMSGKLPESENLEEFWANLIGGVDMVTADDRRWKAGLYGLPRRMGKLKDLSRFDASFFGVHSKQANTMDPQLRMLLEVTYEAIVDGGINPASLRGTSTGVWVGVSSSDASEALSRDPETLVGYSMIGCQRAMMANRLSFFFDFKGPSITIDTACSSSLLALQSAYQAIRGGECSAAVVGGLNVLLKPNSSLQFMKLGMLSQDGTCRSFDAEGTGYCRAEAVVAVLLTKKSLARRVYATILNAGTNTDGSKEQGVTFPSGDVQEQLIRSLYAPAGPDPESLEYIEAHGTGTKVGDPQELNGIVNALCATRREPLLIGSTKSNMGHPEPASGVAALIKVLLSLEHGVWAPNLHYHTPNPEIPALQDGRLQVVDRPLPIRGGNVGINSFGFGGSNVHVILQPNSRPAPPPAQHAALPRLLQASGRTLEAVQTLLEQGLRHSRDLAFVGMLNEIAAVSPVAMPFRGYAVLGGEAGSQEVQQVPGSKRPVWFICSGMGAQWQGMGLSLMRLDRFRDSILRSDQALKPLGLRVSDLLLSTDEAVLDDIVSSFVSLTSIQIALIDLLTSLGLQPDGIIGHSLGEVACGYADGCLTQEEAVLSSYWRGYCIKEANVLPGAMAAVGLSWEECKQRCPPGIVPACHNSKDTVTISGPQAAMSEFLQQLKREDVFVKEVRTGGIAFHSYFMESIAPTLLRQLRKVILDPKPRSKRWLSTSIPEAQWQGSLARTFSAEYSVNNLVSPVLFQEALQHVPAHAVVVEIAPHALLQAVLKRSLESSCTIIPLMKKDHRDNLEFFLSNVGRLHLAGVSVNPNGLFPPVEFPAPRGTPLISPHXKWDHSQAWDVPSAADFPSGSSCSSVAVYKFDVSPESPDHYLVDHCIDGRVLFPGTGYLWLTWKTLARALSQNLEETPVVFEDVTLHQATILPKTGTVSLEVRLLEASHAFEVSDSNGSLIASGKVYQWESPDPKLFDTRAAVDPADSTAEFRLSQGDVYKDLRLRGYDYGPFFQLVLESDLEGNRGRLQWNDSWVSFLDAMLHMSILAPGQLGLYLPTRFTSIRIDPVTHRQKLYTLQDTTQAADVVVDRNLNTVVAGGALFLGAHSSVAPRRPQEHLKPILEKFCFTPHVESGCLAGNTALQEELQLCRGLAQALQTKVAQQGLKMVVPGLDGAQAPREAPQQSLPRLLAAACQLQLNGNLQLELGQVLAQERPLLCDDPLLSGLLDAPALKACVDTALENMASPKMKVVEVLAGDGQLYSRIPALLNTQPVMDLDYTATDRNPQALEAAQAKLEQLHVTQGQWDPANPAPGSLGKADLLVCNCALATLGDPAVAVGNMAATLKEGGFLLLHTLLAGHPLGEMVGFLTSPEQGGRHLLSQDQWESLFAGASLHLVALKRSFYGSVLFLCRQQTPQDSPVFLSVEDTSFRWVDSLKDILADASSRPVWLMAVGCSTSGVVGMVNCLRKEPGGHRIRCVLVSNLSSTSPAPEMHPSSSELQKVLQGDLVMNVYRDGAWGAFRHFPLEQDRPEKQTEHAFVNVLSRGDLSSIRWVCSPLHYALPASCQDRLCSVYYTSLNFRDVMLATGKLSPDSIPGKWLTRDCMLGMEFSGRDASGRRVMGMVPAEGLATSVLLLQHATWEVPSTWTLEEAASVPIVYTTAYYSLVVRGRMQPGESVLIHSGSGGVGQAAIAIALSRGCRVFTTVGSAEKRAYLQARFPQLDETCFANSRDTSFEQHVLRHTAGKGVDLVLNSLAEEKLQASVRCLAQHGRFLEIGKFDLSNNHALGMAVFLKNVTFHGILLDSLFEEGGATWQEVSELLKAGIQEGVVQPLKCTVFPRTKVEAAFRYMAQGKHIGKVVIQVREEEQGPAPRGLPPIALTGLSKTFCPPHKSYVITGGLGGFGLQLAQWLRLRGAQKLVLTSRSGIRTGYQARQVREWRRQGVQVLVSTSNASSLDGARSLITEATQLGPVGGVFNLAMVLRDAVLENQTPEFFQDVSKPKYSGTANLDRVTREACPELDYFVIFSSVSCGRGNAGQANYGFANSAMERICEKRRHDGLPGLAVQWGAIGDVGVVLETMGTNDTVIGGTLPQRIASCLEVLDLFLSQPHPVLSSFVLAEKKAAAPRDGSSQKDLVKAVAHILGIRDVASINPDSTLVDLGLDSLMGVEVRQILEREHDLVLSMREVRQLSLRKLQELSSKTSTDADPATPTSHEDSPVRQQATLNLSTLLVNPEGPTLTRLNSVQSAERPLFLVHPIEGSITVFHGLAAKLSIPTYGLQCTGAAPLDSIQSLASYYIECIRQVQPEGPYRIAGYSYGACVAFEMCSQLQAQQSATPGNHSLFLFDGSHTFVLAYTQSVRAKMTPGCEAEAEAKAMYFFVQQFTDMEQGKVLEALIPLQGLEARVAATVDLITQSHAGLDRHALSFAARSFYQKLRAAENYWPQATYHGNVTLLRAKTGGAYGEDLGADYNLSQVCDGKVSVHVIEGDHRTLLEGSGLESILSIIHSCLAEPRVSVREG

SEQ ID NO: 11 - protein, 2507 aa, Cuculus canorus
MEEVVIAGMAGKLPESANLQEFWENLMNGVDMVTEDDRRWKPGIYGLPRRNGKLKDLTKFDASFFGVHPKQAETMDPQLRMLLEVSYEAILDAGINPATLRGTDTGVWIGTGGSEAGEALSQDPEELSGYSMTGCQRAMLANRLSYFYDIKGPSVTIDTACSSSLVAMENAFKAIRAGQCHTALVGGCSLLLKPNTSVQFMKLGLLSPNGVCKSFDASGDGYCRSEAIVVLFLTKRSLAKRIYATIVNAGINADGFKEQGVMFPSGEMQQKLASSLLKESGIRPEEVEYVETHGTGTKIGDPQELNGITNVLCRCERAPLLIGSVKSNMGHSEPASGVAALAKVTGGLRRKNGRGQQCVNIPALHDGSMQVVCKPTPVKGGFVSINSFGFGGANANVILKPNMKKQQPVETSNVPRLIQFCGRTQEAVEVLIEESKKHAECIPFISLLSDISGIPASSMPYRGYTILGSESDIREVQQVQSTGRPLWYICSGMGTQWKGMGLSLMKLDLFRQSVLRSDEALKHTGLKVSELLLNEDENTFDDTVHAFVGLAAIQIAQIDILKAAGLEPDGIVGHSVGELACGYADNSLSHEEAILAAYWRGRCVKDAKLPPGGMAAVGLSWEECKQICPPNVVPACHNSEDTVTVSGPLGAVSEFVAKLKKDGVFAKEVRTSGVAFHSHYMASIAPVLLSALKKVIPHPKPRSPRWISTSIPESQWQSDLARYSSAEYHVNNLVNPVLFHEGLSHVPGNALVVEIAPHALLQAILKRSLKPTCIILPLMKKEHKNNLEFFLTQLGKFHMSGVNFNGNNLFPRVEYPVPVETPLISPHIKWDHSQEWYVPQAKDFPSGSKGTSSASVYNIDISPESPDHYLVDHCIDGRVLFPATGYLVLAWRTLARSLGMTIEKMPVTFEDVTIHQATILPKKGAVQLEVRLMPVSHCFEVSGNGNLAVSGKIFVLENDAAKKLDNQPVDCGTQVDVSSKVNLLKEDIYQELHLRGYNYGPNFQGVLEWNSEGTKSKVLWNGNWVTFLDTLLHVVILVESGRSLRLPTRIRTMSIDPVLHQERVCQYKDDVKAIDVVTDRCLASVRAGGVQFSGLHASVAPRRQQERIPPTLEKFCFVPYTEKNCLSSSVHLHDYLKQCKDLIQNLVNKVVVHGIKLVIPGLETADPDAEPLSVQKGLQHILAEMRKLEPNGNLHSELQQIVTREKMHLRDDPLLNGLLDSSELKTCLDVAVENVSSRRMKIIEVLAGSGQLFSRVKSVLTTQPLLQPDYIATDRSLEALSAAETELQDAGVVFSQWDPSSPPAGNLTDADLVVYNCSSVTENTPEIFSNLAAAVKEEGFVLIHTLLRGETVGEFVSFLTSPDLQQKHQFLSEAQWDSLFNSASLNLVAMKKSFFGSVIFLCRRRAPAKTPIFLPVDENDFKWVESLKGILAEQSEQPVWLTATSCGISGILGMVNCLRLEAEGHRIRCLFVSNLKPSSVVPPTSPSCPEMQNIVQKDLVMNVYRDGTWGSFRHLPLQQAQPQELTEYAYVNVLTRGDLSSLRWIASPLRHFQRTNPDVQLCKVYYSSLNFRDIMLATGKLPPDAIPGNWALQQCMLGMEFSGRDMSGRRVMGLLPAKGLATVVDCDKKFLWEVPKNWTLEEAASVPVVYATAYYALVVRGGMKKGESVLIHSGSGGVGQAAIAIALSMGCRVFATVGSTEKREYLQARFPQLDANSFASSRNTSFEQHIMRVTKGKGVNLVLNSLAEEKLQASLRCLAQHGRFLEIGKFDLSNNSQLGMALFLKNVAFHGILLDALFEDGNQDWNIVSELLMKGIKDGVVKPLRSTVFNKEEVEAAFRFMAQGKHIGKVMIKVQEEEKEYPLRRSEPVRISAISRTACPPTKSYILVGGLGGFGLELAQWLVERGAQKLVLTSRSGIRTGYQAKRVEEWKALGVQVLISTRDAATLEGAQQLIEEALRLGPIGGIFNLAVVLRDSMIENQTPELYLEVNKPKYSGTLHLDQVSRKKCPDLDYFVVFSSVSCGRGNAGQSNYGFANSTMERICEQRQHDGLPGLAIQWGAIGDVGVLVKTIGNKDVVVGGTVPQPISSCLEVLDVFLHQPHPVMSSFVLAEKVSVKSDGGSQRDLVEAVGNILGIRDMSTLNPDTSLADLGLDSLMGVEVRQTLERDYDIIMNMREIRLLTINKLRELSSMSGRTEEMKPSQMMKAGFPELPKLNLNNLLVNPEGPTITRLNDVQSTERPLFLIHPIEGSITFFHTLASRLHIPCYGFQCTKAAPLDSIQTLASYYIDCMKQIQPEGPYRIAGYSFGACVAFEMCSQLQAQQNASHTLNNLFLFDGSHSFVAAYTQSYRATLDEGDLAAVETEALSVFVQQFTGMEYNKLLEILLPLEDLAARVNATVDLITQVHTDINREELSFAATSYFYKLKAADQYVPASKYHGNVTLMRVKARSEYEEGLGTDYRLSEVCDGKISVHMVDGDHNTLLEDGVESIVGIIHSSLAEPRVSVREG

SEQ ID NO: 12 - protein, 2511 aa, Calypte anna
MEDVVIAGIAGKLPESENLQEFWENLLNGVDMVTEDDRRWKPGIYGLPRRNGKLKDISKFDASFFGVHPKQAHTMDPQLRLLLEVSYEAILDAGIDPATLRGTDTGVWVGASGSEAAEALSQDPEELLGYSMTGCQRGMFANRISYFYDLTGPSLTIDTACSSSLIALENAYKAIRHGQCSAALVGGVNLLLKPNTSVQFMKLGMLSPEGACKAFDASGNGYCRSEAVVIVLLTKRSMAKRIYATIVNAGTNTDGFKEQGVTFPSGEMQQQLISSLYRESGISPEEVEYVEAHGTGTKAGDPQELNSIVNVFCKCEREPLKIGSTKSNMGHPEPAAGLAALAKVTGGLRRKIGQGRKHNSVGLVCFDIPGLQDGSLEVICKPTPVKGGLVSINSFGFGGANAHVILRPNENRRQPPETCNIPRLVQVCGRTQEAVEVLIQESRKHGGCSPFVSLLSDISAMPVSSMPYRGYTLVGTESDIQEIQQVQASGRPLWYICSGMGTQWKGMGLSLMKLDLFRQSILRSDQALKNTGLKVSDLLLQADDNTFDETVHAFVGLAAIQIAQIDMLKAAGLQPDGILGHSVGELACGYADNCLSHEEAILAAYWRGRCVKEAKLPPGGMAAVGLTWEECKQQCPPNVVPACHNSEDTVTISGPLATVSEFVAKLKKAGVFAKEVRSAGVAFHSHYMASIAPVLLSALKKVIPHPKPRSARWISTSIPESQWQSDLAKYSSAEYHVNNLVSPVLFHEGLKHIPENAVVVEIAPHALLQAILKRTLKPTCTILPLMKKDHKNNLEFFLTQAGKIHLTGINVLGNNLFPPVEYPVPVGTPLISPYIKWDHSQGWDVPKAEDFPSGSKGSASASIYNIDVSPDSPDHYLVGHCIDGRVLYPATGYLVLAWRTLARSLGMVMEQTAVKFEDVTIHQATILPKNGSVQLEVRLMPASHSFEVSGNGNLAVSGKISLLENTALKPADFHTRAGMGLKPGLLKEDIYQELHLRGYNYGPTFQGVLECNSEASAAKVLWNGNWVTFLDTLLHVIILSDTGRSLRLPTRIRSVCVDPVLHQEMVCQYQDNVEVCDAVVDLCLDRLQAGGVQLDGLHASVAPRRQQERMTPTLEKFCFVPYTESDCLSSNAHLHDCLDHCKVLIQKMQAKLAVHGVKLVIPGLDTGSTAAKSSPIQKGLQHILTEICRLELNGNLRSELEQIVTREKMHFHDDPLLSGLLDSSELKSCLDVAVENMTSHRMKIIEALAGSGRLFSRVKSILNTQPLLQVDYIATDRVLETLSASETELQDAGVSSSQWDPSSLPSGNLTNADLVVYNCATNVLGNTTEILSNLAAAVKEGGFVLLHTLLKGETLGEIVSFLSSPDLQQKHKFLHETQWEDLFSKASLNLVAMKKSFFGSVIFLCRRQVPAKTPIFLPVDETHYKWVESLKEILADSSEQPVWLTATSCGNSGILGMVNCLRLESEGHRIRCVFISNLNPSSAVPPTSHSSLEMQKIVQGDLVMNVYRDGKWGSFRHLPLQQAQPQELTEYAYVNVLTRGDLSSLRWIVSPLQHFQANNPDIQLCKVYYASLNFRDIMLATGKLSPDAIPGNWVLQQCMLGMEFSGRDMAGRRVMGLLPAKGLATVVDCEKKFLWEVPKNWTLEEAASVPVVYATAYYALVVRGRMKKGESVLVHSGSGGVGQAAIAIALSMGCRVFTTVGSAEKREYLQARFPQLDANSFASSRDTAFEQHVLRVTNGKGVNLVLNSLAEEKLQASLRCLARHGRFLEIGKFDLSNNSQLGMALFLKNVAFHGILLDAIFEGGNQEWDIVSELLTKGIKDGVVKPLKSTVFKKEEVEAAFRFMAQGKHIGKVMIQIQEEEKEYSVRRSEPVKISAISRTSCPPSKSYIITGGLGGFGLELAQWLVERGAQKLILTSRSGIRTGYQARRVREWKALGIQVLVSTSDIGTLEGAQRLIEEALQLGPVGGIFNLAVVLRDAMIENQTPELFVEVNKPKYSGTLHLDWVTRKKCPDLDYFVVFSSVSCGRGNAGQSNYGFANSTMERICEQRHHDGLPGLAIQWGAIGDVGILLKTMGNKEVVVGGTIPQQISSCLEVLDTFLNQPHPVTSSFVLAEKVSVKAEGGSQRDLVEAVAHILGVRDVSSLNADSSLADLGLDSLMGVEVRQTLERDYDIVMTMREIRLLTINKLRELSSKSGTTEELKPSQVMKTGAGEPPKLDLNNLLVNPEGPTITRINDVQSTERPLFLVHPIEGSTAVFKTLASKLHMPCYGFQCTKVAPLDSIQSLATYYINCMKQIQPEGPYRIAGYSFGACVAFEMCSQLQAQHKGSHALNSLFLFDGSHSFVAAYTQRYRAKLSQGNEAALETEALCAFVQQFTGIEYNKLLEILLPLKDLEARVNAAADLITQVHTHINREALCFAATSFYHKLKAADKYIPESKYHGNVTLVRAKSHNEYEEGLGGDYRLSEVCDGKVSVHVVEGDHRTMLEGNGAESIIGIIHSSLAEPRVSVREG

SEQ ID NO: 13 - protein, 2513 aa, Anas platyrhynchos
MEDVVIAGIAGKLPESENLQEFWENLLNGVDMVTEDDRRWKPGMYGLPKRNGKLKDISKFDASFFGVHPKQAHTMDPQLRLLLEVSYEAILDGGINPATLRGTDTGVWVGASGSEAAEAFSQDPEQLLGYSMTGCQRAMFANRISYFFDFKGPSLTIDTACSSSLMALENAYKAIRNGQCSAAVVGGVNLLLKPHTSVQFMKLGMLSPDGACKAFDASGNGYCRSEAVVVVLLTKKSMAKRIYATIVNAGSNTDGFKEQGVTFPSGDMQRQLVSSLHRECGIKPGDIEYVETHGTGTKVGDPQEVNGIADVFCQCEREPLLIGSTKSNMGHPEPASGLAALAKVVLSLEHGLWAPNLHFSDPNPDIPALLNGSLKVVCEPTPTKGGLVSINSFGFGGANVHVILKPNEKKHQPPETCNLPRLVQVCGRTQEAVETLIQESKKQRGCGPFLRLLTDISAIPVSLMPYRGYTLVGTESDIGEVQQVQVSGRPLWYICSGMGTQWKGMGLSLMKLDVFRQSIMRSDEALKNTGLKVSDLLLQADDNTFDETVNAFVGVAAVQIAQIDMLKAAGLQPDGILGHSVGEVACGYADNSLSHEEAILAAYWRGRCVKEAKLPPGGMAAVGLTWEECKQRCPPNVVPACHNSEDTVTISGPLDSVNEFVAKLKKDGVFAKEVRSAGVAFHSYYMASIAPALLSALRKVIPHPKPRSARWISTSIPESQWQSDLARNSSAEYYVNNLVSPVLFHEGLKHIPENAVVVEIAPHALLQAILRRSLKPSCTILPLMKKDQKNNLEFFLTQAGKIHLTGINVLGNNMFPSVEYPVPVGTPLISPYIKWDHSQDWDVPKAEDFPSGSKGSASASVYNIDVSPDSPDHYLVGHCIDGRILYPATGYLVLAWRSLAGSLGMAMEQTAVMFEDVTIHQATILPKKGSVQLEVRIMPASHCFEVSGNGNLAVSGKINLLENDALKNFRNQLAAFQTHLDTSSKSGLLKEDVYQELHLRGYNYGPTFQGVLECNSEGSAGKVLWNGNWVTFLDTLLHMIVLAETGRSLRLPTRIRSVYIDPVLHPEHVCQYQDNVEALDVVVDHCLNSLKAGGVQINGLHASVAPRRQQERIPPTLEKYCFIPYIESNCLSSSAQLHAYLEHCKGLIKNLQAKVAVHGVKLIIHGLETAGAAAGSSPMQKGLQHILAEICHLELNGNLHSELEQIVTQEKMHFQDDPLLNGLLDSSELKACLDVALENMTSHRMKIVEALAGNGHLFSRVTSILNTQPLLHLDYIATDCTLEALSANETELQDAGISFSQWDPSNPPSGNLSNADLVVYNCSTNVLGNTTKIVSNLAAAVKEGGFVLLHTLLQGETLGEIVSFLTSPDLQQKHSFLSQAQWEGLFSKASLNMIAMKRSFFGSVIFLCRRQSPAKTPIFLPIDETHYKWVESLKEILADQSEQPVWLTATSCGNSGILGMVNCLRLEAEGHRVRCVFVSNLNPSSAVPSISLSSLEMQEIVQRDLVMNVYRDGKWGSFRHLPLQQGQPQELTEYAYVNALTRGDLSSLHWIVSPLQHFYTTNPDVQLCKVYYASLNFRDIMLATGKLSPDAIPGNWASQQCMLGMEFSGRDMAGRRVMGLVSAKGLATVVDCNKRFLWEVPKNWTLEEAASVPVVYATAYYALVVRGGMKKGESILIHSGSGGVGQAAIAIALSMGCRVFTTVGSAEKRQYLQARFPQLDANSFASSRNTTFEQHVLRVTNGKGVNLVLNSLAEEKLQASLRCLAQHGRFLEIGKFDLSNNSQLGMALFLKNVSFHGILLDSIFGESNEEWEVVSKLLTKGIENGVVKPLRSTVFNKDEVEAAFRFMAQGKHIGKVMIKVQEEEKQYPLRRSEPVKLSAISRTSCPPTKSYIITGGLGGFGLELAQWLIERGAQKLVLTSRSGIRTGYQAKCVREWKALGIQVLVSTSDIGTLEGTQLLIEEALRLGPVGGIFNLAVVLRDAMIENQTPELFWEVNKAKYSGTLHLDWVTRKKCPDLDYFVVFSSVSCGRGNAGQSNYGFANSAMERICEQRHHDGLPGLAIQWGAIGDVGILKTVGNTDVVIGGTIPQQISSCLEVLDTFLNQSHPVVSSFVLAEKVSVKSEGSNQRDLVEAVAHIIGVRDVSSLNADSTLADLGLDSLMGVEVRQTLERDYDIIMTMREIRLLTINKLRELSSKSGTAEELKPSQLLKTGPGEPPKLDLNNLLVNPEGPTITRLNDVQSTERPLFLVHPIEGSIAVFYTLASRLHMPCYGLQCTKAAPLDSIQSLASYYIDCMKQIQPEGPYRIAGYSFGACVAFEMCSQLQGQQNASHALNSLFLFDGSHSFVAAYTQSYRAKLAQGNEAALETEALCAFVQQFTGIEYNKLLEILLPLKDLEARVNAAADLITQIHKNINREALSFAAASFYHKLKAADKYIPESKYHGNVTLMRAKTHNEYEEGLGGDYRLSEVCDGKVSVHVIEGDHRTLLEGDGVESIIGIIHSSLAEPRVSVREG

SEQ ID NO: 14 - protein, 2512 aa, Gallus gallus
MEDVVIAGIAGKLPESENLQEFWENLLNGVDMVTEDDRRWKPGIYGLPKRNGKLKDIKKFDASFFGVHPKQAHTMDPQLRLLLEVSYEAILDGGINPTALRGTDTGVWVGASGSEALEALSQDPEELLGYSMTGCQRAMLANRISYFYDFTGPSLTIDTACSSSLMALENAYKAIRHGQCSAALVGGVNILLKPNTSVQFMKLGMLSPDGACKAFDVSGNGYCRSEAVVVVLLTKKSMAKRVYATIVNAGSNTDGFKEQGVTFPSGEMQQQLVGSLYRECGIKPGDVEYVEAHGTGTKVGDPQEVNGIVNVFCQCEREPLLIGSTKSNMGHPEPASGLAALAKVILSLEHGLWAPNLHFNDPNPDIPALHDGSLKVVCKPTPVKGGLVSINSFGFGGSNAHVILRPNEKKCQPQETCNLPRLVQVCGRTQEAVEILIEESRKHGGCSPFLSLLSDISAVPVSSMPYRGYTLVGTESDITEIQQVQASGRPLWYICSGMGTQWKGMGLSLMKLDLFRQSILRSDEALKSTGLKVSDLLLNADENTFDDTVHAFVGLAAIQIAQIDVLKAAGLQPDGILGHSVGELACGYADNSLSHEEAVLAAYWRGRCVKEAKLPPGGMAAVGLTWEECKQRCPPNVVPACHNSEDTVTVSGPLDSVSEFVTKLKKDGVFAKEVRRAGVAFHSYYMASIAPALLSALKKVIPHPKPRSARWISTSIPESQWQSDLARNSSAEYHVNNLVNPVLFHEGLKHIPENAVVVEIAPHALLQAILRRTLKPTCTILPLMKKDHKNNLEFFLTQTGKIHLTGINVLGNNLFPPVEYPVPVGTPLISPYIKWDHSQDWDVPKAEDFPSGSKGSASASVYNIDVSPDSPDHYLVGHCIDGRVLYPATGYLVLAWRTLARSLGMVMEQTAVMFEEVTIHQATILPKKGSTQLEVRIMPASHSFEVSGNGNLAVSGKISLLENDALKNFHNQLADFQSQANVTAKSGLLMEDVYQELHLRGYNYGPTFQGVLECNSEGSAGKILWNGNWVTFLDTLLHLIVLAETGRSLRLPTRIRSVYIDPVLHQEQVYQYQDNVEAFDVVVDRCLDSLKAGGVQINGLHASVAPRRQQERISPTLEKFSFVPYIESDCLSSSTQLHAYLEHCKGLIQKLQAKMALHGVKLVIHGLETKGAAAGSPPAQKGLQHILTEICRLELNGNPHSELEQIVTQEKMHLQDDPLLNGLLDSSELKTCLDVAKENTTSHRMKIVEALAGSGRLFSRVQSILNTQPLLQLDYIATDCTPETLSDNETELHDAGISFSQWDPSSLPSGNLTNADLAVCNCSTSVLGNTAEIISNLAAAVKEGGFVLLHTLLKEETLGEIVSFLTSPDLQQKHSFLSQAQWEELFSKASLNLVAMKRSFFGSVIFLCRRQSPAKAPILLPVDDTHYKWVDSLKEILADSSEQPLWLTATNCGNSGILGMVNCLRLEAEGHRIRCVFVSNLSPSSTVPATSLSSLEMQKIIERDLVMNVYRDGKWGSFRHLPLQQAQPQELTECAYVNVLTRGDLSSLRWIVSPLRHFQTTNPNVQLCKVYYASLNFWDIMLATGKLSPDAIPGNWTLQQCMLGMEFSGRDLAGRRVMGLLPAKGLATVVDCDKRFLWEVPENWTLEEAASVPVVYATAYYALVVRGGMKKGESVLIHSGSGGVGQAAIAIALSMGCRVFATVGSAEKREYLQARFPQLDANSFASSRNTTFQQHILRVTNGKGVSLVLNSLAEEKLQASLRCLAQHGRFLEIGKFDLSNNSQLGMALFLKNVAFHGILLDSIFEEGNQEWEVVSELLTKGIKDGVVKPLRTTVFGKEEVEAAFRFMAQGKHIGKVMIKIQEEEKQYPLRSEPVKLSAISRTSCPPTKSYIITGGLGGFGLELAQWLIERGAQKLVLTSRSGIRTGYQAKCVREWKALGIQVLVSTSDVGTLEGTQLLIEEALKLGPVGGIFNLAVVLKDAMIENQTPELFWEVNKPKYSGTLHLDWVTRKKCPDLDYFVVFSSVSCGRGNAGQSNYGFANSAMERICEQRHHDGLPGLAVQWGAIGDVGILKAMGNREVVIGGTVLQQISSCLEVLDMFLNQPHPVMSSFVLAEKVSVKSEGGSQRDLVEAVAHILGVRDVSSLNAESSLADLGLDSLMGVEVRQTLERDYDIVMTMREIRLLTINKLRELSSKTGTAEELKPSQVLKTGPGEPPKLDLNNLLVNPEGPTITRLNEVQSTERPLFLVHPIEGSIAVFYTLASKLHMPCYGLQCTKAAPLDSIQSLASYYIDCMKQIQPEGPYRIAGYSFGACVAFEMCSQLQAQQNASHALNSLFLFDGSHSFVAAYTQSYRAKLTQGNEAALETEALCAFVQQFTGIEYNKLLEILLPLEDLEARVNAAADLITQIHKNINREALSFAAASFYHKLKAADKYIPESKYHGNVTLMRAKTHNEYEEGLGGDYRLSEVCDGKVSVHIIEGDHRTLLEGDGVESIIGIIHGSLAEPRVSVREG

SEQ ID NO: 15 - protein, 2509 aa, Nestor notabilis
MEDVVIAGIAGKLPESENLQEFWENLLNGVDMVTEDDRRWKPGIYGLPKRNGKLKDISKFDASFFGVHPKQAHTMDPQLRLLLEVSYEAILDGGINPATLRGTDTGVWIGASGSEAAEALSQDPEKLLGYSMTGCQRAMLANRISYFYDFTGPSIAIDTACSSSLIALENAFKAIRHGQCSAALVGGVNLLLKPNTSVQFMKLGMLSSDGACKAFDASGSGYCRSEAVVVVLLTKRSMAKRIYATIVNAGSNTDGFKEQGVTFPSGEMQQRLVSSLYRECGIKLEEVEYVEAHGTGTKVGDPQEINGIVKMFHQCERAPLLIGSTKSNMGHPEPASGLAALAKVMGGLRRRIEGGREHNNIPALQDGTLEVVCKPTPVKGGLVGINSFGFGGANAHVILRPHKNKCQPLETCNTPRLVQICGRTQEAVETLIQESREHGGCSPFLSLLTDISAVPVSSMPYRGYTLVGTESDIKEVQHVQASGRPLWYICSGMGSQWKGMGLSLMKLDMFRQSILRSDEALKNTGLKVSDLLLRADENTFDETINAFVGLAAIQIAQIDLLKAAGLQPDGILGHSVGELACGYADNCLSQEEAILGAYWRGRCVKEAKLPPGAMAAVGLTWEECKQRCPPNVVPACHNSEDTVTVSGPLESVTEFVAKLKKDGVFAKEVRSAGVAYHSHYMASIAPVLLNALKKVIPHPKPRSARWISTSIPESQWQSDLARSCSAEYLVNNLVNPVLFHDGLKHVPENAVVVEIAPHALLQAILRRTLKPTCTILPLMKKDQKNNLEFFLTQTGKIHLTGINVLGNNLFPLVEYPVPVGTPLISPYIKWDHSQDWDVPKAEDFPAGSKGSASASVYSIDLSPDSPDHYLVGHCIDGRVLYPATGYLVLAWRTLARSLGMAMEQMAVTFEEVTIHQATILPKNGSVQLEVRLMPASHYFEVSGNGNLTVSGKIFLLENTALKNFHNQLVDFQTQADTSSKSGLLKEDIYQELHLRGYNYGPTFQGVLECNSEASTGKVLWNGNWVTFLDTLLHMMVLAKSGRSLRLPTRIRSVCIDPVLHQEKVCQYQDNVEALDVVVDPCLGSLKAGGVQIDGLHASVAPRRQQERIPPTLEKFCFVPYTESNCLSSSVHLRAYLEHCKDLIRNVQAKVAVHGVKLVIPGLKTAVAAAGSSPIQKGLQHILAEICRLELNGNLSSELEQIVTQEKMHFQDDPLLNGLLDSSELKTCLGVALENMTSHRMKIVEALAGSGCLFSRIKSILNAQPLLQVDYIATDRILKTLSDSETELQDAGVSISQWDPSCLPSGDLANADLVVYNCLTVLGNTTEIVSNLAAAVKEGGFFLLHTLLKGETFGEIVSFLTSPDLQQKHSFLSEAQWEGLFSKASLNVVAMKKSFFGSVIFLCRRQAPAKTPIFLPVDETHFAWVESLKEVLADPSEQPVWLTATSCGNSGILGMVNCLRLEAEGHRIRCVFVSNLNPSSAVPPTSLSSLEMQKIVQRDLVMNVYRDGKWGSFRHLPLQQAQSQELTEYAYVNVLTRGDLSSLHWIVSPLRHFHTTNPNVQLCKVYYASLNFRDIMLATGKLPPDAIPGNWVLQQCMLGMEFSGRDLAGRRVMGLLPAKGLATVVDCDKRFLWEVPKNWTLEEAASVPVVYATAYYALVVRGGMKKGESILIHSGSGGVGQAAIAIALSMGCRVFTTVGSTEKREYLQARFPQLDANSFASSRNTTFEQHILRLTNGKGVNLVLNSLAEEKLQASLRCLAQHGRFLEIGKFDLSNNSQLGMALFLKNVAFHGILLDAIFEENQAWEVVSELLKKGIKDGVVKPLRSTIFNKDEVEAAFRFMAQGKHIGKVMIKVQEEELESPLRRSDPVKISAISRTSCPPTKSYIITGGLGGFGLELAQWLVERGAQKLILTSRSGIRTGYQADRVRQWKALGVQVLVSTSDIATLEGTQLLIEEALQLGPVGGIFNLAVVLRDGMIENQTPELFCEVNKPKYSGTLHLDWVTRKKCPDLDYFVVFSSVSCGRGNAGQSNYGFANSTMERICEQRHHDGLPGLAIQWGAIGDVGILLKTMGDREIVIGGTLPQQISSCLEVLDIFLNQPHPVMSSFVLAEKVSVKTEGGSQQDLVAAVAHILGVRDVSSLNAESTLADLGLDSLMGVEVRQTLERDYDIVMTMREIRLLTVNKLRELSSKSRTAEGIVPARAQLMKTGPGKSPKLDLNNLLVNPEGPTITRLNDVQSTERPLFLVHPIEGSVAVFYTLSSRLHMPCYGLQCTKAAPLDSIQSLAAYYIDCMKQIQPEGPYRIAGYSFGACVAFEMCSQLQDQQNASHALNSLFLFDGSHSFVAAYTQSYRAKLAQGNEAALETEALCAFVQQFTGIEYNKLLEVLLPLKDLEARVNAAADLITQIHANINREALSFAAASFYHKLKAADKYIPESKYRGNVTLMRAKSHSEYEEGLGGDYRLSEVCDGKVSVHIIEGDHRTLLEGDGVESIIGIIHSSLAEPRVSVREG

SEQ ID NO: 16 - protein, 2516 aa, Podiceps cristatus
MEDVVIAGIAGKLPESENLQEFWENLLNGVDMVTEDDRRWKPGIYGLPKRNGKLKDISKFDASFFGVHPKQANTMDPQLRLLLEVSYEAILDAGINPTTLRGTNTGVWVGASGSEAAEAFSRDPEELLGYSMTGCQRAMLANRISYFYDLKGPSLVIDTACSSSLVALESAYKAIRNGRCSAALVGGANLLLKPNTSVQFMKLGLLSPDGTCKAFDASGNGYCRSEAVVVILLTKRSMAKRIYATIVNAGINTDGFKEQGVTFPSGEMQQQLISSLYKECNIKPEELEYIETHGTGTKVGDPQEINGIADLFCQLERPPLLIGSTKSNMGHPEPASGLAALAKVTGGLRRKIGGEGEHNGAWVFVNIPALQDGSLEVICKPTPVKGGLVGINSFGFGGANAHVILRPNEKKSQPLETCNMPRLVQFCGRTKEAVETLIQASRNHGACSPFVSLLSDISTLPVSSMPYRGYALVGTDDSDIKEVQQVQGSGRPLWYICSGMGTQWKGMGVDLMKLDLFRQSILRSDEALKSTGLKVSDLLLQADENTFDDTVHAFVGLAAIQIAQIDMLKAAGLQPDGILGHSVGELACGYADNSLSREEAILAAYWRGRCVKEAKLPPGGMAAVGLTWEECKQCCPPNVVPACHNSEDTVTISGPLDSVHEFVAKLKKDGVFAKEVRSAGVAFHSYYMASIAPVLLSALKKVIPHPKPRSARWISTSIPESQWQSDLARNSSAEYHVNNLVNPVLFHEGLKHVPENAVVVEIAPHALLQAILRRTLKPTCTILPLMKKDHKNNLEFFLTQTGKIHLTGINVLGNNLLPLVEYPVPVGTPLISPYIKWDHSQDWDVPKAEDFPSGSKGSASASVYNIDVSPDSPDHYLVGHCVDGRVLYPATGYLVLAWRTLARSLGMAMEQMAVMFEEVTIHQATILPKKGSIQLEVRLMPASHCFEVSGNGNLAVSGKISLLENTALKDFHNQIVDFQTRVDRSSKSGLLKEDIYQELHLRGYNYGPTFQGVLECNSEASMGKVLWNRNWVTFLDTLLHMIVLTETGRSLRLPTRIRSVCIDPVLHQEYVCQYQDNVEAFDVVVDRCLDSLRAGGVQINGLHASVAPRRQQERTPPTLEKFCFVPYTESNCLSSSVHLNAYLEHCKGLIRNLQAKVAVHGVKLVIPGLETSVAAAKSSPIQKGLQHILAEICHLELNGNLHSELEQIVTQEKMHLQDDPLLNGLLDSSELNTCLDVALENMTSHRIKIVEALAGSGHLFSRVKSILNTRPLLQVDYIATDCILETFSANETELQDAGVSFSQWDPSSLPSGNLTNADLVVYNYSRSVLGNITEILSNLVAAVKEGGFVLLHTLLKGGTLGDIVSFLTSPDLQQKHSFLSEEQWEGLFSKASLNLVAMKKSFFGSVIFLCRRQAPAKTPIFLPVDETHYKWVESLKEILANPSEQPVWLTATSCGNSGILGMVNCLRLEAEGHRIRCVFVTNLNPSSAVPPTSLSSLEMQKIVQRDLVMNVYRDGKWGSFRHLPLQQAQPQELTEYAYVNVLTRGDLSSLHWIVSPLQHFHATNPNVQLCKVYYASLNFRDIMLATGKLSPDAIPGNWALQQCMLGMEFSGRDLAGRRVMGLLPAKGLATVVDCDKKFLWEVPKNWTLEEAASVPVVYATAYYALVVRGGMKKGESILIHSGSGGVGQAAIAIALSMGCRVFATVGSTEKREYLQARFPQLDANSFASSRNTTFEQHILRVTNGKGVNLVLNSLAEEKLQASLRCLARHGRFLEIGKFDLSNNSQLGMALFLKNVSFHGILLDAVFEDGNEEWEVVSELLKKGIKDGVVKPLRSTVFNKEEVEAAFRFMAQGKHIGKVMIKVQEEEKEYLLRKSEPVKVSAISRTSCPPTKVYIITGGLGGFGLELAQWLVERGAQKLILTSRSGIRTGYQAKCVGDWKALGIQVLVSTSDIATLEGTQLLIEEALQLGPVGGIFNLAVVLRDSMIENQTPESFWEVNKPKYSGTLHLDWVTRKKCPDLDYFVVFSSVSCGKGNAGQSNYGFANSTMERICEQRHHDGLPGLAIQWGAIGDVGILLKTIGNKDVVIGGTVPQQISSCLEVLDIFLNQPHPVMSSFVLAEKVSVKPQEGSQRDLVEAVAHILGVRDVSTLNAESSLADLGLDSLMGVEVRQTLERDYDIVMTMREIRNLTINKLRELSSKSGTAEELKPSQLTKTGPGEPPKLDLNNLLVNPEGPTITRLNDVQSTERPLFLVHPIEGSIAVFSTLASRLHLPCYGLQCTKAAPLDSIQSLAAYYIDCMKQIQPEGPYRIAGYSFGACVAFEMCSQLQAQQNASHALNSLFLFDGSHSFVTAYTRSYRAKLTQGNEAALETEALCAFVQQFIGIEYNKLLEVLLPLKDLDARVNAAADLITRIHTNINHEALSFAAASFYHKLKAADKYIPESMYHGNVTLMRAKSYNEYEEGLGGDYRLSEVCDGKVSVHVIEGDHRTLLEGDGVESIIGIIHSSLAEPRVSVREG

SEQ ID NO: 17 - protein, 2518 aa, Balearica regulorum
  source 1..2518: note = Balearica regulorum gibbericeps
MEDVVIAGIAGKLPESENLQEFWENLLNGVDMVTEDDRRWKPGIYGLPKRNGKLKDISKFDASFFGVHPKQAHTMDPQLRLLLEVSYEAILDGGINPATLRGTDTGVWIGASGSEAGEALSQDPEELLGYSMTGCQRAMFANRISYIYDLTGPSITIDTACSSSLVALENAYKAIRHGRCSAALVGGVNLLLKPNTSVQFMKLGMLSPDGACKAFDASGNGYCRSEAVVVILLTKRSMAKRIYATIVNAGSNTDGFKEQGVTFPSGEMQQQLVSSLYRECGIKPGEVEYVEAHGTGTKAGDPQEVNGIVSVFCQCEREPLLIGSTKSNMGHPEPASGLAALAKVTGGLKKKIGEGTHAHPNVYVFLNVDIPALQDGSLEVVCKPTPVKGGIVSINSFGFGGANAHVILRPNENKRQPLETCNMPRLVQICGRTQEAVEILIQESRKHGGCSPFVSLLSDISAVPVSSMPYRGYTLVGTESDIKEVQQVQASGRPLWYICSGMGTQWKGMGLSLMKLDLFRQSILRSDEALKNTGLKVSDLLLQADENTFDDTVHAFVGLAAIQIAQIDMLKAAGLQPDGILGHSVGELACGYADNSLSHEEAILAAYWRGRCVKEAKLPPGGMAAVGLTWEECKQCCPPNVVPACHNSEDTVTVSGPLDSVNEFVAKLKKDGVFAKEVRSAGVAFHSYYMASIAPVLLSALKKVIPHPKPRSARWISTSIPESQWQSDLARNSSAEYHVNNLVNPVLFHEGLKHVPENAVVVEIAPHALLQAILRRTLKPTCTILPLMKKEHKNNLEFFLTQTGKIHLTGINVLGNNLFPLVEYPVPVGTPLISPYIKWDHSQDWDVPKAEDFPSGSKGSASASVYNIDVSPDSPDHYLLGHCIDGRVLYPAAGYLVLAWRTLARSLGMAMEQMAVTFEEVTIHQATILPKKGSVQLEVRLMPASHCFEVSGNGNLAVSGKISLLENTALKNFHNQAVDFQTQVDTSSKSGLLKEDVYQELHLRGYNYGPTFQGVLECNNEASTGKVVWNGNWVTFLDSLLHVIILAETGRSLRLPTRIRSVIIDPVLHQEQVYQYQDNVEAFNVTVDHCLNSLKAGGVQINGLHASAAPRRQQERNPPTLEKFCFVPYTESNCLSSSVHLHAYLGHCKDLIQNLQAKVAVHGVKLVIPGLETAVAAAESSPIQKGLQHILAAICHLELNGNLHSELEQIVTQEKMHFQDDPLLNGLLDSSELKTCLDVALENMTSHRMKIIEALAGSGHLFSRVKSVLNTQPLLQVDYIATDCSLEALSANETELQDAGVSLSQWDPSSLPSGNLTNADLVVYNYSTSVLGNTTEILSNLAAAVKEGGFVLLHTLLKGETLGEIVSFLTSPDLQQKHSFLSEAQWEGLFSKASLNLVAMKKSFFGSVIFLCRRQAPAKTPVFLPIDETHFKWVESLKEVLADPSEQPVWLTATSCGNSGILGMVNCLRLEAEGHRIRCVFVSNLNRSSAVPPMTLSSLEMQKIVQRDLVVNVYRDGKWGSFRHLPLQQAQPQELTEYAYVNVLTRGDLSSLRWIVSPLRHFHATNPNVQLCKVYYASLNFRDIMLATGKLSPDAIPGNWALQQCMLGMEFSGRDLAGRRVMGLLPAKGLATVVDCDKMFLWEVPKNWTLEEAASVPVVYATAYYALVVRGGMRKGESILIHSGSGGVGQAAIAIALSMGCRVFTTVGSTEKREYLQARFPQLDANSFASSRNTTFEQHILRVTNGKGVNLVLNSLAEEKLQASLRCLAQHGRFLEIGKFDLSNNSRLGMALFLKNVAFHGILLDAIFEDGNKEWEVVSELLKKGIKDGVVKPLRSTVFNKEEVEAAFRFMAQGKHIGKVMIKVQEEEKENPLRRSEPVKISAISRTLCPPTKSYIITGGLGGFGLELAQWLVERGAQKLILTSRSGIRTGYQAKRVREWKALGIQVLVSTSDIGTLEGAQLLIEEALQLGPVGGIFNLAVVLRDGMIENQTPELFWEVNKPKYSGTLHLDWVTRKKCSDLDYFVVFSSVSCGRGNAGQSNYGFANSTMERICEQRHHDGLPGLAIQWGAIGDVGILLKTMGNKEIVVGGTVPQQISSCLEVLDIFLNQPHPVMSSFVLAEKISLKTEGGSQRDLVEAVAHILGVRDVNSLNAESSLADLGLDSLMGVEVRQTLERDYDIVMTMREIRLLTINKLRELSSKSGTAEELKPSQLMKTGPGEPPKLDLNNLLVNPEGPTLTRLNDVQSTERPLFLVHPIEGSIAVFYTLASRLHVPCYGLQCTKAAPLDSIQSLATYYIDCMKQIQPEGPYRIAGYSFGACVAFEMCSQLQAQQNASHALNSLFLFDGSHSFVAAYTQSYRAKLTQGNEAALETEALCAFVQQFTGIEYNKLLEVLLPLEDLEARVNAAADLITQIHTNINREALSFAAASFYHKLKAADKYIPESKYHGNVTLMRAKSHNEYEEGLGGDYRLSEVCDGKVSVHIIEGDHRTLLEGDGVESIIGIIHSSLAEPRVSVREG

SEQ ID NO: 18 - protein, 2515 aa, Phaethon lepturus
MEDVVIAGIAGKLPESENLQEFWENLFNGVDMVTEDDRRWKPGIYGLPKRNGKLKDISKFDASFFGVHPKQAHTMDPQLRLLLEVSYEAILDGGINPATLRGTDTGVWVGASGSEAGEALSQDPEQLLGYSMTGCQRAMFANRISYFYDLTGPSITIDTACSSSLVALENAYKAIRHGQCCAALVGGVNLLLKPSTSVQFMKLGMLSPDGACKAFDVSGNGYCRSEAVVVVLLTKRSMAKRIYATIVNAGSNTDGFKEQGVTFPSGEMQQRLVSSLYRECGIRPGEVEYIETHGTGTKVGDPQEVNGIANVFCQCEREPLLIGSTKSNMGHPEPASGLAALAKVTGGLRRKILGGSTTVMRCSLRDIPALQDGSLEVVCKPTPVKGGLVSINSFGFGGANAHVILRPNEKKRQPLETCNTPRLVQICGRTQEAVEILIQESRRHGGCSPFVSLLSDISTVPVSFMPYRGYTLVGTESDIKEVQQVQASDRPLWYICSGMGTQWKGMGLSLMKLDLFRQSILRSDEALKNTGLKVSDLLLQADENTFDDTVHAFVGLAAIQIAQIDMLKAAGLQPDGILGHSVGELACGYADNSLSHEEAILAAYWRGRCVKEAKLPPGGMAAVGLTWEECKQCCPPNVVPACHNSEDTVTVSGPLDSVNEFVAKLKKDGVFAKEVRSAGVAFHSYYMASIAPVLLSALKKVIPHPKPRSARWISTSIPESQWQSDLARNSSAEYHVNNLVNPVLFHEGLKHIPENAVVVEIAPHALLQAILRRTLKPTCTILPLMKKEHKNNLEFFLTQTGKIHLTGINVLGNNLFPLVEYPVPVGTPLISPYIKWDHSQDWDVPKAEDFPAGSKGSASASVYNIDVSPDSPDHYLVGHCIDGRVLYPATGYLVLAWRTLARSLGTAMEQTAVMFEEVTIHQATILPKKGSVQLEVRLMPASHCFEVSGNGNLAVSGKISLLEHTAPKNFHNQPVDFQTQADMSSKSGLLKDDIYQELHLRGYNYGSTFQGVLECNSEASTGKVLWNGNWVTFLDTLLHVIILAETGRSLRLPTRIRSVCIDPVLHQEQVCQYRDNVEAFDVVVDRCLDSLKAGGVQINGLHASVAPRRQQERIPPTLEKFCFVPYNEHNCLSSSVHLHAYLERCKDLIQNLKAKVAVHGVKLVIPGLETTVAAAESSPIQNGLQHILAEICRLELNGNLHSELEQIVTQEKMHFQDDPLLNGLLDSSELKTCLDVALENMTSHRMKIVEALAGSGHLFSRVKSILNTQPLLQVDYIATDHILETLSANETELQDAGVLFSQWDPSSLPSGNLTNADLVVYNCSTSVSGNTIEILSNLAAAVKEGGFVLLHTLLKGETLGEIVSFLTSPDLQQKHSFLNEAQWEGLFSKASLNLVAMKKSFFGSVIFLCRRQAPAKTPVFLPIDETHYKWVESLKEVLADPSEQPVWLTATSCGNSGILGMVNCLRLEAEGHRIRCVFISNLNPSSAVPPTSLSSLEMQKIVQRDLVMNVYRDGKWGSFRHLPLQQEQPQELTEYAYVNVLTRGDLSSLRWIVSPLRHFHATNPNVQLCKVYYASLNFRDIMLATGKLSPDAIPGNWALQQCMLGMEFSGRDLAGRRVMGLLPAKGLATVVDCDKMFLWEVPKNWTLEEAASVPVVYATAYYALVVRGGMKKGESVLIHSGSGGVGQAAIAIALSMGCRVFATVGSTEKREYLQARFPQLDADSFASSRNTTFEQHILRVTNGKGVNLVLNSLAEEKLQASLRCLARHGRFLEIGKFDLSNNSQLGMSLFLKNVAFHGILLDAIFEQGNQEWEVVSELLKKGIKDGVVKPLRSTVFNKEEVEAAFRFMAQGKHIGKVMIKVQEEEKEYSLRRFETVKISAISRTSCPPTKSYIITGGLGGFGLELAQWLVERGAQKLILTSRSGIRTGYQAKRVREWKALGIQVLVSTSDIGTLEGTQLLIEEALQLGPVGGIFNLAVVLRDGMIENQTPEFFWEVNKPKYSGTLHLDWVTRKKCPDLDYFVVFSSVSCGRGNAGQSNYGFANSTMERICEQRHHDGLPGLAIQWGAIGDVGILLKTMGNREVVVGGTIPQQISSCLEVLDIFLNQPHPVMSSFVLAEKVSVKTEGGSQRDLVEAVAHILGVRDVSSLNAESSLADLGLDSLMGVEVRQTLERDYDIVMTMREIRLLTINKLRELSSKSGTAEDLKLSQLMKTGPGEPPKLDLNNLLVNPEGPTITRLNDVQSTERPLFLVHPIEGSIAVFYTLASRLHIPCYGLQCTKAAPLDSIQSLAAYYIDCMKQIQPEGPYRIAGYSFGACVAFEMCSQLQAQQNASHAFNSLFLFDGSHSFVAAYTQSYRAKLTQGNEAALETEALCAFVQQFTGIEYNKLVEVLLPLKDLEARVNAAADLITQIHTNINREALSFAAASFYHKLKAADKYIPESKYHGNVTLMRAKSHNEYEEGLGGDYRLSEVCDGKVSVHIIEGDHRTLLEGDGVESIIGIIHSSLAEPRVSVREG

SEQ ID NO: 19 - protein, 2140 aa, Phoenicopterus ruber
EVVCKPTPVKGGLVGINSFGFGGANAHVILRPNDNKSQPLKTCNMPRLVQICGRTQEAVEVLIQESRKHGGCSPFLSLLSDISTVPVSSMPYRGYTLVGTESDIKEVQQVQASGRPLWYICSGMGTQWKGMGLSLMKLDLFRQSILRSDEALKNTGLKVSDLLLQADENTFDDTVHAFVGLAAIQIAQIDLLKAAGLQPDGILGHSVGELACGYADNSLSHEEAILAAYWRGRCVKEAKLPPGGMAAVGLTWEECKQCCPPNVVPACHNSEDTVTVSGPLDSVREFVAKLKKDGVFAKEVRSAGVAFHSYYMASIAPVLLSALKKVIPHPKPRSARWISTSIPESQWQSDLARNSSAEYHVNNLVNPVLFQEGLKHIPENAVVVEIAPHALLQAILRRALKPTCTILPLMKKEHKNNLEFFLTQTGKIHLTGINVLGNNLFPLVEYPVPVGTPLISPYIKWDHSQDWDVPKAEDFPAGSQGSASASVYNIDVSPDSPDHYLVGHCIDGRVLYPATGYLVLAWRTLARSRGMAMEQMAVMFEEVTIHQATILPKKGSVQLEVRLMPASHCFEVSGNGNLAVSGKISLLEDTALKNFHNQPVDFQTQVDMSSKSGLLKEDIYQELHLRGYNYGPTFQGVLECNSEASTGKVLWNGNWVTFLDTLLHMIILTETGRSLRLPTRIRSVCIDPVLHQEHVCQYQDNIEAFDVVVDRCLDSLKAGGVQINGLHASVAPRRQQERIPPTLEKFCFVPYTESNCLSSSVHLNAYLEHCKDLIQNLQAKVAVHGVKLVIPGLETAVAAAESSPIQKGLQHILAEICRLELNGNLHSELEQIVTQEKMHLQDDPLLNGLLDSSELKTCLDVALENTTSHRIKIVEALAGSGHLFSRIKSILNTQPLLQVDYIATDRILETLSANETELQDAGVSFSQWDPSSLPSENLTNADLVVYNYSTSVLGNTTEILSNLAAAVKEGGFVLLHTLLKGETLGDIVSFLTSPDLQQKHSFLSEEQWEGLFRKASLNLVAMKKSFFGSVIFLCRRQAPAKTPIFLPIDETHYKWVESLKEILADPSEQPVWLTATSCGNSGILGMVNCLRLEAEGHRIRCVFVSNLNPSSAVPPTSLSSLEMQKIVQRDLVMNVYRDGKWGSFRHLPLQQAQPQELTEYAYVNALTRGDLSSLRWIVSPLRHFHATNPNVQLCKVYYASLNFRDIMLATGKLSPDAIPGNWALQQCMLGMEFSGRDLAGRRVMGLLPAKGLATVVDCDKKFLWEVPKNWTLEEAASVPVVYATAYYALVVRGGMKKGESILIHSGSGGVGQAAIAIALSMGCRVFATVGSTEKREYLQARFPQLDASSFASSRNTTFEQHILRVTNGKGVNLVLNSLAEEKLQASLRCLARHGRFLEIGKFDLSNNSQLGMALFLKNVAFHGILLDAIFEDGNEEWEVVSELLKKGIKDGVVKPLRSTVFNKEEVEAAFRFMAQGKHIGKVMIKVQEEEKEYLLRKSEPVTISAISQTSCPPSKSYIITGGLGGFGLELAQWLVERGAQKLILTSRSGIRTGYQAKCVRQWKALGIQVLVSTSDIGTLEGTQLLIEEALQLGPVGGIFNLAVVLRDGMIENQTPELFWEVNKPKYSGTLHLDWVTRKKCPDLDYFVVFSSVSCGRGNAGQSNYGFANSTMERICEQRHHDGLPGLAIQWGAIGDVGILLKTIGNKEVVIGGTVPQQISSCLEVLDIFLNQPHPVVSSFVRAEKVSVKTEGGGQQDLVEAVAHILGVRDTSSLNPESSLADLGLDSLMGVEVRQTLERDYDIVMTMREIRNLTIKKLRELSSKSGTAEELKPSQLMKTGPGEPPKLDLNNLLVNPEGPTITRLNDVQSTERPLFLVHPIEGSIAVFNTLASRLHMPCYGLQCTKAAPLDSIQSLAAYYIDCMKQIQPEGPYRIAGYSFGACVAFEMCSQLQAQQNASHALNSLFLFDGSHSFVAAYTQSYRAKLTQGNEAALETEALCAFVQQFTGIEYNKLLEVLLPLKDFEARVNAAADLITQIHTNINREALSFAAASFYHKLKAADKYIPESKYHGNVTLMRAKSYNEYEEGLGGDYRLSEVCDGKVSVHIIEGDHHTLLEGDGVESIIGIIHSSLAEPRVSVREG

SEQ ID NO: 20 - protein, 2419 aa, Ooceraea biroi
MPAQFESINNPMTRESMARNGVPYSIDSDIVITGISGRLPESSNIEEFKENLMKEMDMVTDDERRWPAGIYGLPLRTAKLKDLDNFDASFFGVHAKQAHVMDPQLRMMLEITYEAIVDAGINPSTIKGSRTGVFVGVSTSESDEYWTKDTEKVNGYGLIGCCRAMFANRVSFAFDFHGPSFVLDTACSSSMVAMHEAVTAMRAGECDAAIVGGMNLLLKPANSLQFHKLGMLSSDGKCKAFDATGKGYVRAEALVAIYLQKAKDARRVYATVVHTKTNMDGYKFQGITYPNGEMQNQLMREVYSETGINPADIVYVEAHGTGTKVGDPEEINSVDQLFCKDRKTPLLIGSVKSNMGHSEPCSGLCSIAKVLIAMESGMIPANLHFSTPNPDIPALMEGRIRVITKATPWNGGLVGINSFGFGGANAHVILRSNSKPKLSPVLDTAKLLPKLVAVSGRTEDAVYTLLDKAKEHRQDDEFLSLLHAMHNNDIPGHGFRGYEILGIDHTRELTEVASYNEKRPIWFVFSGMGTQWSGMGRELLGIEVFRRTLQRCADTLLPHGVDLMNIILNNTNETLENVIDTFVAIAAMQVALIDVLAAIDIYPDGIAGHSVGELGCAYADGAFTAEQTVLAAYWRGKSIVDSTLEPGAMAAVGLSWEDAQKMCPPNVSPACHNSMDSVTISGPTKDVLKFVEELKSKNIFAKLVRSSGIAFHSKYIASAGPKLRASLDKIIPNPKQRSAKWISSSIPEAAWGSPLAQVSSSAYHVNNLLSPVLFQEAIAHIPDNAITIEIAPHCLLQAILRRSLPSTVTNVSLHMRDHTNNLAFLLSNIGKLYMAGAQPNISKLYPPVSFPVGRGTPMIGPLVKWDHSQKWNVASFKKTSGQSGECIVQVDLSKETDAYIAGHQIDGRILFPATGYMLLVWKTLAKLRGTDFELLPVVFENLRFQRATIMPKEGAIKFSINIFEGTGEFEISEAGTVVVRGNIRVSEAIEKDQLKLPPPAVPPVKEEILPLNTKDVYKELKLRGYEYHGIFQGINSCDNYATAGELRWSNEWVSYMDTMLQFSILARKHKLMYIPSRLQYCAINPVLHKQFVEGLPQDGGLPVYYYKNVNIVKSGGIEFRGLNASVVARRQQTQAEPRHERYIFVPYENPHSLVEDPTRGKLHALTILTQIMYENMTALKLKIVEIADERAAEALLTPLVTEIVNNELSSVTVEVQVAAVSPGNYAEAFNHVDVNVSIVAQDANTAPPAQDVHLGVAVDVLSNKSYTILKNLSASLKPSGFILLEETAAHLDLETALKDTDLTLVSRQTDSIGKNYLLLKKLKKSGEPIVIQITEKNLSWVETLKAALKITYTGEQEVLLMSQGEELIGLAGLITCIRKETGGANVRYVFIQDKNSPKFGLSVPYYVNQLDKGLMANVLKGGQWGSYRHLQLDRQNNVSSLQVEHAYVNTLTRGDLGSLRWIEGPLSYYQPDNSSNTMLCSVYYAPLNFKDIMMATGKLPADALPGKMAAEECVLGIEYSGRDENGRRVMGIVEAKGLATTVLTDLDFLWEVPDKWTLEEAATIPVAYATSYYALFVRGQLKAGESVLIHAGSGGVGQAAIAIALRTGCTVFTTVGTLEKRKYLKKRFPQLIDSHIGNSRDTSFEQMILTETQGRGVDLVLNSLAEEKLQAGIRCLAMNGRFLEIGKYDLSNDNNVGMSMFLKNTTFHGVLVDALFYASSLEKKELMRLVSEGIKNGAVQPLPSTVFTEQQVEQGFRYMASGKHIGKVLLKIREEEPKKCVSPAPKTVAAVPRTYMNPEKSYVLIGGLGGFGLELANWMIARGAKFIVLVSRFGITTGYQSLCVRRWRENGVKVVISTMDITTLSGAERLIAQSNQLAPIGGIFNLAAVLRDALIDNQKEADFKAVMLPKVDGTRNLDVVSRKLCPSLDYFVVFSSISSGRGNIGQTNYGFANSAMERMMEERQANGLPGLAIQWGAIGDVGLIIEKMGNSSEIGSTLPQHISSCLATMDIFLQQPHAVLTSVISAEKHKPNTDSNRISLVEAIANILGIKDIKLVNLNNSLADLGMDSLMGTEIKQTLERNYDIALSPQDIRSLTFSKLQELSVTSTTTMKEQQPVAANASTATNSLANAIENNAADNMLLMQWPSNEVLPKEVLVRMKTKSANGPALFIVHAIEGSVNALETLASEFERPVWGLQCVEQAPHDSILELAEFYVKAIRKVQKKGPYHVAGYSFGSCVAIEMAMQLEFAGEKVILSLIDGSPAYIRQQTEMIGKVDTTQEDYIPSDACMKALAYFSIQFNKQLNFFQAYSILKESKSETDMFNKMLQVIGDIPFAQDDLKIAGYLLFKKLTAAMRYSPDKKFKGPVTLIKATDNFLHLTKDYDLSQICVQPARIDEVSGNHRSILLGESAKRIASLLRM

SEQ ID NO: 21 - protein, 2453 aa, Anopheles funestus
MPARFEEVTATDTRRGVPIDLAGGHYDVDAGVGGHAGHRPNIVDDICITGFSGRLPESSDIGEFTRNLLEGVDMVNDDDRRWPAGLYDLPTRIGKIKDEDLQHLDAEFFKIHQKQAECMDPQLRMLLECTHEAIIDAGINPQEIRGSRTGVYIGCSNSETEQHWCADPDLVNGYGLTGCARAMFANRISYTFDFKGPSYAVDTACSSSLFALSQAFADMKAGHCDAAIVAGCGLILKPTMSLQFKRLNMLSKDGMCKAFDESGNGYVRSDGCVVTFLQRASNSRRIYASVLNVRTNTDGFKEQGITYPIGEMQKRLIRETYEEIGLNPADVVYVEAHGTGTKVGDPQEVNAITDFFCKDRKTPLLIGSVKSNMGHSEPASGVCSIAKILIAMEQGVIPGNLHYKNPNPDLYGLLDGRLKVVDRNLPWNGGIIGLNSFGFGGANAHVIMKSNPKPKPISPKDDGFPKLMVASGRTTEAVEAFLDQATVSKDDEEFVGIVNEIHSRNIPLHNYRGYTVVAGDGQSQTVREVLEVTADDKRPVWFIYSGMGSQWASMAKDLMQLEVFHNSIYRCAEALRPEGVDLIDVLTKSDDTKFDNILNSFISIAAVQVALTDVLTHVGITPDGMVGHSVGELGCAYADGCFTPEQTVLAAYWRGRSILDTDLIAGQMAAVGLSWEECKQKLPKDVIPACHNSADSVTISGPVNSVGKVIADLNAQGIFAKGVKSSGIAFHSRYIADAAPKLRKSLDKIIPNPKNRTPRWISTSIPEESWPTPLAQQSSSAYHVNNLLSPVLFSEGLKHVPANAICIEIAPHGLLQAILKRALGKDATNLSLMKRDHANNMIFLLSNLGKLYAAGVQPQVQKLYRPITYPVGRGTPMLNSLVKWDHSINWFLARIGVENKSGETIIDVNLGKDEDAYLAGHTIDGRVLFPATGYLTLAWRTYAKMQGADIEKTPVVIENAVFHRATILPKDGSVKFGINFFDGTGAFEICEGGTLAVSGKLTIPEKIELEELPLNKLEADKSGLALNMSDVYKELRLRGYDYANMFRGVTRSDPRALTGELQWRDNWVSFMDTMLQFSILGKDLRELYLPTRIEKIVINPARHMELVNNLTQTGDDRTLPVYMYRDINVIKSGGVEMRGLRATLAPRRQGTQAPPTLEKYVFVPNNNEKELAEDNSEKARLRSITAAVHLVIENSSGALKIKVAEASFERSPENTMAGTVQAIIEGEPTLASDVAVVTNHQPDTLVQHYGESGVRVINKDAAAGPIEQNCHLAIGYDTFGRADPEAILCNLRDSIKSDGFVLLEESRSTFDARCRATVVKTGFTIISTQVCDKKVFVLLRPIVAELAQRKSIIITISERSFSWVEELKAALAKAEETATYVYIVCQGEELCGAQGLMNCVKNELGGKFARLFFIQDRKADKFSLTSTLYKEQLAKDLICNVLRPANGTPTAAWGCFRHLRLDNQSNAPSLPVEHAYINALTKGDLASLKWIESSLSRDRPDAAARNDRTELCTVYYAPINFRDVMLSSGKLGADALPGDLATQDCILGLEFAGRDSNGRRIMAMVQAKSLATTCVAQRNMIWEIPDNWTMEQASTVPCVYSTVYYALVMRGRMKRGESILIHAGSGGVGQAAISVALAAGVTVYTTVGSKEKREFLKRTFPQLTDRNIGNSRDCSFEQLVMRETQGRGVDLVLNSLAEEKLQASIRCLGLNGRFLEIGKFDLNNNSPLGMSVFLKNTSFHGILLDSVMEGDDDTIAEVVKLVADGIKSGAVRPLPTSVFTEQQVEQAFRFMASGKHIGKVVVRVREEEKAKIVKPSPKLINAIPRTYMHAEKVYILIGGLGGFGLELSNWLVSRGAKIIVLTSRSGVRTGYQSLMIRRWTERGVKVVIDTNDVTTLKGAQKLLTDAARHGPVGGVFNLAAVLRDGLLENSSEADFRAVCVPKVDGTKNLDVATRELCPDLDYFICFSSVSCGRGNQGQVNYGLANSAMERICEARHAAGLPATAIQWGAIGDTGLVLENLGDNDTVVGGTLPQRMPSCLQTMDLFMQQPSPVLASMVIAEKRKTDTGGVSLVGCIANILGLKDTKNVSDGATLADLGMDSLMGAEIKQTLERSFDLVLSAAEIRLLTFGKLRSFEKGGSGGDAGAASGAPAAAAAGAGGKRTDEHAIGDGTQVKFSADLMPKECLVRLESAVPAGSKARPVFAVHAIEGVITALIPLAQTLPVPVYGLQCVEAAPLDSLETLAAYYIKQIRTIQARGPYTIIGYSFGASIAYEMVVQLEKAGDACHLLLLDGSPRYVSWYTEAQKQRNANGEVVQAVDEAYALAYFAMVCGSLDYGRTAKELVEAKSWDDRVAKCAEMVHAKIPQYSRQLLATTARSFVGKIVASHMYKPASKIKATVKLVKPTENYAKLQGDYGLSDLCQQKVEIFTVQGDHRSMLIGDSMKQIASVLQQLF

SEQ ID NO: 22 - protein, 2469 aa, Anopheles darlingi
MPARFEEVTATDTRRGVPIDLAGHYDDHHHDTGSNIGNNHHQQQQHGRRPAIRDDICITGFSGRLPESSNIDEFRRNLFEGVDMVNDDDRRWPSGLYDLPTRIGKIKDEDLQHLDAEFFKIHQKQAECMDPQLRMLLECTHEAIVDAGINPQEIRGSRTGVYIGCSNSETEQHWCADPDLVNGYGLTGCARAMFANRLSFTFDFKGPSYAVDTACSSSLFALSQAFADMKAGHCDAAIVAGCGLILKPTMSLQFKRLNMLSKDGMCKAFDESGNGYVRSDGCVVTFLQRASDSRRVYASVLNVRTNTDGFKNQGITYPIGEMQKRLIRETYEEIGLNAADVVYVEAHGTGTKVGDPQEVNAITDYFCKDRKTPLLIGSVKSNMGHSEPASGVCSIAKILIAMEAGVLPGNLHYRNPNPDLYGLLDGRLKVVDRNMPWNGGIIGLNSFGFGGANAHVILKSNPKPKPISPRDDAFPKLVLASGRTTEAVEAFLDQTAISKDDEEFVGLVNEINSRNTPLHYHRGYTVVSGDGKPPVREVLEVSDEKRPLWFIYSGMGSQWASMARDLMQLEVFHSTIARCAEALRPEGIDLIDVLTKSDESRFDNILNSFISIAAVQVALTDVLTHVGIVPEGMVGHSVGELGCAYADGCFTPEQTVLAAYWRGRSILDTDLIAGQMAAVGLSWEDCKQKLPKDVIPACHNSSDSVTISGPVASVGKVIADLNAQGIFAKGVKSSGIAFHSRYIADAAPKLRKSLDKIIPNPKPRTQRWISTSIPEESWGTALAQQSSSAYHVNNLLSPVLFAEGLKHVPANAICIEIAPHGLLQAILKRALGKEATNLSLMKRDHDNNLIFLLSNLGKLYAAGAQPQVQKLYPPITYPVGRGTPMLNSLVKWDHSDKWFLARIGVENKSGETIIDVNLGKDEDAYLAGHTIDGRVLFPATGYLTLAWRTFAKMRGADLEKTPVVIENAVFHRATILPRDGSVKFGINFFDGTGAFEICEGGTLAVSGKLTIPEKIELEELPLAKLEADRSALPLNTSDIYKELRLRGYDYGGMFRGVTRSDSKALTGELQWRDNWVSFMDTMLQFSILGKDLRELYLPTRIEKIVINPARHLEIVSGLPVAKDGTDRTLPVYMYRDINVIKSGGVEMRGLRATLAPRRQGTQAAPTLEKYVFVPNSNEKELAENADKARLRSITSAVHLVIENSAGALKIKVVEASAERSPENTMAGTVQGIIEGEPTLASDVAIATTHQPDSLVQHYGESGVRVLNKDIAAGAIEQGCHLAIAYDVFGSGATADVLRNLRDTIKTEGFVLLEESRTGIDLSAKGAVRNALSKAGFLLVSEQVCDKKVFLLVRPILAEIAQRKSTIVTITEKNFSWLDSLKTALAKAEESSTYVYVVCQGEELCGAQGLLNCIKNEAGGKFARLFFIQDRSAEKFSLTSALYREQAAKDLICNVLRPANGSPACWGTFRHLRLDSQSNAPSLPVEHAYINALTKGDLASLKWIESSLSRDRPAGDDRTELCTVYYAPINFRDVMLSSGKLGADALPGDLATHDCVLGLEFAGRDSSGRRIMAMVQAKSLATTCVAQRNMIWSIPDSWTMEQASTVPCVYSTVYYALVMRGRMKRGESILIHAGSGGVGQAAISVALAAGVTVYTTVGSAEKRAFLKRTFPQLTDRHIGNSRDCSFEQLVMRETQGRGVDLVLNSLAEEKLQASVRCLGLNGRFLEIGKFDLNNNSPLGMSVFLKNTQFHGILLDSVMEGDDETIAEVVRLVADGIANGAVRPLPTSVFSETQVEQAFRFMASGKHIGKVVIRVRDEEKQKVLKPAPKLINAIPRTYMHAEKAYILIGGLGGFGLELSNWLVSRGAKILVLTSRSGIRSGYQALMVRRWTERGVKVVIDTNDVTTLKGAQKLLTEAARHGPVGGVFNLAAVLRDGLLENSSEADFKAVCVPKVDGSKNLDQATRELCPDLDYFVCFSSVSCGRGNIGQVNYGLANSAMERICEARHAAGLPATAIQWGAIGDTGLVLENLGDNDTVVGGTLPQRMPSCLQTMDLFMQQPCPVLASMVIAEKRKTETGGVSLVSCIANILGLKDTKNVSDASTLADLGMDSLMGAEIKQTLERSFDLVLSAAEIRLLTFGKLRSFEKGGITSDGAAGGDGAAADGGSGAGGAAAKSAADQQTAIGDGTQVMFSAELMPKECLVKLESAAPPSKSPARPVFVVHAIEGVITALIPLAKTLPVPVYGLQCVEAAPLESLVVLAGYYIQQIKTVQPRGPYTIVGYSFGASIAYEMVAQLEAAGEKCSLLLLDGSPRYVSWYTEAQKQRNANGEVVQAEDEAYALAYFAMVCGKLDYGKTAHELVSAKSWNERVAKCAEMVHAKAPQYSKQLLETTARSFVGKIVASHMYKPSSKINANVKLVKPTENYAKLQGDYGLSDLCKQKVEILTVKGDHRSMLTGESMKQIAAALHQLC

SEQ ID NO: 23 - protein, 2540 aa, Glossina austeni
MYISVDFKSNDQIFILLHGAKANKINPSQVNHNRQHTNNNSNNENKNDSQKSSNKGKSANRRRKRRQKNSQNSNFSENPQQNHQDDVAQIVVKDNPSTSFPFHFSSSNSNYDSSSFPLVNGRLHKDSIMPARFVENSEPSVPMNLENRYDHPSSNGVNSDIVITGISGRLPESTNIEEFRKNLFEGVDMVNDEPRRWSKGLYGLPERNGKIKEEDLENFDQTFFGIHQKQADGMDPQMRMLLECTYEAIIDAGLNPAEIRGTRTGVYVGASSADSENYQLSDPDRVDGYGLIGCARAMFPNRISFSFDLKGPSYCVDTACSSSLYALSQAFADMNSGKCDAAIVAGSNLCLRPTMSLQFKRLSMLSAEGKCKAFDESGSGYVRSDAVVVILLQRVSVAKRVYATILNARTNVDGHKEQGITFPNGQMQNQLMRETYGEINLDPAEVNYVEAHGTGTKVGDPQEVNSITDFFCKNRKSPLLVGSVKSNMGHSEPSSGLCSIAKVLLAMEQNVLPPNLHYKNPNPDLYGLLDGRLKVVDKPTPWEGGIVGINSFGFGGANAHVILKSNPKPKVITPTVGPPKLILCSGRTSDAVQEFLEDAEQHKDDDEYLTLINDIHSRPISGHYYRGFSVMDSKGALQKDVAEINPESRPIWFVYSGMGSQWASMAKDLMVFDTFKKTIHRCCEILRPEGLDLMEVLTRSTEKTFENILNSFVGIAAMQVALTDLLTSLNIVPDGIVGHSVGEVACAYADGCLSMEQTILAAYWRGKSILDTKLTKGKMAAVGLSWEEAHKRLPADCFPACHNSAENCTISGPEESIDAVCQKLTAEGVFARAVKSSGYAFHSKYIADAGPKLRKSLEKVIPNAKNRSPRWISSSIPEVAWNTAIAQQASAAYHVNNLLSPVLFHQALQHVPKNAICIEVAPTGLLQAILKRSLGNETTNLSLIKRDYENNPEFFLASIGKLYAAGAQPQIMTLSKPISYPVGRGTPMLGCKVGWDHSQKWHVPKFDKMTSSGETIIEVDLSKEEDAFLAGHTIDGRILFPATGYMTLAWMTYAKMRGHEFQKTPVVMENVVFHRATILNKEGVVKFGINFFDGTGAFEICEGGSLAVSGKISIPENVDNEQLPLDPLPVSTVAKELSTSDVYKELRLRGYDYAGIFRGITASDSLSSTGKLQWVDNWISFMDTMLQFSILSKNLRELYLPTRIEKAIINPDHHLKEIAKLTPEQQTKEGVPVYMYDDINVIKSGGIELRGMKASLAQKRPSNQNPPTLERYAFIPNENGVDLNENHEKAHFHALSVALRLLNENSSGALKIKGVELADGRNPDSLLAAKIVQVLEGEPSLTAEIAVATSNSNEEAISAALGPDAGVRVISKNILKEPVDQNNHFVFGVDVLSRPDTAVLVNSLASIKDNGFLIFEESAYGYRNTGRNLLTEFGLVVASEQSCGNSRVLVMARRPVDLKQRKSVVINVTEKNFDWLEELKAALAKAAENEQYVYIVCQGEEAFGAVGLMTCIRRENGGNFARLVFVQDGNAKPFSFNDAFYTKQLAKDLISNVLKNGLWGTYRHMKLETNAATLQVEHAYVNALVKGDLASLKWIESPRLTPNISNDFELCTVYYAPINFRDVMLSSGKLSADALPGDLAQQDCVLGLEFSGRDSKGRRIMAMVPAKSLATTCVAAKIMTWQIPDKWSMEEASTVPCVYSTVYYALMVRGQMKKGEKILIHAGSGGVGQAAISVALHHGLTVFTTVGSKEKREFLKKRFPQLKDNHIGNSRDTSFEQMIMRETQGRGVDLVLNSLAEEKLQASVRCLGLNGRFLEIGKFDLSNNSPLGMSVFLKNTSFHGILLDSVMEGEEAMQKQVVDLVAEGIKNGAVRPLPTSVFNDQQVEAAFRFMASGKHIGKVVVKIRDEEPGSKAIKPPTHLVNAIPRTYMHPEKSYVLIGGLGGFGLELTNWLVFRGAKHIVLNSRSGLRTGYQALMVRRWQEKGVKVLVDTSDVTNASGCKQLLTNANKLATVGGIFSLAAVLRDDILENQTAKDFKTVCDPKVTATKLLDQCSRSLCTSLDHFVCFSSVSCGRGNIGQSNYGLANSAMERICEARQASGFPGLAIQWGAIGDTGLVIETLGDNDTVIGGTLPQRMNSCLQTIDLFLQQPHPVLASMVVAEKRKSDQSGGVSLIASVANILGIRNIKNIPEKSSLADLGMDSLMGAEIKQTLERNFDIVLSAQEIRQLTFGALTQMDSGPARAESATSPQATSPSAFGDGTQDVFSSELMPTETIVRLKSKAPADSNKRPLFIASPIEGFADPLKNLAELLDCPVYGLQCTANADLDTIQSLASFYLKEVRKIQAKGPYVIAGYSFGAAVAFEMVINLQSHDIVSNYIALDGAPKYVSWNTSSFKDRRSMDDGDNYDYGLAYFAMVVANMDYAFVVKMLLDKPTWQEKLAKCAEMVAQEIKKPIDLIKQAGEIFYKKLSAGHNYKATTKITCPVTLVKPSENYVQLEEDYGFNEICQKPVKVFTVEGNHRTFLVEEASLKTIESELNRLTA

SEQ ID NO: 24 - protein, 2540 aa, Drosophila melanogaster
MPLQLNLLQAVDQPHPVAFKPNNCSTHQPQHSPSTQNNGKSARANRRRRRRRNKQQQNSQQPDAFRDTDAQLTPSTSSSTPHSAPNDRQDHLNSQFNPESINMPARFAEEVITAEPAQRAAPQLDLGGGHYVPRQQHLNDEIAITGFSGRLPESSTIEEFKQNLFDGVDMVNDDPRRWERGLYGLPDRIGKLKDSDLENFDQQFFGVHQKQAECMDPLLRMLLELTHEAIIDAGLNPSDLRGSRTGVYIGVSNSETEQHWCSDADRVNGYGLTGCARAMFANRISFTFDFKGPSYSIDTACSSSLYALEQAFSDMREGKVDNALVAGAGLILKPTMSLQFKRLNMLSPDGSCKAFDESGNGYVRSDGCVVLLLQRTSAARRVYASILNVRTNTDGFKEQGITYPIGKMQNRLIRETYEEIGLNPADVVYVEAHGTGTKVGDPQEVNSITDFFCKDRTTPLLIGSVKSNMGHSEPASGVCSVAKILIAMEEGVIPGNLHYNKPNPDLYGLVDGRLKVVDRNLPWNGGIIGLNSFGFGGANAHVILKSNPKPKALTPKDGALKVVLASGRTFEAVEQLLESASTNADDDEYLQLINEIHSKAIPNHFFRGYGVVSSKGTHQREVIESNDDKRPIWYIYSGMGSQWASMAKDLMKIEAFAKTIQRCADVLKPEGVDLIDVLTRSTDKSFENILNSFISIAAMQVALTDLLSSLGIHPDGIVGHSVGELGCAYADGCFTPEQTVLAAYWRGKSILDTQLAKGKMAAVGLSWEDAHSRVPSDCFPVCHNSEDNCTISGPEASIEALVAKLNAEGVFAKAVNSSGYAFHSKYIAEAGPKLRKSLEKIIPNAKNRTARWISTSIPESAWNTPVAKQSSAAYHVNNLLSPVLFHEALQHVPKNAISVEIAPHGLLQAILKRALGPDATNLSLVKRGHENNVEFFLTNVGKLFAAGAQPQVLTLVRPISYPVGRGTPMLNSKVGWDHTQKWLVAKFGKETSSGETIVEVDLSKEDDAFLAGHTIDGRILFPATGYMTLAWQTFAKMQGSEFHKTPVVMENLVFHRATILNKNAVVKFGINFFDGTGAFEICESGSLAVSGKITIPESIDNEELPLEEQTPSAVAKELGTNDVYKELRLRGYDYGGIFRGIVRSDTVASTGKLQWVDNWISFMDTMLQFSILSKNLRELYLPTRIERAVINPAKHFELLSALTKEEQVETGLPVQWYSDINVIKSAGVELRGLKANLAQRRPGTQAPPTLERYQFVPNINTTDLNENSEKARLHALDVAIQVIIENSSGAVKLKGVELANGRNPDVLVANRLLQIIEGEPVLTGDVAVVTSNNNEETITAALGDSGVRVVSKDVLKEPVEQNCHFVFGIDVLSRPDTKTLENSIASIRENGFLILEETLPTYTKTGRALLTKFGFVAVQEQSLGATRVLVLARKAVDLKTRKSVVVVATEQNFNWVDDLKAALATAATEEQYVYVVCQGEELFGAVGLMTCIKNENGGKLARLVFVQDAKAEKFSLTSTLYRQQLEKDLISNVLKNGAWGTFRHLKLETQQATLQVEHAYVNALVKGDLASLKWIEAAQADTAATVDKNLETCTVYYAPINFRDVMLTSGKLAADALPGDLAEQDCVLGLEFAGRDTQGRRVMAMVPAKSLATTCVASKRMMWQIPEKWTMEEASTVPCVYSTVYYALVVRGQMKKGEKILIHAGSGGVGQAAISVALAHGLTVFTTVGSKEKREFLLKRFPKLQERNIGNSRDTSFEQLVLRETKGRGVDLVLNSLSEEKLQASIRCLGLNGRFLEIGKFDLSNNSPLGMSVFLKNTSFHGILLDSVMEGEEEMQNQVVSLVAEGIKTGAVVPLPTSVFNDQQVEQAFRFMASGKHIGKVVIKVRDEEAGKKALQPKPRLINAIPRTYMHPEKSYILVGGLGGFGLELTNWLVTRGARYIVLTSRSGVKTGYQGLMIRRWQERGVKVVIDTSDVTTAAGAKKLLENSNKLALVGGIFNLAAVLRDALIEDQTAKDFKTVADPKVTATKYLDQFSRDICTELDYFICFSSVSCGRGNIGQTNYGLANSAMERICEQRQVSGFPGTAIQWGAIGDTGLVLENLGDNDTVIGGTLPQRMPSCLQTIDLFLQQPHPVVASMVVAEKRKSDQSAGVSLIATIANILGLRDTKNIQDGASLADLGMDSLMSAEIKQTLERNFDIVLSAQEIRQLTFGALKAMDGGADVKPAAAAPAAAAGVPEANITSGGSSRTASPMGDGTQVVFTTSLIPTEAIVQLDTKAPANSKQSPIFFISPIEGFASALEPLAKRLEVPAYGLQYTEAVPSDSLESAAKFFIKQLRTVQPKGPYKLAGYSFGCLLTYVMAGILEETNEVANVIMLDGAPSYVNWYTSSFKQRYTDGTNADNDNQSYGLAYFGIVLANIDYKALVRLLIVIPTWEEKLERFAELMSNEITQPVETIKKSATLFYKKLELADGYQPTLKLKTNVTLVKPTDNSAKLDEDYRLKEVCTKPVEVHTVEGNHRTFLIEDQSLKTIQSILKRLFN

SEQ ID NO: 25 - protein, 2574 aa, Brugia malayi
MNSSGEVPFWRDQEEIVITGISGRFPRCENVQEFGDLLLAGEDLVTEDSLRWPPGVFDLPKRHGKLKDLKKFDAQYFGVTPKQANYLDPQVRKLLEVTLEAIIDAGLNPTELRGSRTGVFVGCSASETGGVLTQDPETVTGYTLTGCVRSMFSNRLSFTFDLRGPSFSVDTACSSSLCALQLAVDAIRQEQCDAAIVAGAHLTLTPTAALQFLRLGMLSDKGSCRSFDASGDGYCRTEAIAAILLQRQSAARRIYATVVHAKSNTDGYKEQGITFPSGERQAALLEEVYREAGVDPNTVTYVESHGTGTKVGDPQEANAICQVFCQNRNSALLIGSVKSNMGHAEPASGLCSIAKVLIAMERGFIPPNLHYNEPNPYIPGLTDGRLQVVTEKTPFQRGLVGINSFGFGGSNTHIILRPANHSERKPAPTTFMKIIPYSGRTAEAVNNILDCVLAHPENAYLQQLLANQANLPAKDTPYRGYVIINQLPPLRDVQKIMITEPKQIYFIYSGMGSQWAGMVRQLMSIPAFDESLRSSSDAIVDFGVNVYEMLQSDDPSFYKNNTLNCMLAITAIQIALTDVLFLLGVMPDGIIGHSTGEMCCGYADGGLTREQTMQLAYHRGHTIMNANIKGGMAAVGLSWEEAGKRCPEGVIPACHNAADSVTISGDAEKIKEFVEELKKEDIFGKLVDSSGIPFHSPAMLKVKDKMLKAMRTSVPNPKPRSSRWISTSIPESNWENELAQMCSADYHTNNAVSPVLFYEALQKIPANAVTIEIAPHCLMHSILRRSLQKTCTNVGLINMKEKDRELESFLQALGKIYQTGITIHIEALYPAIQYPVPIGTPMISPMWRWDHSQDWPVVDGKTLSAAGGRQLPASYCYTVDPFASDSKETFLLDHIIDGRVLYPFTGHMVLAWKTIAKLNGVDFLKTPVILEEIRVYSATIVTKPIRLDVIVTPGNGYFEILDGDQLAASGYIRIVDEDVPFYYKSIQEIQTSEIAERIELDTEDAYKEFLLRGYEYGQAFRGIYRACNSGERGMLYWTGNWVTFLDSLLQTALLAERADSLRLPTRVRYLRIDPVKHMEHIQERDGIQVIELRNDVATNGCIAGGVECCDLTAHTVARRLQSSGQLYYEKIYFTKHFDMKAFDEFPQIREELNAYRDFLRSLLANGLAKWEVNGCLKELTNGALLSGAVRKFTKSPVATVFDEIFAIEIGNNPKDFENKVAEKMQSMLKIFNVDRLWSAAIVHDRILKTIQDTCIENSTGHNCKACALEFNSTEQLKFCVDAVNSHPLLEVEWLCVGPKVDDMDESTLVQLGVKKVTTVLDEKQFVPSAEIKNCDIIILDKILSQKKDVVRYLSRCKEMLRDDGFIILVETTSDYEIALAIQGLNAETISISDSGRIYGAYFTHDQLLKLFEECDFRLCNYQSDPSMMTTMYAIRKIPSQPREPIVIDVDDIKEFTWIEPLQKAIEERLNEPDYKTIWLTSTTVRNNGLLGLALCFNEENLKSNRFRTLIDMSVKKENRTGPAQIGMEHESVKQLVKLDLHANNYRDGVWGSMRHLVVKDDEMHLYKDVEHAFINTLIRGDVSSLTWFESPNQFFEDTCQKNPSLELCNVYYSAINFRDVMLAYGRLPPDAIPGQFADRECLLGMEFSGRLKDGTRLMGILPAQALATSVIVNREYAWTVPDNWSLTDAATVPVVYTTAYYALVMRGRIRRGDKVLIHGGSGGVGQAAISVALSRGCEVFTTVGNAEKKAFLQKRFPQLKDRHFANSRNSDFELHIRHQTRGRGVDVVLNSLAQHMLQASIRCLAQNGRFLEIGKVDLSQNSPLGMAVFLKNITFHGILLDAVMDPSVGKKEDWQEVARLVQDGIKSGIVQPLSYTTFSSEKAEEAFRFMSSGKHIGKVLMEIRREEPERVCVPSPIKVRAICRTLCHPNHVYLITGGLGGFGLELSQWLINRGAKKLVLTSRMGIRTGYQARCVHFWRRTGISVLVSTLNIAHLSDAHELISQCKALGPVGGVFHLAMVLRDCLFENQNVQNFKDAAEAKYWGTLNLDAATRDACGKELRWFVAFSSITSGRGNAGQTNYGWSNCTMERIIEHRREDGFPGIAIQWGAIGDVGVILENMGDNNTVVGGTLPQRMPSCLAALDLFLSWNHPIVASYIKADIGAKKVGSSGNLWQTMAHILGVNDAAQLNPDAYLGDLGLDSLMGVEIKQALERDYDIVLSMKDIRTLTLNKLQQLVDSGGTTSTVLQTTELELKKESEKEAEQNTVEQLERQMNQLFKMRVDVNDLEPMDLIIKCNKVEAGPPTFFVHSIEGIATPLKKVMSKCNFPAYCFQSTREVPQDSIEKVAQKYILEMKKIQPEGPYRIIGYSYGACIGFEMATMLQESDGANSVERLILLDGSHLYMQTYRNVYRMAFGVTGDTLVNNPLFESEIMCAMTLRFANVDYKKFRVELLQQPGFKARVQKVVDTVMTTGLFKSADTIDFACCAMRSKFVMADKYKPERKFKGLITLIRAEQGAAREEDVGSDYGISQVSDENKVYIVEGDHDSFVQGKTSAKTVNIINDLIAEANKKAKNV

SEQ ID NO: 26 - protein, 2613 aa, Caenorhabditis elegans
MDNTGEGSSDSSGTWERISDNSQSSDNMDPTQWWQKQDDIVISGVSGRFPRCDNVKMFGDMLLAGEDLVTEDSLRWTPGFCDLPKRHGKLKVLNKFDAGFFQVTPKQANFMDPQVRLLLEASWEAMVDAGINPTDLRGSKTGVFVGCSASETSGMLTQDPDTVTGYTLTGCVRSMFSNRISYTFDLQGPSFSVDTACSSSLLALQLAVDSIRQGQCDAAIVAGAHLTLTPTAALQFLRLGMLTDKGSCRSFDESGDGYCRTEGVAAIFIQRKKKAQRLYATVVHAKSNTDGHKEHGITFPSGERQAQLLQEVYSEAGIDPNSVYYVEAHGTGTKVGDPQEANAICEVFCSKRTDSLLIGSVKSNMGHAEPASGVCSLTKILLSIERQLIPPNLHYNTPNQYIPGLTDGRLKVVTEPTALPGGLIGINSFGFGGSNTHVILKAADHIAPPITPHPFTKLVTYCGRTQEAVENIFTEIESNKDDLYLQALLANQANMPANLLPFRGYMLLDRENNVETLKSITKVPITEARPIYFIYSGMGSQWPGMAIKLMKIPMFDDSLRASSKTLEEFGLDVYGMLCNPDPEQYSNNTMNCMLAITAIQIALTDVLTALGVSPDGIIGHSTGEMGCGYADGGITREQTMRLAYHRGTTIMKHTEIKGAMAAVGLTWEQVKEQAPPGVVAACHNGADSVTISGDAEGVATFCAQLKEKDIFAKVVDTSGIPFHSPAMLAVQDEMIECMRTAVPEPKPRSSKWISTSIPEDDWESDLAATCSAEYHVHNACSPVLFYEAIQKIPANAVTIEMAPHSLMQAILRRSLQKTVTNVGLMNRPKSENDDELESFLGSLGKIYQAGVNIQITELYPGGQYKGVVPKGTPMIGPMWKWDHTQDWLTIDGRQVLAGGSGSVASSATYNIDPFATDSKETYLLDHVIDGRVLYPFTGHMVLAWRTLCKLKGLDYTKTPVVFENINVFSATILTKPIKLDVVLSPGNGYFEIISDDQVAASGRIYIPEDNQPFYYGKLEDIRTSEIADRIELDTEDAYKEFLLRGYEYGQAFRGIYKTCNSGERGFLYWTGNWVTFLDSLLQTALLAERSDTLRLPTRVRHLRIDPNKHLEHVVEKDGIQVIELRNDHSTNGCIAGGVECCDLNAHSVARRIQVSGQLYHEKIFFVPHFDHNCLSGHKKTSTILKDYSAVIKQQLYTGFSKWQSAGLLKKLKNGAQIVKALAVLKASQSDVVLDDTVTRFTHDGKCTVLHHIADMFKIEDCEDFEDRVAAKLKSVRGIFELDRLWAGAVLNDRIVKSLQDICIENSAGHHATMAAVDLVSTDQIRHCIEANSSHPLLETDYTCIGANVDHLDESTLEIIGGKKQKIDLENNFTGHGEVKNLDYVLLDKVISKKADPIAFIEACKHLIRETGFLLVVEVTSQYEIALAIEGLLGNEMVGDASRKYNQFFTHEQLLDMFKSTGFLICNFQSDPALMTTTYAVRRVSPIPRDPVFIDVDDVKEFNWIEPLQKVSEERLNEPDSKTIWLVSNKCRNNGIVGLGLCFVEENLKINRFRSAFDMSANKEIRDGPPVWNIGDEETKKIVELDLHANDYMDGQWGSMRHIVVKDEDVHVYKDCEHAFINTLTRGDVSSLTWFESPNQYFDSMVKSKATQELCSVYYAPINFRDIMLAYGRLPPDAIPGNFADRECLLGMEFSGRLKDGTRLMGILPAQALATTVMVDRDYAWEVPRDWTLAEASTVPVVYTTAYYALVRRGLMKKGDKILIHGGAGGVGQAAIAIALAAGCEVFTTVGSAEKREFLKNLFPQLQEHHFANSRSADFELHIRQHTKGRGVNIVLNSLANEMLQASLRCLARHGRFLEIGKVDLSQNSSLGMAKLLDNVSVHGILLDSIMDPTVGDLDEWKEIARLLEQGIKSGVVKPLHSHSFPADKAEEAFRFMSAGKHIGKVIMEIRPDEGTKVCPPSKISVRAICRTLCHPQHTYLITGGLGGFGLELAQWLINRGARKLVLTSRTGIRTGYQARCVHFWRRTGVSVLVSTLNIAKKSDAVELINQCTAMGPIGGIFHLAMVLRDCLFENQNVQNFKDAAEAKYYGTINLDYASREHCDKNILKWFVVFSSITSGRGNAGQTNYGWSNSCMERMIDQRRADGFPGIAIQWGAIGDVGVILENMGDNNTVVGGTLPQRMPSCLSSLDNFLSWNHPIVSSFIKAELGSKKNVGGGDLMATIAHILGVNDISQLNADANLSDLGLDSLMGVEIKQALERDHDIVLSMKEIRTLTLNKLQQLADQGGTGRTALQVNELEMKKDGERDAELNTAEMLEQQMNQLFKMRVDVNDLDPQDIIVKANKVEEGPITFFVHSIEGIATPLKKVMNKCEFPAYCFQSTKNVPQTSIEDVAKCYIREMKKIQPSGPYRLVGYSYGACIGFEMANMLQESDGRDAVERLILLDGSHLYMQTYRNVYRMAFGVTGDSLVNNPLFESEIMCAMTLRFANVDYKKFRFELLQQPGFKARVQKVVDQVMLTGLFKSPETVAFACEAMHSKFLMADKYKPRRNFGGHITLIRAEQGAAREEDVGEDYGVAAVSEDCEVLKVKGDHDTFVQGKSSSVTVEHINRIILQ

SEQ ID NO: 27 - protein, 2731 aa, Caenorhabditis briggsae
MDNTGEGSSDSSGTWERISDNSQVSLLPEFRLSVSPNLSTVLLRSGRGHHHLRFSSLLLFYLLPSLPRARIRIVFASLLLLFLNVFVRSADAFLFFFSFFVYLFPLSFFRSSDNMESTNWWQKQDDIVISGVSGRFPRCDNVKEFGDLLLAGEDLVTEDDLRWPPGFYDLPKRHGKLKELKKFDAGFFSVTPKQANFMDPQVRILLEASWEAMVDAGMFLSISHFIPLFGTETEIGKLCLSPDVPGSINPIDLRGSKTGVFVGCSASETSGALTQDPESVTGYTLTGCVRSMFSNRISYTFDLQGPSFSVDTACSSSLLALQLAIDSIRQGQCDAAIVAGAHLTLTPTAALQFLRLGMLTDKGSCRSFDDSGDGYCRTEGVAAIFIQRKKKAQRIYATVLHAKSNTDGYKEQGITFPSGERQAQLLQEVYSEAGVDPNSVYYVESHGTGTKVGDPQEANAICQVFCSSRSDSLLIGSVKSNMGHAEPASGVMSLTKILLSIERQMIPPNLHYNTPNQYIPGLVDGRLKVVTEPTPLPGGIIGVNSFGFGGSNTHVILKAADHVAPAITQHPFTKIVTYCGRTQESVEKIFGEIEANKDDLYLQSLLANQANMPANLLPFRGFMLLDRENNQAALKNITKVPITEPRPIYFIYSGMGSQWPGMAIELMKIPMYDESLRASSKTLEEFGLDVYGMLCNPDPEQYSNNTMNCMLAITAIQIALTDTLTALGVSPDGIIGHSTGEMGCGYADGGITREQTMRLAYHRGTTIMKHTEIKGAMAAVGLTWEEVKAQAPPGVVAACHNGADSVTISGDAEGVASFCAQLKEKEIFAKVVDTSGIPFHSPAMLAVKDEMIESMRTAVPEPKPRSSKWISTSIPEEDWESDLAATCSAEYHVHNACSPVLFYEALQKIPANAVTIEMAPHSLMQAILRRSLQKTVTNVGLMNKPKSENDNELEGFLGSLGKIYQAGVNIQISELYPGGQYKGVVPKGTPMIGPMWQWDHSQDWQTIDGRHMVAGGGGSIPASATYNIDPFAADSKEAYLLDHVIDGRVLYPFTGHMVLAWKTLCKLKSLDFQKTPVVFENINVYSATIVTKPIKLDVVLTPGNGYFEIISDEQVAASGRIYVPEDNQPFYYGKLEDIRTSEIADRIELDTEDAYKEFLLRGYEYGQAFRGIYKTCNSGERGYLYWTGNWVTFLDSLLQTALLAERSDTLRLPTRVRHLRIDPNKHLEHVVERDGIQVVELRNDHSTNGCIAGGVECCDLNAHSVARRIQVSGQLYHEKVFFVPHFDTNCLKQHNETAATLKDYTSVIKQTLFNGFSAWKSAGLLKKLKNGALIEKALPALKSSLSDVVLDDTVTRFMHDGKCTVLPHFTEMFKIQDSEDFEDQVIGKLKSVRGIFELDRLWAGAVLNDRIVKSLQDICIENSAGHHAKMAAVDLVSTDQIRHCIEANSSHPLLEVDYTCVGATVDHLDESTLEIVGAKKQKIVLDEAFTGHGELKNMDYVLLDKVLNKKADPIAFIEACKNLIRDDGFLLVVEVTAQYEIALAIEALLGTDLAGDANRQYGQFFTHEQLLKMFETTGFKICNYQSDPALMTTTYAVRRIASVPRDPAFIDVDDIKEFSWIEPLQKTVEERLNEPDAKTIWLVSNKCRNNGIVGLALCFVEENLKSNRFRSAFDMSATKAIRDGPPVWNIGDEETKKIIDLDMHANDYMDGQWGSMRHIVVKDEDAHVYKDCEHAFINTLTRGDVSSLTWFESPNQYFDSMAKTKSSQELCSVYYAPINFRDIMLAYGRLPPDAIPGNFADRECLLGMEFSGRLKDGTRLMGILPAQALATTVMVDRDYAWEVPSDWTLAEASTVPVVYTTAYYALVRRGMMKKGDKVLIHGGAGGVGQAAIAIALAAGCEVFTTVGSTEKREFLKKLFPQLKEHHFANSRSADFELHIRQHTKGRGVNIVLNSLANEMLQASLRCLARHGRFLEIGKVDLSQNSSLGMAKLLDNVSVHGILLDSIMDPTVGDLEEWKEIARLLEQGIKSGVVKPLHSHSFPADKAEEAFRFMSAGKHIGKVIMEIRQEETTKVCPPSRISVRAICRTLCHPQHTYLITGGLGGFGLELAQWLINRGARKLVLTSRTGIRTGYQARCVHFWRRTGVSILVSTLNIAKKSDAVELVKQCTAMGPVGGVFHLAMVLRDCLFENQNIQNFKDAAEAKYYGTINLDYATREDTVKEHLKWFVVFSSITSGRGNAGQTNYGWSNSCMERMIDQRRADGFPGIAIQWGAIGDVGVILENMGDNNTVVGGTLPQRMPSCLSSLDNFLSWNHPIVSSYIKADMGAKKSAGGGNLMQTIAHILGVNDISQLNPDANLGDLGLDSLMGVEIKQALERDYDIVLSMKDIRTLTLNKLQQLAEQGGTGGTALQVNELEMKKDGERDAELNTVEMLEKQMNQLFKMRVDVNDLDPQDVIVKANKAEEGPITFFVHSIEGIATPLKKVMSKCEFPVYCFQATKNVPQTSIEDVAKYYIREMKKVQPTGPYRLVGYSYGACIGFEMACMLQQSDGQDAVEKLVLLDGSHLYMQTYRNVYRMAFGVTGDTLVNNPLFESEIMCAMTLRFANVDYKKFRVELLQQPGFKARVQKVVDTVMTTGLFKSPETVAFACMAMHSKFLMADKYKPERKFRGHITLIRAEQGAAREEDVGRDYGISQVSDDSDVHVVEGDHDTFVQGKSSAKTVSIINSLILNN

SEQ ID NO: 28 - protein, 2587 aa, Caenorhabditis remanei
MESNSWWQKQDDIVISGVSGRFPRCDNVKEFGDLLLAGEDLVTEDDLRWPPGFYDLPKRHGKLKELKKFDAGFFQVTPKQANFMDPQVRILLEASWEAMVDAGINPIDLRGSKTGVFVGCSASETSGALTQDPESVTGYTLTGCVRSMFSNRISYTFDLQGPSFSVDTACSSSLLALQLAIDSIRQGQCDAALVAGAHLTLTPTAALQFLRLGMLTDKGSCRSFDDSGDGYCRTEGVAAIFIQRKKKAQRIYATVLHAKSNTDGYKEQGITFPSGERQAQLLQEVYSEAGVDPNSVYYVESHGTGTKVGDPQEANAICQVFCSNRSDSLLIGSVKSNMGHAEPASGVCSLTKILLAIERQMIPPNLHYNTPNQYIPGLVDGRLKVVTEPTPLPGGVIGVNSFGFGGSNTHVILRAADHVAPAIHQHPFTKIVTYCGRTQESVEKMFAEIEANKENLYLQALLANQANMPANLLPFRGYMLLDRENAQSPMKNITKVPITEPRPIYFIYSGMGSQWPGMAIKLMKIPMFDESLRASSKTLDEYGLDVYGMLCNPDPEQYSNNTMNCMLAITAIQIALTDTLTALGVSPDGIIGHSTGEMGCGYADGGITREQTMRLAYYRGTTIMNHTEIKGAMAAVGLTWEEVKAQAPKGVVAACHNGADSVTISGDAEGVATFCAQLKEKDIFAKVVDTSGIPFHSPAMLAVKDEMIESMRTAVPEPKPRSSKWISTSIPEEDWESDLAATCSAEYHVHNACSPVLFYEALQKIPANAVTIEMAPHSLMQAILRRSLMKTVTNVGLMNKPKSENDDELESFLGSLGKIYQAGVNIQISELYPGGQYKGVVPKGTPMIGPMWQWDHSQDWQTIDGRHMVAGGGGSIPASATYNIDPFAADSKEAYLLDHCIDGRVLYPFTGHMVLAWKTLCKLKSLDFQKTPVVFENINVYSATIVTKPIKLDVVLSPGNGYFEIISDEQVAASGRIYVPEDNQPFYYGKLEDIRTSEIADRIELDTEDAYKEFLLRGYEYGQAFRGIYKTCNSGERGYLYWTGNWVTFLDSLLQTALLAERSDTLRLPTRVRHLRIDPNKHLEHVVERDGIQVVELRNDHSTNGCIAGGVECCDLNAHSVARRIQVSGQLYHEKVYFVPHFDQNCLKEQPETSTILKDYAAVIKQTLYNGFSKWQKAGLLKKLTNGPLIEKALPVLKSSLNEVVLDDTVTRFMHDGKCTILPHFTELFKIPDSDDFAEMVIGKLKSVRGIFELDRLWAGAVINDRIVKSLQDICIENSAGHHAKMAAVDLVSTDQIRHCIEANSSHPLLEVDYMCVGANVDHLDESTLEIVGGKKQKIVLDENFTGHGEVKNMDYVLLDKVLNKKANPIAFIEACKHLIRDDGFLLVVEVTSQFEIALALESLLGNEMAGDADRKYTQFFTHEQLLEIFKATGFKICNFQSDPALMTTTYAVRRVAPVPRDPAFIDVDDIKEFSWIEPLQKTVEERLNEPDSKTIWLVSNKCRNNGIVGLALCFVEENLKSNRFRSAFDMSATKAIRDGPPVWTIDDEETKKIIDLDLHANDYMDGQWGSMRHIVVKDEDAHVYKDCEHAFINTLTRGDVSSLTWFESPNQYFDSMAKTKSSQELCSVYYAPINFRDIMLAYGRLPPDAIPGNFADRECLLGMEFSGRLKDGTRLMGILPAQALATTVMVDRDYAWEVPSDWTLAEASTVPVVYTTAYYALVRRGMMKKGDKVLIHGGAGGVGQAAIAIALAAGCEVFTTVGSAEKRQFLKNLFPQLQEHHFANSRSADFELHIRQHTKGRGVNIVLNSLANEMLQASLRCLARHGRFLEIGKVDLSQNSSLGMAKLLDNVSIHGILLDSIMDPTVGDLEEWKEIARLLEQGIKSGVVKPLHSHSFPANKAEEAFRFMSAGKHIGKVIMEIRTEESTKICPPSRISVRAICRTLCHPQHVYLITGGLGGFGLELAQWLINRGARKLVLTSRTGIRTGYQARCVHFWRRTGVSVLVSTLNISKKSDAIELVKQCTQMGPLGGVFHLAMVLRDCLFENQNIQNFKDAAEAKYYGTINLDYATRDHSDKETLKWFVVFSSITSGRGNAGQTNYGWSNSTMERMIDQRRADGFPGIAIQWGAIGDVGVILENMGDNNTVVGGTLPQRMPSCLSSLDNFLSWNHPIVSSFIKADMGAKKSAGGGNLMQTIAHILGVNDISQLNPDANLGDLGLDSLMGVEIKQALERDYDIVLSMKDIRTLTLNKLQQLAEQGGTGGTALQVNELEMKKDGERDAELNTVEMLEKQMNQLFKMRVDVNDLDPQDIIVKANKVEEGPITFFVHSIEGIATPLKKVMSKCEFPVYCFQSTKNVPQTSIEDVAKCYIREMKKIQPTGPYRLIGYSYGACIGFEMACMLQQSDGQDAVEKLVLLDGSHLYMQTYRNVYRMAFGVTGDTLVNNPLFESEIMCAMTLRFANVDYKKFRVELLQQSGFKARVQKVVDTVMTTGLFKSDETVAFACMAMHSKFLMADKYKPERKFRGHITLIRAEQGAAREEDVGRDYGISQVSDDSDVHVVEGDHDTFVQGKSSAKTVSIINSIILNK

SEQ ID NO: 29 - protein, 320 aa, Mus musculus
NKRPLWFICSGMGTQWRGMGLSLMRLDSFRESILRSDEAVKPLGVKVSDLLLSTDERTFDDIVHAFVSLTAIQIALIDLLTSVGLKPDGIIGHSLGEVACGYADGCLSQREAVLAAYWRGQCIKDAHLPPGSMAAVGLSWEECKQRCPAGVVPACHNSEDTVTISGPQAAVNEFVEQLKQEGVFAKEVRTGGLAFHSYFMEGIAPTLLQALKKVIREPRPRSARWLSTSIPEAQWQSSLARTSSAEYNVNNLVSPVLFQEALWHIPEHAVVLEIAPHALLQAVLKRGVKSSCTIIPLMKRDHKDNLEFFLTNLGKVHLTG

SEQ ID NO: 30 - protein, 319 aa, Rattus norvegicus
SQRPLWFICSGMGTQWRGMGLSLMRLDSFRESILRSDEALKPLGVKVSDLLLSTDEHTFDDIVHSFVSLTAIQIALIDLLTSMGLKPDGIIGHSLGEVACGYADGCLSQREAVLAAYWRGQCIKDANLPAGSMAAVGLSWEECKQRCPPGVVPACHNSEDTVTISGPQAAVNEFVEQLKQEGVFAKEVRTGGLAFHSYFMEGIAPTLLQALKKVIREPRPRSARWLSTSIPEAQWQSSLARTSSAEYNVNNLVSPVLFQEALWHVPEHAVVLEIAPHALLQAVLKRGVKPSCTIIPLMKRDHKDNLEFFLTNLGKVHLT

SEQ ID NO: 31 - protein, 319 aa, Cricetulus griseus
SKRPLWFICSGMGTQWRGMGLSLMRLDSFRESILRSDEAVKPLGIKVSDLLLSTDESTFDDIVHAFVGLTAIQIALIDLLTSVGLKPDGIIGHSLGEVACGYADGCLSQREAVLAAYWRGQCIKDAHLPPGSMAAVGLSWEECKQRCPSGVVPACHNSEDTVTISGPQAAVSEFVEQLKQEGVFAKEVRTGGLAFHSYFMEGIAPMLLQALKKVIREPRPRSARWLSTSIPEAQWQSSLARTSSAEYNVNNLVSPVLFQEALWHVPEHAVLLEIAPHALLQAVLKRGVKSSCTIIPLMKRDHKDNLEFFLTNLGKVHLT

SEQ ID NO: 32 - protein, 319 aa, Homo sapiens
GERPLWFICSGMGTQWRGMGLSLMRLDRFRDSILRSDEAVKPFGLKVSQLLLSTDESTFDDIVHSFVSLTAIQIGLIDLLSCMGLRPDGIVGHSLGEVACGYADGCLSQEEAVLAAYWRGQCIKEAHLPPGAMAAVGLSWEECKQRCPPGVVPACHNSKDTVTISGPQAPVFEFVEQLRKEGVFAKEVRTGGMAFHSYFMEAIAPPLLQELKKVIREPKPRSARWLSTSIPEAQWHSSLARTSSAEYNVNNLVSPVLFQEALWHVPEHAVVLEIAPHALLQAVLKRGLKPSCTIIPLMKKDHRDNLEFFLAGIGRLHLS

SEQ ID NO: 33 - protein, 319 aa, Macaca mulatta
GERPLWFICSGMGTQWRGMGLSLMRLDRFRDSILRSDEAVKPFGLKVSQLLLSMDESTFDDIVHAFVSLTAIQIGLIDLLSCMGLRPDGIIGHSLGEVACGYADGCLSQEEAVLAAYWRGQCIKEAHLPPGAMAAVGLSWEECKQRCPPGVVPACHNSKDTVTISGPQASVFEFMEQLRKEGVFAKEVRTGGMAFHSYFMEAIAPPLLQALKKVIREPKPRSARWLSTSIPEAQWHSSLARTSSAEYNVNNLVSPVLFQEALCHVPEHAVVLEVAPHALLQAVLKRGLKPGCTIIPLMKKDHRDNLEFFLTGIGRLHLS

SEQ ID NO: 34 - protein, 319 aa, Bos taurus
GKRPLWFICSGMGTQWRGMGLSLMRLSRFRDSILRSDEAVKPLGLQVSQLLLSTDEAIFDDMVISFVSLTAIQIALIDLLTSMGLQPDGIIGHSLGEVACGYADGCISQEEAILSAYWRGQCIKEANIPPGAMAAVGLTWEECKQRCPPGIVPACHNCIDTVTISGPQASMLEFVQQLKQEGVFAKEVRTGGMAFHSYFMDAIAPMLLQQLKKVIREPQPRSPRWLSTSIPETQWQESLARTFSAEYNVNNLVSPVLFQEALWRVPEDAVVLEIAPHALLQAVLKRGLKSSCTIIPLMKKDHRDNLEFFLSNVGQLYLT

SEQ ID NO: 35 - protein, 318 aa, Capra hircus
SKRPLWFICSGMGTQWRGMGLSLMRLSSFRDSILRSDEAVKPLGLRVSQLLLSADDIFDDIIVSFVSLTAFQIALIDLLTSMGLRPDGIIGHSLGEVACAYADGCISQEEAILSAYWRGQCIKEANIPPGAMAAVGLTWEECKQRCPPGIVPACHNSIDTVTISGPQASMLEFVKQLKQEGVFAKEVQTGGMAFHSYFMDAIAPTLLQQLKKVIREPQLRSPRWLSTSIPESQWHESLARTFSAEYNVNNLVSPVLFQEALWHVPENAVVLEIAPHALLQAILKRGLQPSCTIIPLMKKDHRDNLEFFLSNVGQLYLT

SEQ ID NO: 36 - protein, 319 aa, Equus caballus
GQRPLWFICSGMGAQWRGMGLSLMRLGTFRDSILRSDKAVKPLGLQVSDLLLSADEATFDDTVPGFVSLTAIQIALIDLLTSMGLRPDGIIGHSLGEVACGYADGCVSQEEAILAAYWRGQCIKEANIPPGAMAAVGLSWEECKQRCPPGVVPACHNSKDTVTISGPQAAVSEFVEQLKQEGVFAKEVRTGGLAFHSYFMDSISHTLLQALKKVIREPRPRSVRWLSTSIPEAQWQSSLARTFSAEYNVNNLVSPVLFQEALCHVPEHAVVLEIAPHALLQAVLKRGLKPSCTIVPLMKKDHRDNLEFFLSNVGRLHLM

SEQ ID NO: 37 - protein, 319 aa, Felis catus
GKRPLWFICSGMGAQWCGMGLSLMRLGSFRDSILRSDEAVKPLGLQVSELLLSTDEATFDDIIHAFVSLTAIQIALIDLLNSMGLRPDGIIGHSLGEVACGYADGCLSQEEAILAAYWRGQCIKETNIPPGTMAAVGLSWEECKQRCPPGVVPACHNSEDTVTISGPQAEVAAFVAELKREGVFAKEVRTGGMAFHSYFMDSIAPTLLQALKKVIREPRPRSARWLSTSIPEAQWQGSLARTFSAEYNVNNLVSPVLFQEALWHVPGDAVVLEIAPHALLQAVLKRGLKSSCTIVPLMKKDQRDNLEFFLSNVGKLHLL

SEQ ID NO: 38 - protein, 319 aa, Sus scrofa
SKRPVWFICSGMGAQWQGMGLSLMRLDRFRDSILRSDQALKPLGLRVSDLLLSTDEAVLDDIVSSFVSLTSIQIALIDLLTSLGLQPDGIIGHSLGEVACGYADGCLTQEEAVLSSYWRGYCIKEANVLPGAMAAVGLSWEECKQRCPPGIVPACHNSKDTVTISGPQAAMSEFLQQLKREDVFVKEVRTGGIAFHSYFMESIAPTLLRQLRKVILDPKPRSKRWLSTSIPEAQWQGSLARTFSAEYSVNNLVSPVLFQEALQHVPAHAVVVEIAPHALLQAVLKRSLESSCTIIPLMKKDHRDNLEFFLSNVGRLHLA

SEQ ID NO: 39 - protein, 319 aa, Cuculus canorus
TGRPLWYICSGMGTQWKGMGLSLMKLDLFRQSVLRSDEALKHTGLKVSELLLNEDENTFDDTVHAFVGLAAIQIAQIDILKAAGLEPDGIVGHSVGELACGYADNSLSHEEAILAAYWRGRCVKDAKLPPGGMAAVGLSWEECKQICPPNVVPACHNSEDTVTVSGPLGAVSEFVAKLKKDGVFAKEVRTSGVAFHSHYMASIAPVLLSALKKVIPHPKPRSPRWISTSIPESQWQSDLARYSSAEYHVNNLVNPVLFHEGLSHVPGNALVVEIAPHALLQAILKRSLKPTCIILPLMKKEHKNNLEFFLTQLGKFHMS

SEQ ID NO: 40 - protein, 319 aa, Calypte anna
SGRPLWYICSGMGTQWKGMGLSLMKLDLFRQSILRSDQALKNTGLKVSDLLLQADDNTFDETVHAFVGLAAIQIAQIDMLKAAGLQPDGILGHSVGELACGYADNCLSHEEAILAAYWRGRCVKEAKLPPGGMAAVGLTWEECKQQCPPNVVPACHNSEDTVTISGPLATVSEFVAKLKKAGVFAKEVRSAGVAFHSHYMASIAPVLLSALKKVIPHPKPRSARWISTSIPESQWQSDLAKYSSAEYHVNNLVSPVLFHEGLKHIPENAVVVEIAPHALLQAILKRTLKPTCTILPLMKKDHKNNLEFFLTQAGKIHLT

SEQ ID NO: 41 - protein, 319 aa, Anas platyrhynchos
SGRPLWYICSGMGTQWKGMGLSLMKLDVFRQSIMRSDEALKNTGLKVSDLLLQADDNTFDETVNAFVGVAAVQIAQIDMLKAAGLQPDGILGHSVGEVACGYADNSLSHEEAILAAYWRGRCVKEAKLPPGGMAAVGLTWEECKQRCPPNVVPACHNSEDTVTISGPLDSVNEFVAKLKKDGVFAKEVRSAGVAFHSYYMASIAPALLSALRKVIPHPKPRSARWISTSIPESQWQSDLARNSSAEYYVNNLVSPVLFHEGLKHIPENAVVVEIAPHALLQAILRRSLKPSCTILPLMKKDQKNNLEFFLTQAGKIHLT

SEQ ID NO: 42 - protein, 319 aa, Gallus gallus
SGRPLWYICSGMGTQWKGMGLSLMKLDLFRQSILRSDEALKSTGLKVSDLLLNADENTFDDTVHAFVGLAAIQIAQIDVLKAAGLQPDGILGHSVGELACGYADNSLSHEEAVLAAYWRGRCVKEAKLPPGGMAAVGLTWEECKQRCPPNVVPACHNSEDTVTVSGPLDSVSEFVTKLKKDGVFAKEVRRAGVAFHSYYMASIAPALLSALKKVIPHPKPRSARWISTSIPESQWQSDLARNSSAEYHVNNLVNPVLFHEGLKHIPENAVVVEIAPHALLQAILRRTLKPTCTILPLMKKDHKNNLEFFLTQTGKIHLT

SEQ ID NO: 43 - protein, 319 aa, Nestor notabilis
SGRPLWYICSGMGSQWKGMGLSLMKLDMFRQSILRSDEALKNTGLKVSDLLLRADENTFDETINAFVGLAAIQIAQIDLLKAAGLQPDGILGHSVGELACGYADNCLSQEEAILGAYWRGRCVKEAKLPPGAMAAVGLTWEECKQRCPPNVVPACHNSEDTVTVSGPLESVTEFVAKLKKDGVFAKEVRSAGVAYHSHYMASIAPVLLNALKKVIPHPKPRSARWISTSIPESQWQSDLARSCSAEYLVNNLVNPVLFHDGLKHVPENAVVVEIAPHALLQAILRRTLKPTCTILPLMKKDQKNNLEFFLTQTGKIHLT

SEQ ID NO: 44 - protein, 319 aa, Podiceps cristatus
SGRPLWYICSGMGTQWKGMGVDLMKLDLFRQSILRSDEALKSTGLKVSDLLLQADENTFDDTVHAFVGLAAIQIAQIDMLKAAGLQPDGILGHSVGELACGYADNSLSREEAILAAYWRGRCVKEAKLPPGGMAAVGLTWEECKQCCPPNVVPACHNSEDTVTISGPLDSVHEFVAKLKKDGVFAKEVRSAGVAFHSYYMASIAPVLLSALKKVIPHPKPRSARWISTSIPESQWQSDLARNSSAEYHVNNLVNPVLFHEGLKHVPENAVVVEIAPHALLQAILRRTLKPTCTILPLMKKDHKNNLEFFLTQTGKIHLT

SEQ ID NO: 45 - protein, 319 aa, Balearica regulorum
  source 1..319: note = Balearica regulorum gibbericeps
SGRPLWYICSGMGTQWKGMGLSLMKLDLFRQSILRSDEALKNTGLKVSDLLLQADENTFDDTVHAFVGLAAIQIAQIDMLKAAGLQPDGILGHSVGELACGYADNSLSHEEAILAAYWRGRCVKEAKLPPGGMAAVGLTWEECKQCCPPNVVPACHNSEDTVTVSGPLDSVNEFVAKLKKDGVFAKEVRSAGVAFHSYYMASIAPVLLSALKKVIPHPKPRSARWISTSIPESQWQSDLARNSSAEYHVNNLVNPVLFHEGLKHVPENAVVVEIAPHALLQAILRRTLKPTCTILPLMKKEHKNNLEFFLTQTGKIHLT

SEQ ID NO: 46 - protein, 319 aa, Phaethon lepturus
SDRPLWYICSGMGTQWKGMGLSLMKLDLFRQSILRSDEALKNTGLKVSDLLLQADENTFDDTVHAFVGLAAIQIAQIDMLKAAGLQPDGILGHSVGELACGYADNSLSHEEAILAAYWRGRCVKEAKLPPGGMAAVGLTWEECKQCCPPNVVPACHNSEDTVTVSGPLDSVNEFVAKLKKDGVFAKEVRSAGVAFHSYYMASIAPVLLSALKKVIPHPKPRSARWISTSIPESQWQSDLARNSSAEYHVNNLVNPVLFHEGLKHIPENAVVVEIAPHALLQAILRRTLKPTCTILPLMKKEHKNNLEFFLTQTGKIHLT

SEQ ID NO: 47 - protein, 319 aa, Phoenicopterus ruber
SGRPLWYICSGMGTQWKGMGLSLMKLDLFRQSILRSDEALKNTGLKVSDLLLQADENTFDDTVHAFVGLAAIQIAQIDLLKAAGLQPDGILGHSVGELACGYADNSLSHEEAILAAYWRGRCVKEAKLPPGGMAAVGLTWEECKQCCPPNVVPACHNSEDTVTVSGPLDSVREFVAKLKKDGVFAKEVRSAGVAFHSYYMASIAPVLLSALKKVIPHPKPRSARWISTSIPESQWQSDLARNSSAEYHVNNLVNPVLFQEGLKHIPENAVVVEIAPHALLQAILRRALKPTCTILPLMKKEHKNNLEFFLTQTGKIHLT

SEQ ID NO: 48 - protein, 319 aa, Ooceraea biroi
EKRPIWFVFSGMGTQWSGMGRELLGIEVFRRTLQRCADTLLPHGVDLMNIILNNTNETLENVIDTFVAIAAMQVALIDVLAAIDIYPDGIAGHSVGELGCAYADGAFTAEQTVLAAYWRGKSIVDSTLEPGAMAAVGLSWEDAQKMCPPNVSPACHNSMDSVTISGPTKDVLKFVEELKSKNIFAKLVRSSGIAFHSKYIASAGPKLRASLDKIIPNPKQRSAKWISSSIPEAAWGSPLAQVSSSAYHVNNLLSPVLFQEAIAHIPDNAITIEIAPHCLLQAILRRSLPSTVTNVSLHMRDHTNNLAFLLSNIGKLYMA

SEQ ID NO: 49 - protein, 319 aa, Anopheles funestus
DKRPVWFIYSGMGSQWASMAKDLMQLEVFHNSIYRCAEALRPEGVDLIDVLTKSDDTKFDNILNSFISIAAVQVALTDVLTHVGITPDGMVGHSVGELGCAYADGCFTPEQTVLAAYWRGRSILDTDLIAGQMAAVGLSWEECKQKLPKDVIPACHNSADSVTISGPVNSVGKVIADLNAQGIFAKGVKSSGIAFHSRYIADAAPKLRKSLDKIIPNPKNRTPRWISTSIPEESWPTPLAQQSSSAYHVNNLLSPVLFSEGLKHVPANAICIEIAPHGLLQAILKRALGKDATNLSLMKRDHANNMIFLLSNLGKLYAA

SEQ ID NO: 50 - protein, 319 aa, Anopheles darlingi
EKRPLWFIYSGMGSQWASMARDLMQLEVFHSTIARCAEALRPEGIDLIDVLTKSDESRFDNILNSFISIAAVQVALTDVLTHVGIVPEGMVGHSVGELGCAYADGCFTPEQTVLAAYWRGRSILDTDLIAGQMAAVGLSWEDCKQKLPKDVIPACHNSSDSVTISGPVASVGKVIADLNAQGIFAKGVKSSGIAFHSRYIADAAPKLRKSLDKIIPNPKPRTQRWISTSIPEESWGTALAQQSSSAYHVNNLLSPVLFAEGLKHVPANAICIEIAPHGLLQAILKRALGKEATNLSLMKRDHDNNLIFLLSNLGKLYAA

SEQ ID NO: 51 - protein, 319 aa, Glossina austeni
ESRPIWFVYSGMGSQWASMAKDLMVFDTFKKTIHRCCEILRPEGLDLMEVLTRSTEKTFENILNSFVGIAAMQVALTDLLTSLNIVPDGIVGHSVGEVACAYADGCLSMEQTILAAYWRGKSILDTKLTKGKMAAVGLSWEEAHKRLPADCFPACHNSAENCTISGPEESIDAVCQKLTAEGVFARAVKSSGYAFHSKYIADAGPKLRKSLEKVIPNAKNRSPRWISSSIPEVAWNTAIAQQASAAYHVNNLLSPVLFHQALQHVPKNAICIEVAPTGLLQAILKRSLGNETTNLSLIKRDYENNPEFFLASIGKLYAA

SEQ ID NO: 52 - protein, 319 aa, Drosophila melanogaster
DKRPIWYIYSGMGSQWASMAKDLMKIEAFAKTIQRCADVLKPEGVDLIDVLTRSTDKSFENILNSFISIAAMQVALTDLLSSLGIHPDGIVGHSVGELGCAYADGCFTPEQTVLAAYWRGKSILDTQLAKGKMAAVGLSWEDAHSRVPSDCFPVCHNSEDNCTISGPEASIEALVAKLNAEGVFAKAVNSSGYAFHSKYIAEAGPKLRKSLEKIIPNAKNRTARWISTSIPESAWNTPVAKQSSAAYHVNNLLSPVLFHEALQHVPKNAISVEIAPHGLLQAILKRALGPDATNLSLVKRGHENNVEFFLTNVGKLFAA

SEQ ID NO: 53 - protein, 320 aa, Brugia malayi
EPKQIYFIYSGMGSQWAGMVRQLMSIPAFDESLRSSSDAIVDFGVNVYEMLQSDDPSFYKNNTLNCMLAITAIQIALTDVLFLLGVMPDGIIGHSTGEMCCGYADGGLTREQTMQLAYHRGHTIMNANIKGGMAAVGLSWEEAGKRCPEGVIPACHNAADSVTISGDAEKIKEFVEELKKEDIFGKLVDSSGIPFHSPAMLKVKDKMLKAMRTSVPNPKPRSSRWISTSIPESNWENELAQMCSADYHTNNAVSPVLFYEALQKIPANAVTIEIAPHCLMHSILRRSLQKTCTNVGLINMKEKDRELESFLQALGKIYQT

SEQ ID NO: 54 - protein, 323 aa, Caenorhabditis elegans
EARPIYFIYSGMGSQWPGMAIKLMKIPMFDDSLRASSKTLEEFGLDVYGMLCNPDPEQYSNNTMNCMLAITAIQIALTDVLTALGVSPDGIIGHSTGEMGCGYADGGITREQTMRLAYHRGTTIMKHTEIKGAMAAVGLTWEQVKEQAPPGVVAACHNGADSVTISGDAEGVATFCAQLKEKDIFAKVVDTSGIPFHSPAMLAVQDEMIECMRTAVPEPKPRSSKWISTSIPEDDWESDLAATCSAEYHVHNACSPVLFYEAIQKIPANAVTIEMAPHSLMQAILRRSLQKTVTNVGLMNRPKSENDDELESFLGSLGKIYQA

SEQ ID NO: 55 - protein, 323 aa, Caenorhabditis briggsae
EPRPIYFIYSGMGSQWPGMAIELMKIPMYDESLRASSKTLEEFGLDVYGMLCNPDPEQYSNNTMNCMLAITAIQIALTDTLTALGVSPDGIIGHSTGEMGCGYADGGITREQTMRLAYHRGTTIMKHTEIKGAMAAVGLTWEEVKAQAPPGVVAACHNGADSVTISGDAEGVASFCAQLKEKEIFAKVVDTSGIPFHSPAMLAVKDEMIESMRTAVPEPKPRSSKWISTSIPEEDWESDLAATCSAEYHVHNACSPVLFYEALQKIPANAVTIEMAPHSLMQAILRRSLQKTVTNVGLMNKPKSENDNELEGFLGSLGKIYQA

SEQ ID NO: 56 - protein, 323 aa, Caenorhabditis remanei
EPRPIYFIYSGMGSQWPGMAIKLMKIPMFDESLRASSKTLDEYGLDVYGMLCNPDPEQYSNNTMNCMLAITAIQIALTDTLTALGVSPDGIIGHSTGEMGCGYADGGITREQTMRLAYYRGTTIMNHTEIKGAMAAVGLTWEEVKAQAPKGVVAACHNGADSVTISGDAEGVATFCAQLKEKDIFAKVVDTSGIPFHSPAMLAVKDEMIESMRTAVPEPKPRSSKWISTSIPEEDWESDLAATCSAEYHVHNACSPVLFYEALQKIPANAVTIEMAPHSLMQAILRRSLMKTVTNVGLMNKPKSENDDELESFLGSLGKIYQA

SEQ ID NO: 57 - protein, 319 aa, synthetic construct
NKRPLWFICSGMGTQWRGMGLSLMRLDSFRESILRSDEAVKPLGVKVSDLLLSTDERTFDDIVHAFVSLTAIQIALIDLLTSVGLKPDGIIGHSLGEVACGYADGCLSQREAVLAAYWRGQCIKDAHLPPGSMAAVGLSWEECKQRCPAGVVPACHNSEDAVTISGPQAAVNEFVEQLKQEGVFAKEVRTGGLAFHSYFMEGIAPTLLQALKKVIREPRPRSARWLSTSIPEAQWQSSLARTSSAEYNVNNLVSPVLFQEALWHIPEHAVVLEIAPHALLQAVLKRGVKSSCTIIPLMKRDHKDNLEFFLTNLGKVHLT

SEQ ID NO: 58 - protein, 319 aa, synthetic construct
NKRPLWFICSGMGTQWRGMGLSLMRLDSFRESILRSDEAVKPLGVKVSDLLLSTDERTFDDIVHAFVSLTAIQIALIDLLTSVGLKPDGIIGHSLGEVACGYADGCLSQREAVLAAYWRGQCIKDAHLPPGSMAAVGLSWEECKQRCPAGVVPACHNSEDYVTISGPQAAVNEFVEQLKQEGVFAKEVRTGGLAFHSYFMEGIAPTLLQALKKVIREPRPRSARWLSTSIPEAQWQSSLARTSSAEYNVNNLVSPVLFQEALWHIPEHAVVLEIAPHALLQAVLKRGVKSSCTIIPLMKRDHKDNLEFFLTNLGKVHLT

SEQ ID NO: 59 - protein, 319 aa, synthetic construct
NKRPLWFICSGMGTQWRGMGLSLMRLDSFRESILRSDEAVKPLGVKVSDLLLSTDERTFDDIVHAFVSLTAIQIALIDLLTSVGLKPDGIIGHSLGEVACGYADGCLSQREAVLAAYWRGQCIKDAHLPPGSMAAVGLSWEECKQRCPAGVVPACHNSEDAVTISGPQAAVNEFVEQLKQEGVAAKEVRTGGLAFHSYFMEGIAPTLLQALKKVIREPRPRSARWLSTSIPEAQWQSSLARTSSAEYNVNNLVSPVLFQEALWHIPEHAVVLEIAPHALLQAVLKAGVKSSCTIIPLMKRDHKDNLEFFLTNLGKVHLT

SEQ ID NO: 60 - protein, 319 aa, synthetic construct
NKRPLWFICSGMGTQWRGMGLSLMRLDSFRESILRSDEAVKPLGVKVSDLLLSTDERTFDDIVHAFVSLTAIQIALIDLLTSVGLKPDGIIGHSLGEVACGYADGCLSQREAVLAAYWRGQCIKDAHLPPGSMAAVGLSWEECKQRCPAGVVPACHNSEDAVTISGPQAAVNEFVEQLKQEGVAAAEVRTGGLAFHSYFMEGIAPTLLQALKKVIREPRPRSARWLSTSIPEAQWQSSLARTSSAEYNVNNLVSPVLFQEALWHIPEHAVVLEIAPHALLQAVLKAGVKSSCTIIPLMKRDHKDNLEFFLTNLGKVHLT

SEQ ID NO: 61 - protein, 319 aa, synthetic construct
NKRPLWFICSGMGTQWRGMGLSLMRLDSFRESILRSDEAVKPLGVKVSDLLLSTDERTFDDIVHAFVSLTAIQIALIDLLTSVGLKPDGIIGHSLGEVACGYADGCLSQREAVLAAYWRGQCIKDAHLPPGSMAAVGLSWEECKQRCPAGVVPACHNSEDTVTISGPQAAVNEFVEQLKQEGVFAEEVRTGGLAFHSYFMEGIAPTLLQALKKVIREPRPRSARWLSTSIPEAQWQSSLARTSSAEYNVNNLVSPVLFQEALWHIPEHAVVLEIAPHALLQAVLKRGVKSSCTIIPLMKRDHKDNLEFFLTNLGKVHLT

SEQ ID NO: 62 - protein, 319 aa, synthetic construct
NKRPLWFICSGMGTQWRGMGLSLMRLDSFRESILRSDEAVKPLGVKVSDLLLSTDERTFDDIVHAFVSLTAIQIALIDLLTSVGLKPDGIIGHSLGEVACGYADGCLSQREAVLAAYWRGQCIKDAHLPPGSMAAVGLSWEECKQRCPAGVVPACHNSEDTVTISGPQAAVNEFVEQLKQEGVFADEVRTGGLAFHSYFMEGIAPTLLQALKKVIREPRPRSARWLSTSIPEAQWQSSLARTSSAEYNVNNLVSPVLFQEALWHIPEHAVVLEIAPHALLQAVLKRGVKSSCTIIPLMKRDHKDNLEFFLTNLGKVHLT

SEQ ID NO: 63 - protein, 319 aa, synthetic construct
NKRPLWFICSGMGTQWRGMGLSLMRLDSFRESILRSDEAVKPLGVKVSDLLLSTDERTFDDIVHAFVSLTAIQIALIDLLTSVGLKPDGIIGHSLGEVACGYADGCLSQREAVLAAYWRGQCIKDAHLPPGSMAAVGLSWEECKQRCPAGVVPACHNSEDTVTISGPQAAVNEFVEQLKQEGVFAKEVRTGGLAFHSYFMEGIAPTLLQALKKVIREPRPRSARWLSTSIPEAQWQSSLARTSSAEYNVNNLVSPVLFQEALWHIPEHAVVLEIAPHALLQAVLDRGVKSSCTIIPLMKRDHKDNLEFFLTNLGKVHLT

SEQ ID NO: 64 - protein, 319 aa, synthetic construct
NKRPLWFICSGMGTQWRGMGLSLMRLDSFRESILRSDEAVKPLGVKVSDLLLSTDERTFDDIVHAFVSLTAIQIALIDLLTSVGLKPDGIIGHSLGEVACGYADGCLSQREAVLAAYWRGQCIKDAHLPPGSMAAVGLSWEECKQRCPAGVVPACHNSEDTVTISGPQAAVNEFVEQLKQEGVFAKEVRTGGLAFHSYFMEGIAPTLLQALKKVIREPRPRSARWLSTSIPEAQWQSSLARTSSAEYNVNNLVSPVLFQEALWHIPEHAVVLEIAPHALLQAVLERGVKSSCTIIPLMKRDHKDNLEFFLTNLGKVHLT

SEQ ID NO: 65 - protein, 319 aa, synthetic construct
NKRPLWFICSGMGTQWRGMGLSLMRLDSFRESILRSDEAVKPLGVKVSDLLLSTDERTFDDIVHAFVSLTAIQIALIDLLTSVGLKPDGIIGHSLGEVACGYADGCLSQREAVLAAYWRGQCIKDAHLPPGSMAAVGLSWEECKQRCPAGVVPACHNSEDTVTISGPQAAVNEFVEQLKQEGVFAKEVRTGGLAFHSYFMEGIAPTLLQALKKVIREPRPRSARWLSTSIPEAQWQSSLARTSSAEYNVNNLVSPVLFQEALWHIPEHAVVLEIAPHALLQAVLKRGVKSSCTIIPLMKDDHKDNLEFFLTNLGKVHLT

SEQ ID NO: 66 - protein, 319 aa, synthetic construct
NKRPLWFICSGMGTQWRGMGLSLMRLDSFRESILRSDEAVKPLGVKVSDLLLSTDERTFDDIVHAFVSLTAIQIALIDLLTSVGLKPDGIIGHSLGEVACGYADGCLSQREAVLAAYWRGQCIKDAHLPPGSMAAVGLSWEECKQRCPAGVVPACHNSEDTVTISGPQAAVNEFVEQLKQEGVFAKEVRTGGLAFHSYFMEGIAPTLLQALKKVIREPRPRSARWLSTSIPEAQWQSSLARTSSAEYNVNNLVSPVLFQEALWHIPEHAVVLEIAPHALLQAVLKRGVKSSCTIIPLMKEDHKDNLEFFLTNLGKVHLT

SEQ ID NO: 67 - protein, 319 aa, synthetic construct
NKRPLWFICSGMGTQWRGMGLSLMRLDSFRESILRSDEAVKPLGVKVSDLLLSTDERTFDDIVHAFVSLTAIQIALIDLLTSVGLKPDGIIGHSLGEVACGYADGCLSQREAVLAAYWRGQCIKDAHLPPGSMAAVGLSWEECKQRCPAGVVPACHNSEDTVTISGPQAAVNEFVEQLKQEGVFADEVRTGGLAFHSYFMEGIAPTLLQALKKVIREPRPRSARWLSTSIPEAQWQSSLARTSSAEYNVNNLVSPVLFQEALWHIPEHAVVLEIAPHALLQAVLKRGVKSSCTIIPLMKDDHKDNLEFFLTNLGKVHLT

SEQ ID NO: 68 - protein, 319 aa, synthetic construct
NKRPLWFICSGMGTQWRGMGLSLMRLDSFRESILRSDEAVKPLGVKVSDLLLSTDERTFDDIVHAFVSLTAIQIALIDLLTSVGLKPDGIIGHSLGEVACGYADGCLSQREAVLAAYWRGQCIKDAHLPPGSMAAVGLSWEECKQRCPAGVVPACHNSEDTVTISGPQAAVNEFVEQLKQEGVFADEVRTGGLAFHSYFMEGIAPTLLQALKKVIREPRPRSARWLSTSIPEAQWQSSLARTSSAEYNVNNLVSPVLFQEALWHIPEHAVVLEIAPHALLQAVLKRGVKSSCTIIPLMKEDHKDNLEFFLTNLGKVHLT

SEQ ID NO: 69 - protein, 319 aa, synthetic construct
NKRPLWFICSGMGTQWRGMGLSLMRLDSFRESILRSDEAVKPLGVKVSDLLLSTDERTFDDIVHAFVSLTAIQIALIDLLTSVGLKPDGIIGHSLGEVACGYADGCLSQREAVLAAYWRGQCIKDAHLPPGSMAAVGLSWEECKQRCPAGVVPACHNSEDTVTISGPQAAVNEFVEQLKQEGVFAEEVRTGGLAFHSYFMEGIAPTLLQALKKVIREPRPRSARWLSTSIPEAQWQSSLARTSSAEYNVNNLVSPVLFQEALWHIPEHAVVLEIAPHALLQAVLKRGVKSSCTIIPLMKDDHKDNLEFFLTNLGKVHLT

SEQ ID NO: 70 - protein, 319 aa, synthetic construct
NKRPLWFICSGMGTQWRGMGLSLMRLDSFRESILRSDEAVKPLGVKVSDLLLSTDERTFDDIVHAFVSLTAIQIALIDLLTSVGLKPDGIIGHSLGEVACGYADGCLSQREAVLAAYWRGQCIKDAHLPPGSMAAVGLSWEECKQRCPAGVVPACHNSEDTVTISGPQAAVNEFVEQLKQEGVFAEEVRTGGLAFHSYFMEGIAPTLLQALKKVIREPRPRSARWLSTSIPEAQWQSSLARTSSAEYNVNNLVSPVLFQEALWHIPEHAVVLEIAPHALLQAVLKRGVKSSCTIIPLMKEDHKDNLEFFLTNLGKVHLT

SEQ ID NO: 71 - protein, 319 aa, synthetic construct
NKRPLWFICSGMGTQWRGMGLSLMRLDSFRESILRSDEAVKPLGVKVSDLLLSTDERTFDDIVHAFVSLTAIQIALIDLLTSVGLKPDGIIGHSLGEVACGYADGCLSQREAVLAAYWRGQCIKDAHLPPGSMAAVGLSWEECKQRCPAGVVPACHNSEDTVTISGPQAAVNEFVEQLKQEGVFAKEVRTGGLAFHSYFMEGIAPTLLQALKKVIREPRPRSARWLSTSIPEAQWQSSLARTSSAEYNVNNLVSPVLFQEALWHIPEHAVVLEIAPHALLQVVLKRGVKSSCTIIPLMKRDHKDNLEFFLTNLGKVHLT

SEQ ID NO: 72 - protein, 319 aa, synthetic construct
NKRPLWFICSGMGTQWRGMGLSLMRLDSFRESILRSDEAVKPLGVKVSDLLLSTDERTFDDIVHAFVSLTAIQIALIDLLTSVGLKPDGIIGHSLGEVACGYADGCLSQREAVLAAYWRGQCIKDAHLPPGSMAAVGLSWEECKQRCPAGVVPACHNSEDTVTISGPQAAVNEFVEQLKQEGVFAKEVRTGGLAFHSYFMEGIAPTLLQALKKVIREPRPRSARWLSTSIPEAQWQSSLARTSSAEYNVNNLVSPVLFQEALWHIPEHAVVLEIAPHALLQLVLKRGVKSSCTIIPLMKRDHKDNLEFFLTNLGKVHLT

SEQ ID NO: 73 - protein, 319 aa, synthetic construct
NKRPLWFICSGMGTQWRGMGLSLMRLDSFRESILRSDEAVKPLGVKVSDLLLSTDERTFDDIVHAFVSLTAIQIALIDLLTSVGLKPDGIIGHSLGEVACGYADGCLSQREAVLAAYWRGQCIKDAHLPPGSMAAVVLSWEECKQRCPAGVVPACHNSEDTVTISGPQAAVNEFVEQLKQEGVFAKEVRTGGLAFHSYFMEGIAPTLLQALKKVIREPRPRSARWLSTSIPEAQWQSSLARTSSAEYNVNNLVSPVLFQEALWHIPEHAVVLEIAPHALLQAVLKRGVKSSCTIIPLMKRDHKDNLEFFLTNLGKVHLT

SEQ ID NO: 74 - protein, 319 aa, synthetic construct
NKRPLWFICSGMGTQWRGMGLSLMRLDSFRESILRSDEAVKPLGVKVSDLLLSTDERTFDDIVHAFVSLTAIQIALIDLLTSVGLKPDGIIGHSLGEVACGYADGCLSQREAVLAAYWRGQCIKDAHLPPGSMAAVLLSWEECKQRCPAGVVPACHNSEDTVTISGPQAAVNEFVEQLKQEGVFAKEVRTGGLAFHSYFMEGIAPTLLQALKKVIREPRPRSARWLSTSIPEAQWQSSLARTSSAEYNVNNLVSPVLFQEALWHIPEHAVVLEIAPHALLQAVLKRGVKSSCTIIPLMKRDHKDNLEFFLTNLGKVHLT

SEQ ID NO: 75 - protein, 319 aa, synthetic construct
NKRPLWFICSGMGTQWRGMGLSLMRLDSFRESILRSDEAVKPLGVKVSDLLLSTDERTFDDIVHAFVSLTAIQIALIDLLTSVGLKPDGIIGHSLGEVACGYADGCLSQREAVLAAYWRGQCIKDAHLPPGSMAAVGLSWEECKQRCPAGVVPACHNSEDVVTISGPQAAVNEFVEQLKQEGVFAKEVRTGGLAFHSYFMEGIAPTLLQALKKVIREPRPRSARWLSTSIPEAQWQSSLARTSSAEYNVNNLVSPVLFQEALWHIPEHAVVLEIAPHALLQAVLKRGVKSSCTIIPLMKRDHKDNLEFFLTNLGKVHLT

SEQ ID NO: 76 - protein, 319 aa, synthetic construct
NKRPLWFICSGMGTQWRGMGLSLMRLDSFRESILRSDEAVKPLGVKVSDLLLSTDERTFDDIVHAFVSLTAIQIALIDLLTSVGLKPDGIIGHSLGEVACGYADGCLSQREAVLAAYWRGQCIKDAHLPPGSMAAVGLSWEECKQRCPAGVVPACHNSEDLVTISGPQAAVNEFVEQLKQEGVFAKEVRTGGLAFHSYFMEGIAPTLLQALKKVIREPRPRSARWLSTSIPEAQWQSSLARTSSAEYNVNNLVSPVLFQEALWHIPEHAVVLEIAPHALLQAVLKRGVKSSCTIIPLMKRDHKDNLEFFLTNLGKVHLT

SEQ ID NO: 77 - protein, 319 aa, synthetic construct
NKRPLWFICSGMGTQWRGMGLSLMRLDSFRESILRSDEAVKPLGVKVSDLLLSTDERTFDDIVHAFVSLTAIQIALIDLLTSVGLKPDGIIGHSLGEVACGYADGCLSQREAVLAAYWRGQCIKDAHLPPGSMAAVGLSWEECKQRCPAGVVPACHNSEDTVTISGPQAAVNEFVEQLKQEGVLAKEVRTGGLAFHSYFMEGIAPTLLQALKKVIREPRPRSARWLSTSIPEAQWQSSLARTSSAEYNVNNLVSPVLFQEALWHIPEHAVVLEIAPHALLQAVLKLGVKSSCTIIPLMKRDHKDNLEFFLTNLGKVHLT

SEQ ID NO: 78 - protein, 319 aa, synthetic construct
NKRPLWFICSGMGTQWRGMGLSLMRLDSFRESILRSDEAVKPLGVKVSDLLLSTDERTFDDIVHAFVSLTAIQIALIDLLTSVGLKPDGIIGHSLGEVACGYADGCLSQREAVLAAYWRGQCIKDAHLPPGSMAAVGLSWEECKQRCPAGVVPACHNSEDLVTISGPQAAVNEFVEQLKQEGVLAKEVRTGGLAFHSYFMEGIAPTLLQALKKVIREPRPRSARWLSTSIPEAQWQSSLARTSSAEYNVNNLVSPVLFQEALWHIPEHAVVLEIAPHALLQAVLKLGVKSSCTIIPLMKRDHKDNLEFFLTNLGKVHLT

SEQ ID NO: 79 - protein, 319 aa, synthetic construct
NKRPLWFICSGMGTQWRGMGLSLMRLDSFRESILRSDEAVKPLGVKVSDLLLSTDERTFDDIVHAFVSLTAIQIALIDLLTSVGLKPDGIIGHSLGEVACGYADGCLSQREAVLAAYWRGQCIKDAHLPPGSMAAVGLSWEECKQRCPAGVVPACHNSEDAVTISGPQAAVNEFVEQLKQEGVAADEVRTGGLAFHSYFMEGIAPTLLQALKKVIREPRPRSARWLSTSIPEAQWQSSLARTSSAEYNVNNLVSPVLFQEALWHIPEHAVVLEIAPHALLQAVLKAGVKSSCTIIPLMKDDHKDNLEFFLTNLGKVHLT

SEQ ID NO: 80 - protein, 319 aa, synthetic construct
NKRPLWFICSGMGTQWRGMGLSLMRLDSFRESILRSDEAVKPLGVKVSDLLLSTDERTFDDIVHAFVSLTAIQIALIDLLTSVGLKPDGIIGHSLGEVACGYADGCLSQREAVLAAYWRGQCIKDAHLPPGSMAAVGLSWEECKQRCPAGVVPACHNSEDAVTISGPQAAVNEFVEQLKQEGVAADEVRTGGLAFHSYFMEGIAPTLLQALKKVIREPRPRSARWLSTSIPEAQWQSSLARTSSAEYNVNNLVSPVLFQEALWHIPEHAVVLEIAPHALLQAVLKAGVKSSCTIIPLMKEDHKDNLEFFLTNLGKVHLT

SEQ ID NO: 81 - protein, 319 aa, synthetic construct
NKRPLWFICSGMGTQWRGMGLSLMRLDSFRESILRSDEAVKPLGVKVSDLLLSTDERTFDDIVHAFVSLTAIQIALIDLLTSVGLKPDGIIGHSLGEVACGYADGCLSQREAVLAAYWRGQCIKDAHLPPGSMAAVGLSWEECKQRCPAGVVPACHNSEDAVTISGPQAAVNEFVEQLKQEGVAAEEVRTGGLAFHSYFMEGIAPTLLQALKKVIREPRPRSARWLSTSIPEAQWQSSLARTSSAEYNVNNLVSPVLFQEALWHIPEHAVVLEIAPHALLQAVLKAGVKSSCTIIPLMKDDHKDNLEFFLTNLGKVHLT

SEQ ID NO: 82 - protein, 319 aa, synthetic construct
NKRPLWFICSGMGTQWRGMGLSLMRLDSFRESILRSDEAVKPLGVKVSDLLLSTDERTFDDIVHAFVSLTAIQIALIDLLTSVGLKPDGIIGHSLGEVACGYADGCLSQREAVLAAYWRGQCIKDAHLPPGSMAAVGLSWEECKQRCPAGVVPACHNSEDAVTISGPQAAVNEFVEQLKQEGVAAEEVRTGGLAFHSYFMEGIAPTLLQALKKVIREPRPRSARWLSTSIPEAQWQSSLARTSSAEYNVNNLVSPVLFQEALWHIPEHAVVLEIAPHALLQAVLKAGVKSSCTIIPLMKEDHKDNLEFFLTNLGKVHLT

SEQ ID NO: 83 - protein, 214 aa, Mus musculus
  source 1..214: note = Sequence of SEQ 1 in Table 1
AAVGLSWEECKQRCPAGVVPACHNSEDTVTISGPQAAVNEFVEQLKQEGVFAKEVRTGGLAFHSYFMEGIAPTLLQALKKVIREPRPRSARWLSTSIPEAQWQSSLARTSSAEYNVNNLVSPVLFQEALWHIPEHAVVLEIAPHALLQAVLKRGVKSSCTIIPLMKRDHKDNLEFFLTNLGKVHLTGINVNPNALFPPVEFPAPRGTPLISPHI

SEQ ID NO: 84 - protein, 214 aa, Rattus norvegicus
  source 1..214: note = Sequence of SEQ 2 in Table 1
AAVGLSWEECKQRCPPGVVPACHNSEDTVTISGPQAAVNEFVEQLKQEGVFAKEVRTGGLAFHSYFMEGIAPTLLQALKKVIREPRPRSARWLSTSIPEAQWQSSLARTSSAEYNVNNLVSPVLFQEALWHVPEHAVVLEIAPHALLQAVLKRGVKPSCTIIPLMKRDHKDNLEFFLTNLGKVHLTGIDINPNALFPPVEFPVPRGTPLISPHI

SEQ ID NO: 85 - protein, 214 aa, Cricetulus griseus
  source 1..214: note = Sequence of SEQ 3 in Table 1
AAVGLSWEECKQRCPSGVVPACHNSEDTVTISGPQAAVSEFVEQLKQEGVFAKEVRTGGLAFHSYFMEGIAPMLLQALKKVIREPRPRSARWLSTSIPEAQWQSSLARTSSAEYNVNNLVSPVLFQEALWHVPEHAVLLEIAPHALLQAVLKRGVKSSCTIIPLMKRDHKDNLEFFLTNLGKVHLTGIDVNPNALFPPVDFPAPRGTPLISPHI

SEQ ID NO: 86 - protein, 214 aa, Homo sapiens
  source 1..214: note = Sequence of SEQ 4 in Table 1
AAVGLSWEECKQRCPPGVVPACHNSKDTVTISGPQAPVFEFVEQLRKEGVFAKEVRTGGMAFHSYFMEAIAPPLLQELKKVIREPKPRSARWLSTSIPEAQWHSSLARTSSAEYNVNNLVSPVLFQEALWHVPEHAVVLEIAPHALLQAVLKRGLKPSCTIIPLMKKDHRDNLEFFLAGIGRLHLSGIDANPNALFPPVEFPAPRGTPLISPLI

SEQ ID NO: 87 - protein, 214 aa, Macaca mulatta
  source 1..214: note = Sequence of SEQ 5 in Table 1
AAVGLSWEECKQRCPPGVVPACHNSKDTVTISGPQASVFEFMEQLRKEGVFAKEVRTGGMAFHSYFMEAIAPPLLQALKKVIREPKPRSARWLSTSIPEAQWHSSLARTSSAEYNVNNLVSPVLFQEALCHVPEHAVVLEVAPHALLQAVLKRGLKPGCTIIPLMKKDHRDNLEFFLTGIGRLHLSGIDANPNALFPPVEFPAPRGTPLISPLI

SEQ ID NO: 88 - protein, 214 aa, Bos taurus
  source 1..214: note = Sequence of SEQ 6 in Table 1
AAVGLTWEECKQRCPPGIVPACHNCIDTVTISGPQASMLEFVQQLKQEGVFAKEVRTGGMAFHSYFMDAIAPMLLQQLKKVIREPQPRSPRWLSTSIPETQWQESLARTFSAEYNVNNLVSPVLFQEALWRVPEDAVVLEIAPHALLQAVLKRGLKSSCTIIPLMKKDHRDNLEFFLSNVGQLYLTGIDVNPNGLFPPVEFPAPRGTPLISPHI

SEQ ID NO: 89 - protein, 214 aa, Capra hircus
  source 1..214: note = Sequence of SEQ 7 in Table 1
AAVGLTWEECKQRCPPGIVPACHNSIDTVTISGPQASMLEFVKQLKQEGVFAKEVQTGGMAFHSYFMDAIAPTLLQQLKKVIREPQLRSPRWLSTSIPESQWHESLARTFSAEYNVNNLVSPVLFQEALWHVPENAVVLEIAPHALLQAILKRGLQPSCTIIPLMKKDHRDNLEFFLSNVGQLYLTGIDVNPNGLFPPVEFPAPRGTPLISPHI

SEQ ID NO: 90 - protein, 214 aa, Equus caballus
  source 1..214: note = Sequence of SEQ 8 in Table 1
AAVGLSWEECKQRCPPGVVPACHNSKDTVTISGPQAAVSEFVEQLKQEGVFAKEVRTGGLAFHSYFMDSISHTLLQALKKVIREPRPRSVRWLSTSIPEAQWQSSLARTFSAEYNVNNLVSPVLFQEALCHVPEHAVVLEIAPHALLQAVLKRGLKPSCTIVPLMKKDHRDNLEFFLSNVGRLHLMGIDVNPNGLFPPVEFPAPRGTPLISPHI

SEQ ID NO: 91 - protein, 214 aa, Felis catus
  source 1..214: note = Sequence of SEQ 9 in Table 1
AAVGLSWEECKQRCPPGVVPACHNSEDTVTISGPQAEVAAFVAELKREGVFAKEVRTGGMAFHSYFMDSIAPTLLQALKKVIREPRPRSARWLSTSIPEAQWQGSLARTFSAEYNVNNLVSPVLFQEALWHVPGDAVVLEIAPHALLQAVLKRGLKSSCTIVPLMKKDQRDNLEFFLSNVGKLHLLGFDVNPNGLLPPVEFPVPRGTPLISPHI

SEQ ID NO: 92 - protein, 214 aa, Sus scrofa
  source 1..214: note = Sequence of SEQ 10 in Table 1
AAVGLSWEECKQRCPPGIVPACHNSKDTVTISGPQAAMSEFLQQLKREDVFVKEVRTGGIAFHSYFMESIAPTLLRQLRKVILDPKPRSKRWLSTSIPEAQWQGSLARTFSAEYSVNNLVSPVLFQEALQHVPAHAVVVEIAPHALLQAVLKRSLESSCTIIPLMKKDHRDNLEFFLSNVGRLHLAGVSVNPNGLFPPVEFPAPRGTPLISPHX

SEQ ID NO: 93 - protein, 214 aa, Cuculus canorus
  source 1..214: note = Sequence of SEQ 11 in Table 1
AAVGLSWEECKQICPPNVVPACHNSEDTVTVSGPLGAVSEFVAKLKKDGVFAKEVRTSGVAFHSHYMASIAPVLLSALKKVIPHPKPRSPRWISTSIPESQWQSDLARYSSAEYHVNNLVNPVLFHEGLSHVPGNALVVEIAPHALLQAILKRSLKPTCIILPLMKKEHKNNLEFFLTQLGKFHMSGVNFNGNNLFPRVEYPVPVETPLISPHI

SEQ ID NO: 94 - protein, 214 aa, Calypte anna
  source 1..214: note = Sequence of SEQ 12 in Table 1
AAVGLTWEECKQQCPPNVVPACHNSEDTVTISGPLATVSEFVAKLKKAGVFAKEVRSAGVAFHSHYMASIAPVLLSALKKVIPHPKPRSARWISTSIPESQWQSDLAKYSSAEYHVNNLVSPVLFHEGLKHIPENAVVVEIAPHALLQAILKRTLKPTCTILPLMKKDHKNNLEFFLTQAGKIHLTGINVLGNNLFPPVEYPVPVGTPLISPYI

SEQ ID NO: 95 - protein, 214 aa, Anas platyrhynchos
  source 1..214: note = Sequence of SEQ 13 in Table 1
AAVGLTWEECKQRCPPNVVPACHNSEDTVTISGPLDSVNEFVAKLKKDGVFAKEVRSAGVAFHSYYMASIAPALLSALRKVIPHPKPRSARWISTSIPESQWQSDLARNSSAEYYVNNLVSPVLFHEGLKHIPENAVVVEIAPHALLQAILRRSLKPSCTILPLMKKDQKNNLEFFLTQAGKIHLTGINVLGNNMFPSVEYPVPVGTPLISPYI

SEQ ID NO: 96 - protein, 214 aa, Gallus gallus
  source 1..214: note = Sequence of SEQ 14 in Table 1
AAVGLTWEECKQRCPPNVVPACHNSEDTVTVSGPLDSVSEFVTKLKKDGVFAKEVRRAGVAFHSYYMASIAPALLSALKKVIPHPKPRSARWISTSIPESQWQSDLARNSSAEYHVNNLVNPVLFHEGLKHIPENAVVVEIAPHALLQAILRRTLKPTCTILPLMKKDHKNNLEFFLTQTGKIHLTGINVLGNNLFPPVEYPVPVGTPLISPYI

SEQ ID NO: 97 - protein, 214 aa, Nestor notabilis
  source 1..214: note = Sequence of SEQ 15 in Table 1
AAVGLTWEECKQRCPPNVVPACHNSEDTVTVSGPLESVTEFVAKLKKDGVFAKEVRSAGVAYHSHYMASIAPVLLNALKKVIPHPKPRSARWISTSIPESQWQSDLARSCSAEYLVNNLVNPVLFHDGLKHVPENAVVVEIAPHALLQAILRRTLKPTCTILPLMKKDQKNNLEFFLTQTGKIHLTGINVLGNNLFPLVEYPVPVGTPLISPYI

SEQ ID NO: 98 - protein, 214 aa, Podiceps cristatus
  source 1..214: note = Sequence of SEQ 16 in Table 1
AAVGLTWEECKQCCPPNVVPACHNSEDTVTISGPLDSVHEFVAKLKKDGVFAKEVRSAGVAFHSYYMASIAPVLLSALKKVIPHPKPRSARWISTSIPESQWQSDLARNSSAEYHVNNLVNPVLFHEGLKHVPENAVVVEIAPHALLQAILRRTLKPTCTILPLMKKDHKNNLEFFLTQTGKIHLTGINVLGNNLLPLVEYPVPVGTPLISPYI

SEQ ID NO: 99 - protein, 214 aa, Balearica regulorum
  source 1..214: note = Sequence of SEQ 17 in Table 1
AAVGLTWEECKQCCPPNVVPACHNSEDTVTVSGPLDSVNEFVAKLKKDGVFAKEVRSAGVAFHSYYMASIAPVLLSALKKVIPHPKPRSARWISTSIPESQWQSDLARNSSAEYHVNNLVNPVLFHEGLKHVPENAVVVEIAPHALLQAILRRTLKPTCTILPLMKKEHKNNLEFFLTQTGKIHLTGINVLGNNLFPLVEYPVPVGTPLISPYI

SEQ ID NO: 100 - protein, 214 aa, Phaethon lepturus
  source 1..214: note = Sequence of SEQ 18 in Table 1
AAVGLTWEECKQCCPPNVVPACHNSEDTVTVSGPLDSVNEFVAKLKKDGVFAKEVRSAGVAFHSYYMASIAPVLLSALKKVIPHPKPRSARWISTSIPESQWQSDLARNSSAEYHVNNLVNPVLFHEGLKHIPENAVVVEIAPHALLQAILRRTLKPTCTILPLMKKEHKNNLEFFLTQTGKIHLTGINVLGNNLFPLVEYPVPVGTPLISPYI

SEQ ID NO: 101 - protein, 214 aa, Phoenicopterus ruber
  source 1..214: note = Sequence of SEQ 19 in Table 1
AAVGLTWEECKQCCPPNVVPACHNSEDTVTVSGPLDSVREFVAKLKKDGVFAKEVRSAGVAFHSYYMASIAPVLLSALKKVIPHPKPRSARWISTSIPESQWQSDLARNSSAEYHVNNLVNPVLFQEGLKHIPENAVVVEIAPHALLQAILRRALKPTCTILPLMKKEHKNNLEFFLTQTGKIHLTGINVLGNNLFPLVEYPVPVGTPLISPYI

SEQ ID NO: 102 - protein, 214 aa, Ooceraea biroi
  source 1..214: note = Sequence of SEQ 20 in Table 1
AAVGLSWEDAQKMCPPNVSPACHNSMDSVTISGPTKDVLKFVEELKSKNIFAKLVRSSGIAFHSKYIASAGPKLRASLDKIIPNPKQRSAKWISSSIPEAAWGSPLAQVSSSAYHVNNLLSPVLFQEAIAHIPDNAITIEIAPHCLLQAILRRSLPSTVTNVSLHMRDHTNNLAFLLSNIGKLYMAGAQPNISKLYPPVSFPVGRGTPMIGPLV

SEQ ID NO: 103 - protein, 214 aa, Anopheles funestus
  source 1..214: note = Sequence of SEQ 21 in Table 1
AAVGLSWEECKQKLPKDVIPACHNSADSVTISGPVNSVGKVIADLNAQGIFAKGVKSSGIAFHSRYIADAAPKLRKSLDKIIPNPKNRTPRWISTSIPEESWPTPLAQQSSSAYHVNNLLSPVLFSEGLKHVPANAICIEIAPHGLLQAILKRALGKDATNLSLMKRDHANNMIFLLSNLGKLYAAGVQPQVQKLYRPITYPVGRGTPMLNSLV

SEQ ID NO: 104 - protein, 214 aa, Anopheles darlingi
  source 1..214: note = Sequence of SEQ 22 in Table 1
AAVGLSWEDCKQKLPKDVIPACHNSSDSVTISGPVASVGKVIADLNAQGIFAKGVKSSGIAFHSRYIADAAPKLRKSLDKIIPNPKPRTQRWISTSIPEESWGTALAQQSSSAYHVNNLLSPVLFAEGLKHVPANAICIEIAPHGLLQAILKRALGKEATNLSLMKRDHDNNLIFLLSNLGKLYAAGAQPQVQKLYPPITYPVGRGTPMLNSLV

SEQ ID NO: 105 - protein, 214 aa, Glossina austeni
  source 1..214: note = Sequence of SEQ 23 in Table 1
AAVGLSWEEAHKRLPADCFPACHNSAENCTISGPEESIDAVCQKLTAEGVFARAVKSSGYAFHSKYIADAGPKLRKSLEKVIPNAKNRSPRWISSSIPEVAWNTAIAQQASAAYHVNNLLSPVLFHQALQHVPKNAICIEVAPTGLLQAILKRSLGNETTNLSLIKRDYENNPEFFLASIGKLYAAGAQPQIMTLSKPISYPVGRGTPMLGCKV

SEQ ID NO: 106 - protein, 214 aa, Drosophila melanogaster
  source 1..214: note = Sequence of SEQ 24 in Table 1
AAVGLSWEDAHSRVPSDCFPVCHNSEDNCTISGPEASIEALVAKLNAEGVFAKAVNSSGYAFHSKYIAEAGPKLRKSLEKIIPNAKNRTARWISTSIPESAWNTPVAKQSSAAYHVNNLLSPVLFHEALQHVPKNAISVEIAPHGLLQAILKRALGPDATNLSLVKRGHENNVEFFLTNVGKLFAAGAQPQVLTLVRPISYPVGRGTPMLNSKV

SEQ ID NO: 107 - protein, 215 aa, Brugia malayi
  source 1..215: note = Sequence of SEQ 25 in Table 1
AAVGLSWEEAGKRCPEGVIPACHNAADSVTISGDAEKIKEFVEELKKEDIFGKLVDSSGIPFHSPAMLKVKDKMLKAMRTSVPNPKPRSSRWISTSIPESNWENELAQMCSADYHTNNAVSPVLFYEALQKIPANAVTIEIAPHCLMHSILRRSLQKTCTNVGLINMKEKDRELESFLQALGKIYQTGITIHIEALYPAIQYPVPIGTPMISPMW

SEQ ID NO: 108 - protein, 219 aa, Caenorhabditis elegans
  source 1..219: note = Sequence of SEQ 26 in Table 1
AAVGLTWEQVKEQAPPGVVAACHNGADSVTISGDAEGVATFCAQLKEKDIFAKVVDTSGIPFHSPAMLAVQDEMIECMRTAVPEPKPRSSKWISTSIPEDDWESDLAATCSAEYHVHNACSPVLFYEAIQKIPANAVTIEMAPHSLMQAILRRSLQKTVTNVGLMNRPKSENDDELESFLGSLGKIYQAGVNIQITELYPGGQYKGVVPKGTPMIGPMW

SEQ ID NO: 109 - protein, 219 aa, Caenorhabditis briggsae
  source 1..219: note = Sequence of SEQ 27 in Table 1
AAVGLTWEEVKAQAPPGVVAACHNGADSVTISGDAEGVASFCAQLKEKEIFAKVVDTSGIPFHSPAMLAVKDEMIESMRTAVPEPKPRSSKWISTSIPEEDWESDLAATCSAEYHVHNACSPVLFYEALQKIPANAVTIEMAPHSLMQAILRRSLQKTVTNVGLMNKPKSENDNELEGFLGSLGKIYQAGVNIQISELYPGGQYKGVVPKGTPMIGPMW

SEQ ID NO: 110 - protein, 219 aa, Caenorhabditis remanei
  source 1..219: note = Sequence of SEQ 28 in Table 1
AAVGLTWEEVKAQAPKGVVAACHNGADSVTISGDAEGVATFCAQLKEKDIFAKVVDTSGIPFHSPAMLAVKDEMIESMRTAVPEPKPRSSKWISTSIPEEDWESDLAATCSAEYHVHNACSPVLFYEALQKIPANAVTIEMAPHSLMQAILRRSLMKTVTNVGLMNKPKSENDDELESFLGSLGKIYQAGVNIQISELYPGGQYKGVVPKGTPMIGPMW

SEQ ID NO: 111 - protein, 319 aa, synthetic construct; identical to SEQ ID NO: 78

SEQ ID NO: 112 - protein, 319 aa, synthetic construct
NKRPLWFICSGMGTQWRGMGLSLMRLDSFRESILRSDEAVKPLGVKVSDLLLSTDERTFDDIVHAFVSLTAIQIALIDLLTSVGLKPDGIIGHSLGEVACGYADGCLSQREAVLAAYWRGQCIKDAHLPPGSMAAVGLSWEECKQRCPAGVVPACHNSEDAVTISGPQAAVNEFVEQLKQEGVAADEVRTGGLAFHSYFMEGIAPTLLQALKKVIREPRPRSARWLSTSIPEAQWQSSLARTSSAEYNVNNLVSPVLFQEALWHIPEHAVVLEIAPHALLQAVLKAGVKSSCTIIPLMKRDHKDNLEFFLTNLGKVHLT

SEQ ID NO: 113 - protein, 319 aa, synthetic construct
NKRPLWFICSGMGTQWRGMGLSLMRLDSFRESILRSDEAVKPLGVKVSDLLLSTDERTFDDIVHAFVSLTAIQIALIDLLTSVGLKPDGIIGHSLGEVACGYADGCLSQREAVLAAYWRGQCIKDAHLPPGSMAAVGLSWEECKQRCPAGVVPACHNSEDAVTISGPQAAVNEFVEQLKQEGVAAEEVRTGGLAFHSYFMEGIAPTLLQALKKVIREPRPRSARWLSTSIPEAQWQSSLARTSSAEYNVNNLVSPVLFQEALWHIPEHAVVLEIAPHALLQAVLKAGVKSSCTIIPLMKRDHKDNLEFFLTNLGKVHLT

SEQ ID NO: 114 - protein, 319 aa, synthetic construct
NKRPLWFICSGMGTQWRGMGLSLMRLDSFRESILRSDEAVKPLGVKVSDLLLSTDERTFDDIVHAFVSLTAIQIALIDLLTSVGLKPDGIIGHSLGEVACGYADGCLSQREAVLAAYWRGQCIKDAHLPPGSMAAVGLSWEECKQRCPAGVVPACHNSEDLVTISGPQAAVNEFVEQLKQEGVAADEVRTGGLAFHSYFMEGIAPTLLQALKKVIREPRPRSARWLSTSIPEAQWQSSLARTSSAEYNVNNLVSPVLFQEALWHIPEHAVVLEIAPHALLQAVLKAGVKSSCTIIPLMKRDHKDNLEFFLTNLGKVHLT

SEQ ID NO: 115 - protein, 319 aa, synthetic construct; identical to SEQ ID NO: 79

SEQ ID NO: 116 - protein, 319 aa, synthetic construct; identical to SEQ ID NO: 81

SEQ ID NO: 117 - protein, 319 aa, synthetic construct
NKRPLWFICSGMGTQWRGMGLSLMRLDSFRESILRSDEAVKPLGVKVSDLLLSTDERTFDDIVHAFVSLTAIQIALIDLLTSVGLKPDGIIGHSLGEVACGYADGCLSQREAVLAAYWRGQCIKDAHLPPGSMAAVGLSWEECKQRCPAGVVPACHNSEDLVTISGPQAAVNEFVEQLKQEGVLADEVRTGGLAFHSYFMEGIAPTLLQALKKVIREPRPRSARWLSTSIPEAQWQSSLARTSSAEYNVNNLVSPVLFQEALWHIPEHAVVLEIAPHALLQAVLKLGVKSSCTIIPLMKRDHKDNLEFFLTNLGKVHLT

SEQ ID NO: 118 - protein, 319 aa, synthetic construct
NKRPLWFICSGMGTQWRGMGLSLMRLDSFRESILRSDEAVKPLGVKVSDLLLSTDERTFDDIVHAFVSLTAIQIALIDLLTSVGLKPDGIIGHSLGEVACGYADGCLSQREAVLAAYWRGQCIKDAHLPPGSMAAVGLSWEECKQRCPAGVVPACHNSEDLVTISGPQAAVNEFVEQLKQEGVLADEVRTGGLAFHSYFMEGIAPTLLQALKKVIREPRPRSARWLSTSIPEAQWQSSLARTSSAEYNVNNLVSPVLFQEALWHIPEHAVVLEIAPHALLQAVLKLGVKSSCTIIPLMKDDHKDNLEFFLTNLGKVHLT

SEQ ID NO: 119 - protein, 319 aa, synthetic construct
NKRPLWFICSGMGTQWRGMGLSLMRLDSFRESILRSDEAVKPLGVKVSDLLLSTDERTFDDIVHAFVSLTAIQIALIDLLTSVGLKPDGIIGHSLGEVACGYADGCLSQREAVLAAYWRGQCIKDAHLPPGSMAAVGLSWEECKQRCPAGVVPACHNSEDDVTISGPQAAVNEFVEQLKQEGVAADEVRTGGLAFHSYFMEGIAPTLLQALKKVIREPRPRSARWLSTSIPEAQWQSSLARTSSAEYNVNNLVSPVLFQEALWHIPEHAVVLEIAPHALLQAVLKAGVKSSCTIIPLMKRDHKDNLEFFLTNLGKVHLT

SEQ ID NO: 120 - protein, 319 aa, synthetic construct
NKRPLWFICSGMGTQWRGMGLSLMRLDSFRESILRSDEAVKPLGVKVSDLLLSTDERTFDDIVHAFVSLTAIQIALIDLLTSVGLKPDGIIGHSLGEVACGYADGCLSQREAVLAAYWRGQCIKDAHLPPGSMAAVGLSWEECKQRCPAGVVPACHNSEDDVTISGPQAAVNEFVEQLKQEGVAAEEVRTGGLAFHSYFMEGIAPTLLQALKKVIREPRPRSARWLSTSIPEAQWQSSLARTSSAEYNVNNLVSPVLFQEALWHIPEHAVVLEIAPHALLQAVLKAGVKSSCTIIPLMKRDHKDNLEFFLTNLGKVHLT

SEQ ID NO: 121 - protein, 319 aa, synthetic construct
NKRPLWFICSGMGTQWRGMGLSLMRLDSFRESILRSDEAVKPLGVKVSDLLLSTDERTFDDIVHAFVSLTAIQIALIDLLTSVGLKPDGIIGHSLGEVACGYADGCLSQREAVLAAYWRGQCIKDAHLPPGSMAAVGLSWEECKQRCPAGVVPACHNSEDAVTISGPQAAVNEFVEQLKQEGVEADEVRTGGLAFHSYFMEGIAPTLLQALKKVIREPRPRSARWLSTSIPEAQWQSSLARTSSAEYNVNNLVSPVLFQEALWHIPEHAVVLEIAPHALLQAVLKAGVKSSCTIIPLMKRDHKDNLEFFLTNLGKVHLT

SEQ ID NO: 122 - protein, 319 aa, synthetic construct
NKRPLWFICSGMGTQWRGMGLSLMRLDSFRESILRSDEAVKPLGVKVSDLLLSTDERTFDDIVHAFVSLTAIQIALIDLLTSVGLKPDGIIGHSLGEVACGYADGCLSQREAVLAAYWRGQCIKDAHLPPGSMAAVGLSWEECKQRCPAGVVPACHNSEDAVTISGPQAAVNEFVEQLKQEGVEAEEVRTGGLAFHSYFMEGIAPTLLQALKKVIREPRPRSARWLSTSIPEAQWQSSLARTSSAEYNVNNLVSPVLFQEALWHIPEHAVVLEIAPHALLQAVLKAGVKSSCTIIPLMKRDHKDNLEFFLTNLGKVHLT

SEQ ID NO: 123 - protein, 319 aa, synthetic construct
NKRPLWFICSGMGTQWRGMGLSLMRLDSFRESILRSDEAVKPLGVKVSDLLLSTDERTFDDIVHAFVSLTAIQIALIDLLTSVGLKPDGIIGHSLGEVACGYADGCLSQREAVLAAYWRGQCIKDAHLPPGSMAAVGLSWEECKQRCPAGVVPACHNSEDLVTISGPQAAVNEFVEQLKQEGVEADEVRTGGLAFHSYFMEGIAPTLLQALKKVIREPRPRSARWLSTSIPEAQWQSSLARTSSAEYNVNNLVSPVLFQEALWHIPEHAVVLEIAPHALLQAVLKAGVKSSCTIIPLMKRDHKDNLEFFLTNLGKVHLT

SEQ ID NO: 124 - protein, 319 aa, synthetic construct
NKRPLWFICSGMGTQWRGMGLSLMRLDSFRESILRSDEAVKPLGVKVSDLLLSTDERTFDDIVHAFVSLTAIQIALIDLLTSVGLKPDGIIGHSLGEVACGYADGCLSQREAVLAAYWRGQCIKDAHLPPGSMAAVGLSWEECKQRCPAGVVPACHNSEDLVTISGPQAAVNEFVEQLKQEGVEAEEVRTGGLAFHSYFMEGIAPTLLQALKKVIREPRPRSARWLSTSIPEAQWQSSLARTSSAEYNVNNLVSPVLFQEALWHIPEHAVVLEIAPHALLQAVLKAGVKSSCTIIPLMKRDHKDNLEFFLTNLGKVHLT

SEQ ID NO: 125 - protein, 319 aa, synthetic construct
NKRPLWFICSGMGTQWRGMGLSLMRLDSFRESILRSDEAVKPLGVKVSDLLLSTDERTFDDIVHAFVSLTAIQIALIDLLTSVGLKPDGIIGHSLGEVACGYADGCLSQREAVLAAYWRGQCIKDAHLPPGSMAAVGLSWEECKQRCPAGVVPACHNSEDLVTISGPQAAVNEFVEQLKQEGVEADEVRTGGLAFHSYFMEGIAPTLLQALKKVIREPRPRSARWLSTSIPEAQWQSSLARTSSAEYNVNNLVSPVLFQEALWHIPEHAVVLEIAPHALLQAVLKAGVKSSCTIIPLMKDDHKDNLEFFLTNLGKVHLT

SEQ ID NO: 126 - protein, 319 aa, synthetic construct
NKRPLWFICSGMGTQWRGMGLSLMRLDSFRESILRSDEAVKPLGVKVSDLLLSTDERTFDDIVHAFVSLTAIQIALIDLLTSVGLKPDGIIGHSLGEVACGYADGCLSQREAVLAAYWRGQCIKDAHLPPGSMAAVGLSWEECKQRCPAGVVPACHNSEDLVTISGPQAAVNEFVEQLKQEGVEAEEVRTGGLAFHSYFMEGIAPTLLQALKKVIREPRPRSARWLSTSIPEAQWQSSLARTSSAEYNVNNLVSPVLFQEALWHIPEHAVVLEIAPHALLQAVLKAGVKSSCTIIPLMKDDHKDNLEFFLTNLGKVHLT

SEQ ID NO: 127 - protein, 319 aa, synthetic construct
NKRPLWFICSGMGTQWRGMGLSLMRLDSFRESILRSDEAVKPLGVKVSDLLLSTDERTFDDIVHAFVSLTAIQIALIDLLTSVGLKPDGIIGHSLGEVACGYADGCLSQREAVLAAYWRGQCIKDAHLPPGSMAAVGLSWEECKQRCPAGVVPACHNSEDDVTISGPQAAVNEFVEQLKQEGVEADEVRTGGLAFHSYFMEGIAPTLLQALKKVIREPRPRSARWLSTSIPEAQWQSSLARTSSAEYNVNNLVSPVLFQEALWHIPEHAVVLEIAPHALLQAVLKAGVKSSCTIIPLMKRDHKDNLEFFLTNLGKVHLT

SEQ ID NO: 128 - protein, 319 aa, synthetic construct
NKRPLWFICSGMGTQWRGMGLSLMRLDSFRESILRSDEAVKPLGVKVSDLLLSTDERTFDDIVHAFVSLTAIQIALIDLLTSVGLKPDGIIGHSLGEVACGYADGCLSQREAVLAAYWRGQCIKDAHLPPGSMAAVGLSWEECKQRCPAGVVPACHNSEDDVTISGPQAAVNEFVEQLKQEGVEAEEVRTGGLAFHSYFMEGIAPTLLQALKKVIREPRPRSARWLSTSIPEAQWQSSLARTSSAEYNVNNLVSPVLFQEALWHIPEHAVVLEIAPHALLQAVLKAGVKSSCTIIPLMKRDHKDNLEFFLTNLGKVHLT

SEQ ID NO: 129 - protein, 319 aa, synthetic construct
NKRPLWFICSGMGTQWRGMGLSLMRLDSFRESILRSDEAVKPLGVKVSDLLLSTDERTFDDIVHAFVSLTAIQIALIDLLTSVGLKPDGIIGHSLGEVACGYADGCLSQREAVLAAYWRGQCIKDAHLPPGSMAAVGLSWEECKQRCPAGVVPACHNSEDDVTISGPQAAVNEFVEQLKQEGVEADEVRTGGLAFHSYFMEGIAPTLLQALKKVIREPRPRSARWLSTSIPEAQWQSSLARTSSAEYNVNNLVSPVLFQEALWHIPEHAVVLEIAPHALLQAVLKAGVKSSCTIIPLMKDDHKDNLEFFLTNLGKVHLT

SEQ ID NO: 130 - protein, 319 aa, synthetic construct
NKRPLWFICSGMGTQWRGMGLSLMRLDSFRESILRSDEAVKPLGVKVSDLLLSTDERTFDDIVHAFVSLTAIQIALIDLLTSVGLKPDGIIGHSLGEVACGYADGCLSQREAVLAAYWRGQCIKDAHLPPGSMAAVGLSWEECKQRCPAGVVPACHNSEDDVTISGPQAAVNEFVEQLKQEGVEAEEVRTGGLAFHSYFMEGIAPTLLQALKKVIREPRPRSARWLSTSIPEAQWQSSLARTSSAEYNVNNLVSPVLFQEALWHIPEHAVVLEIAPHALLQAVLKAGVKSSCTIIPLMKDDHKDNLEFFLTNLGKVHLT

SEQ ID NO: 131 - protein, 319 aa, synthetic construct
NKRPLWFICSGMGTQWRGMGLSLMRLDSFRESILRSDEAVKPLGVKVSDLLLSTDERTFDDIVHAFVSLTAIQIALIDLLTSVGLKPDGIIGHSLGEVACGYADGCLSQREAVLAAYWRGQCIKDAHLPPGSMAAVGLSWEECKQRCPAGVVPACHNSERAVTISGPQAAVNEFVEQLKQEGVEADEVRTGGLAFHSYFMEGIAPTLLQALKKVIREPRPRSARWLSTSIPEAQWQSSLARTSSAEYNVNNLVSPVLFQEALWHIPEHAVVLEIAPHALLQAVLKDGVKSSCTIIPLMKRDHKDNLEFFLTNLGKVHLT

SEQ ID NO: 132 - protein, 319 aa, synthetic construct
NKRPLWFICSGMGTQWRGMGLSLMRLDSFRESILRSDEAVKPLGVKVSDLLLSTDERTFDDIVHAFVSLTAIQIALIDLLTSVGLKPDGIIGHSLGEVACGYADGCLSQREAVLAAYWRGQCIKDAHLPPGSMAAVGLSWEECKQRCPAGVVPACHNSEDTVTISGPQAAVNEFVEQLKQEGVFAKEVRTGGLAFHSYFMEGIAPTLLQALKKVIREPRPRSARWLSTSIPEAQWQSSLARTSSAEYNVNNLVSPVLFQEALWHIPEHAVVLEIAPHALLQAVLKAGVKSSCTIIPLMKRDHKDNLEFFLTNLGKVHLT

SEQ ID NO: 133 - protein, 319 aa, synthetic construct
NKRPLWFICSGMGTQWRGMGLSLMRLDSFRESILRSDEAVKPLGVKVSDLLLSTDERTFDDIVHAFVSLTAIQIALIDLLTSVGLKPDGIIGHSLGEVACGYADGCLSQREAVLAAYWRGQCIKDAHLPPGSMAAVGLSWEECKQRCPAGVVPACHNSEDTVTISGPQAAVNEFVEQLKQEGVFAKEVRTGGLAFHSYFMEGIAPTLLQALKKVIREPRPRSARWLSTSIPEAQWQSSLARTSSAEYNVNNLVSPVLFQEALWHIPEHAVVLEIAPHALLQAVLKLGVKSSCTIIPLMKRDHKDNLEFFLTNLGKVHLT

SEQ ID NO: 134 - protein, 323 aa, Saccharopolyspora erythraea
AVFVFPGQGWQWAGMAVDLLDTSPVFAAALRECADALEPHLDFEVIPFLRAEAARREQDAALSTERVDVVQPVMFAVMVSLASMWRAHGVEPAAVIGHSQGEIAAACVAGALSLDDAARVVALRSRVIATMPGNKGMASIAAPAGEVRARIGDRVEIAAVNGPRSVVVAGDSDELDRLVASCTTECIRAKRLAVDYASHSSHVETIRDALHAELGEDFHPLPGFVPFFSTVTGRWTQPDELDAGYWYRNLRRTVRFADAVRALAEQGYRTFLEVSAHPILTAAIEEIGDGSGADLSAIHSLRRGDGSLADFGEALSRAFAAGV

SEQ ID NO: 135 - protein, 320 aa, Saccharopolyspora erythraea
SVFVFPGQGAQWEGMARELLPVPVFAESIAECDAVLSEVAGFSVSEVLEPRPDAPSLERVDVVQPVLFAVMVSLARLWRACGAVPSAVIGHSQGEIAAAVVAGALSLEDGMRVVARRSRAVRAVAGRGSMLSVRGGRSDVEKLLADDSWTGRLEVAAVNGPDAVVVAGDAQAAREFLEYCEGVGIRARAIPVDYASHTAHVEPVRDELVQALAGITPRRAEVPFFSTLTGDFLDGTELDAGYWYRNLRHPVEFHSAVQALTDQGYATFIEVSPHPVLASSVQETLDDAESDAAVLGTLERDAGDADRFLTALADAHTRGV

SEQ ID NO: 136 - protein, 321 aa, Saccharopolyspora erythraea
VVFLFPGQGSQWAGMGAELLSSSPVFAGKIRACDESMAPMQDWKVSDVLRQAPGAPGLDRVDVVQPVLFAVMVSLAELWRSYGVEPAAVVGHSQGEIAAAHVAGALTLEDAAKLVVGRSRLMRSLSGEGGMAAVALGEAAVRERLRPWQDRLSVAAVNGPRSVVVSGEPGALRAFSEDCAAEGIRVRDIDVDYASHSPQIERVREELLETTGDIAPRPARVTFHSTVESRSMDGTELDARYWYRNLRETVRFADAVTRLAESGYDAFIEVSPHPVVVQAVEEAVEEADGAEDAVVVGSLHRDGGDLSAFLRSMATAHVSGV

SEQ ID NO: 137 - protein, 319 aa, Saccharopolyspora erythraea
PVLVFPGQGAQWVGMARDLLESSEVFAESMSRCAEALSPHTDWKLLDVVRGDGGPDPHERVDVLQPVLFSIMVSLAELWRAHGVTPAAVVGHSQGEIAAAHVAGALSLEAAAKVVALRSQVLRELDDQGGMVSVGASRDELETVLARWDGRVAVAAVNGPGTSVVAGPTAELDEFFAEAEAREMKPRRIAVRYASHSPEVARIEDRLAAELGTITAVRGSVPLHSTVTGEVIDTSAMDASYWYRNLRRPVLFEQAVRGLVEQGFDTFVEVSPHPVLLMAVEETAEHAGAEVTCVPTLRREQSGPHEFLRNLLRAHVHGV

SEQ ID NO: 138 - protein, 319 aa, Saccharopolyspora erythraea
VAMVFPGQGAQWQGMARDLLRESQVFADSIRDCERALAPHVDWSLTDLLSGARPLDRVDVVQPALFAVMVSLAALWRSHGVEPAAVVGHSQGEIAAAHVAGALTLEDAAKLVAVRSRVLRRLGGQGGMASFGLGTEQAAERIGRFAGALSIASVNGPRSVVVAGESGPLDELIAECEAEGITARRIPVDYASHSPQVESLREELLTELAGISPVSADVALYSTTTGQPIDTATMDTAYWYANLREQVRFQDATRQLAEAGFDAFVEVSPHPVLTVGIEATLDSALPADAGACVVGTLRRDRGGLADFHTALGEAYAQGV

SEQ ID NO: 139 - protein, 313 aa, Saccharopolyspora erythraea
VVFVFPGQGAQWEGMARGLLSVPVFAESIAECDAVLSEVAGFSASEVLEQRPDAPSLERVDVVQPVLFSVMVSLARLWGACGVSPSAVIGHSQGEIAAAVVAGVLSLEDGVRVVALRAKALRALAGKGGMVSLAAPGERARALIAPWEDRISVAAVNSPSSVVVSGDPEALAELVARCEDEGVRAKTLPVDYASHSRHVEEIRETILADLDGISARRAAIPLYSTLHGERRDGADMGPRYWYDNLRSQVRFDEAVSAAVADGHATFVEMSPHPVLTAAVQEIAADAVAIGSLHRDTAEEHLIAELARAHVHGV

SEQ ID NO: 140 - protein, 318 aa, Streptomyces hygroscopicus
VAFLFDGQGTQRLGMGKELYDSYPAFARAWDTVSAGFDKHLDHSLTDVCFGEGGSTTAGLVDDTLYAQAGIFAMEAALFGLLEDWGVRPDFVAGHSIGEATAAYASGMLSLENVTTLIVARGRALRTTPPGAMVALRAGEEEVREFLSRTGAALDLAAVNSPEAVVVSGEPEPVADFEAAWTASGREARKLKVRHAFHSRHVEAVLDEFRTALESLKFRAPALPVVSTVTGRLIDQDEMGTPEYWLRQVRRPVRFQDAVRELAEQGVGTFVEVGPSGALASAGVECLGGDASFHAVLRPRSPEDVCLMTAIAELHAGG

SEQ ID NO: 141 - protein, 275 aa, Streptomyces hygroscopicus
AVFVFPGQGSQRAGMGEELAAAFPVFARIHQQVWDLLDVPDLEVNETGYAQPALFAMQVALFGLLESWGVRPDAVIGHSVGELAAAYVSGVWSLEDACTLVSARARLMQALPAGGVMVAVPVSEDEARAVLGEGVEIAAVNGPSSVVLSGDEAAVLQAAEGLGKWTRLATSHAFHSARMEPMLEEFRAVAEGLTYRTPQVSMAVGDQVTTAEYWVRQVRDTVRFGEQVASYEDAVFVELGADRSLARLVDGVAMLHGDHEIQAAIGALAHLYVNG

SEQ ID NO: 142 - protein, 303 aa, Streptomyces hygroscopicus
VVFVFPGQGWQWLGMGSALRDSSIVFAERMAECAPALREFVDWDLFTVLDDPAVVDRVDVVQPASWRMMVSLAAVWQAAGVRPDAVIGHSQGEIAAACVAGAVSMRDAARIVTLRSEAIARGLAGRGAMASVALPAQDVELVDGAWIAAHNGPASTVIAGTPEAVDHVLTAHEARGVRVRRITVDYASHTPHVELIRDELLDITSDSSSQAPVVPWLSTVDGSWVDSPLDVEYWYRNLREPVGFHPAVGQLQAEGDTVFVEVSASPVLLQAMDDDVVTVATLRRDDGDATRMLTALAQAYVHG

SEQ ID NO: 143 - protein, 316 aa, Actinomadura vulgaris
AVLVFPGQGAQWAGMGVELAQASPVFAARLEECFGEIRRWVDWDPAQVLADADALESIERLQPVAFAVGVALAALWESVGVRPAAVVGHSQGEVAAACVAGVLSLADAVRVVVLRSRLFAAELWGRGAIAAVGLPAEVVRERIASLGGGLEVSADNGPASCAVAGPGQVLEEFVERLRGEGVRARVIATTVASHSQMVEPLREQLLEMLGPITPEAGRVPVYSTVTGGVLAGSELGAEYWFANARRPVDFQGAVRALLADGRTAFIEVSPHPVLTMAVQDILDATGTSGVAVGSLRRGEGGPDRFMRSAGEAFTAG

SEQ ID NO: 144 - protein, 315 aa, Actinomadura vulgaris
TAFLYSGQGAQHPGMGRQLYETFPTFATALNNTLDALDPHLDHPLRDIMWAPPHTPQAHLLNQTTYTQPALFALQTALTHLLTSFGIHPHYLAGHSLGEITAAHTAGILTLTDAATLITQRAHLMQTLPETGAMTAINATPEEITPHLTPHTAIAAINSPTSTVISGNAQDIQHITHHFTTLGRKTRPLTVSHAFHSPLLDPILTPLNTLAHTLTHHPAHTPLITNTTATPTHTLTPTHWAHHARQPVQFANTITHLHHAGVTTYLEIGPDTTLTAIAPHNLPPTTHTTFTPTLRKNTPEPDTLLTAIATTHTHN

SEQ ID NO: 145 - protein, 319 aa, Sorangium cellulosum
LAFLFTGQGAQTPGMGRGLCAAWPAFREAFDRCVALFDRELDRPLCEVMWAEPGSAESLLLDQTAFTQPALFTVEYALTALWRSWGVEPELVAGHSAGELVAACVAGVFSLEDGVRLVAARGRLMQGLSAGGAMVSLGAPEAEVAAAVAPHAAWVSIAAVNGPEQVVIAGVEQAVQAIAAGFAARGVRTKRLHVSHASHSPLMEPMLEEFGRVAASVTYRRPSVSLVSNLSGKVVTDELSAPGYWVRHVREAVRFADGVKALHEAGAGTFLEVGPKPTLLGLLPACLPEAEPTLLASLRAGREEAAGVLEALGRLWAAG

SEQ ID NO: 146 - protein, 316 aa, Streptomyces virginiae
PVMVFPGQGGQWVGMGARLLDESPVFAARIAECEQALSAYVDWSLTDVLRGDGSELARIDVVQPVLWAVMVALAAVWADQGIEPAAVVGHSQGEIAAACVVGAISLDEAARIVAVRSVLLRQLSGRGGMASLGMGQEQAADLIDGHPGVVVAAVNGPSSTVISGPPEGIAAVVADAQERGLRARAVASDVAGHGPQLDAILDQLTEGLAGIRPAATDVAFYSTVTAGHLTDTTELDTAYWVRNVRRTVRFADTIDALLADGYRLFIEVSPHPVLNLALEGLIERAAVPATVVPTLRRDHGDTTQLARAAAHAFAAG

SEQ ID NO: 147 - protein, 319 aa, Streptomyces caelestis
VVFVFPGQGSQWAGMAEGLLERSGAFRSAADSCDAALRPYLGWSVLSVLRGEPDAPSLDRVDVVQPVLFTMMVSLAAVWRALGVEPAAVVGHSQGEIAAAHVAGALSLDDSARIVALRSRAWLGLAGKGGMVAVPMPAEELRPRLVTWGDRLAVAAVNSPGSCAVAGDPEALAELVALLTGEGVHARPIPGVDTAGHSPQVDALRAHLLEVLAPVAPRPADIPFYSTVTGGLLDGTELDATYWYRNMREPVEFERATRALIADGHDVFLETSPHPMLAVALEQTVTDAGTDAAVLGTLRRRHGGPRALALAVCRAFAHG

SEQ ID NO: 148 - protein, 319 aa, Streptomyces sp. W112
VAFVFPGQGSQWLGMGAELLASSSVFAAAMAECDAALGDYVGWSVIDVIRQDPAAPDPNLIEVVQPSLFAVHVSLAALWQHVGVRPAAVVGHSQGEIAAAVVSGALSLSDGARVIVARSALLAEELLGKGAMAWIGTSADDVEDRLAQWADRLSVAGRNSPRAVTVVGETEALHELVAGCEADGIRTRIVGSSVASHCAQIEPLRDRLLAMFDEVTPRAARVPFYSSVTGTVIDTTGMDAEYWYRNAREPVDLEAAVRALLADGYAFFVELSAHPVLTVPVQETAEAVGADVAAVGSLRRDDGGPRRFLTSMAEGFVRG

SEQ ID NO: 149 - protein, 319 aa, Streptomyces flaveolus
AVFVFPGHGAQWPGMARRLFDDFPVFRESVLQCADAFAEFVDWSLLDVLRDEEGAPPLHRVDVVQPALFTMMVSLAALWRSYGVEPSAVVGHSQGEIAAAYVAGALDLRDAARIVATRGKAWLTLAGTGGMASVALPRAEAAERLRPFGHRLDIAAVNDPRSVTVAGDLDALEEFLTGLETEGVRVRRVRQIVGAGHTAHVDALRDQLIETLAPTAPRSAPIAFCSTVTGGLLDTAGLDHHYWYRNARRTVLFEQAVRTLAEQGYGPFLEISAHPMFTVAVQETLEDAGVGAAVLATLRRDEGGPDRFLRAAAEAHTAG

SEQ ID NO: 150 - protein, 320 aa, Sorangium cellulosum
VAFLFSGFGSESVGMGRELYETEPAFREAMDRCADLLAPHLPRRLTDVLYPARDAAGGAAASLGDLSYAQPALFALEYCLAELWKSWGITPSAVVGHSLGECVAACVAGVFSLEDALTLVAARGRLMESLAGEGETFLVSADEATVRRVIASDPVSIGSINGPANIVISGAPAGVKSVVERLSQEGIEVKKLDVRRAAHSPLMDPMLEAFGKVARSIRYARPTIDLVANLTGEVAGEEIATPEYWCRQIRETVRMSACLRTLHDALGFEVFLELGPSPALVWNGMQCVPKRSGAWIASLRPGRPDRAQILAALASLYANG

SEQ ID NO: 151 - protein, 327 aa, Streptomyces avermitilis
VVFVFPGQGPQWPGMGRELLDASDVFRESVRACEAAFAPYVDWSVEQVLRDSPDAPGLDRVDVVQPTLFAVMISLAALWRSQGVEPCAVLGHSLGEIAAAHVSGGLSLADAARVVTLWSQAQTTLAGTGALVSVAATPDELLPRIAPWTEDNPARLAVAAVNGPRSTVVSGAREAVADLVADLTAAQVRTRMIPVDVPAHSPLMYAIEERVVSGLLPITPRPSRIPFHSSVTGGRLDTRELDAAYWYRNMSSTVRFEPAARLLLQQGPKTFVEMSPHPVLTMGLQELAPDLGDTTGTADTVIMGTLRRGQGTLDHFLTSLAQLRGHG

SEQ ID NO: 152 - protein, 316 aa, Saccharopolyspora erythraea
VVFVFPGQGAQWAGMAGELLGESRVFAAAMDACARAFEPVTDWTLAQVLDSPEQSRRVEVVQPALFAVQTSLAALWRSFGVTPDAVVGHSIGELAAAHVCGAAGAADAARAAALWSREMIPLVGNGDMAAVALSADEIEPRIARWDDDVVLAGVNGPRSVLLTGSPEPVARRVQELSAEGVRAQVINVSMAAHSAQVDDIAEGMRSALAWFAPGGSEVPFYASLTGGAVDTRELVADYWRRSFRLPVRFDEAIRSALEVGPGTFVEASPHPVLAAALQQTLDAEGSSAAVVPTLQRGQGGMRRFLLAAAQAFTGGV

SEQ ID NO: 153 - protein, 317 aa, Streptomyces collinus
LVFVFAGQGAQWDGMGLELLDTEPVFGAALRRCDERVRELAGFSVIQQLRAGPAMSRLGEIDVLQPTMVSLQIALVALWRSWRVEPDAVTGHSMGEISAGYAAGALTLDDALLIACRRSALLRRIAGRGALATTELSPEAAHALAASSGGRICVAGENSPRSTVLAGDTATLTALVEDLDRRGVYCRMVRGTVASHSHYVDELRDDLAGALRPLSPVPSRVPFYSTVTAAPVPGTDLGPAYWMRNLREPVRLAAATGRLAEDGHEIFVEVSTHPVLLSSLRQTLESAGRPGEVLPSGRRRTERRAMLSSLGTLFTYG

SEQ ID NO: 154 - protein, 313 aa, Saccharopolyspora erythraea
VVFVFPGQGAQWEGMARGLLSVPVFAESIAECDAVLSEVAGFSASEVLEQRPDAPSLERVDVVQPVLFSVMVSLARLWGACGVSPSAVIGHSQGEIAAAVVAGVLSLEDGVRVVALRAKALRALAGKGGMVSLAAPGERARALIAPWEDRISVAAVNSPSAVVVSGDPEALAELVARCEDEGVAAKTLPVDYASHSRHVEEIRETILADLDGISARRAAIPLYSTLHGERRDGADMGPRYWYDNLRSQVRFDEAVSAAVADGHATFVEMSPHPVLTAAVQAIAADAVAIGSLHRDTAEEHLIAELARAHVHGV

SEQ ID NO: 155 - protein, 313 aa, Saccharopolyspora erythraea
VVFVFPGQGAQWEGMARGLLSVPVFAESIAECDAVLSEVAGFSASEVLEQRPDAPSLERVDVVQPVLFSVMVSLARLWGACGVSPSAVIGHSQGEIAAAVVAGVLSLEDGVRVVALRAKALRALAGKGGMVSLAAPGERARALIAPWEDRISVAAVNSPSSVVVSGDPEALAELVARCEDEGVRAATLPVDYASHSRHVEEIRETILADLDGISARRAAIPLYSTLHGERRDGADMGPRYWYDNLRSQVRFDEAVSAAVADGHATFVEMSPHPVLTAAVQEIAADAVAIGSLHRDTAEEHLIAELARAHVHGV

SEQ ID NO: 156 - protein, 313 aa, Saccharopolyspora erythraea
VVFVFPGQGAQWEGMARGLLSVPVFAESIAECDAVLSEVAGFSASEVLEQRPDAPSLERVDVVQPVLFSVMVSLARLWGACGVSPSAVIGHSQGEIAAAVVAGVLSLEDGVRVVALRAKALRALAGKGGMVSLAAPGERARALIAPWEDRISVAAVNSPSSVVVSGDPEALAELVARCEDEGVRAETLPVDYASHSRHVEEIRETILADLDGISARRAAIPLYSTLHGERRDGADMGPRYWYDNLRSQVRFDEAVSAAVADGHATFVEMSPHPVLTAAVQEIAADAVAIGSLHRDTAEEHLIAELARAHVHGV

SEQ ID NO: 157 - protein, 313 aa, Saccharopolyspora erythraea
VVFVFPGQGAQWEGMARGLLSVPVFAESIAECDAVLSEVAGFSASEVLEQRPDAPSLERVDVVQPVLFSVMVSLARLWGACGVSPSAVIGHSQGEIAAAVVAGVLSLEDGVRVVALRAKALRALAGKGGMVSLAAPGERARALIAPWEDRISVAAVNSPSSVVVSGDPEALAELVARCEDEGVRAKTLPVDYASHSRHVEEIRETILADLDGISARRAAIPLYSTLHGERRDGADMGPRYWYDNLRSQVRFDEAVSAAVADGHATFVEMSPHPVLTAAVQEIAADAVAIGSLHADTAEEHLIAELARAHVHGV

SEQ ID NO: 158 - protein, 313 aa, Saccharopolyspora erythraea
VVFVFPGQGAQWEGMARGLLSVPVFAESIAECDAVLSEVAGFSASEVLEQRPDAPSLERVDVVQPVLFSVMVSLARLWGACGVSPSAVIGHSQGEIAAAVVAGVLSLEDGVRVVALRAKALRALAGKGGMVSLAAPGERARALIAPWEDRISVAAVNSPSSVVVSGDPEALAELVARCEDEGVRAKTLPVDYASHSRHVEEIRETILADLDGISARRAAIPLYSTLHGERRDGADMGPRYWYDNLRSQVRFDEAVSAAVADGHATFVEMSPHPVLTAAVQEIAADAVAIGSLHEDTAEEHLIAELARAHVHGV

SEQ ID NO: 159 - protein, 313 aa, Saccharopolyspora erythraea
VVFVFPGQGAQWEGMARGLLSVPVFAESIAECDAVLSEVAGFSASEVLEQRPDAPSLERVDVVQPVLFSVMVSLARLWGACGVSPSAVIGHSQGEIAAAVVAGVLSLEDGVRVVALRAKALRALAGKGGMVSLAAPGERARALIAPWEDRISVAAVNSPSAVVVSGDPEALAELVARCEDEGVAAATLPVDYASHSRHVEEIRETILADLDGISARRAAIPLYSTLHGERRDGADMGPRYWYDNLRSQVRFDEAVSAAVADGHATFVEMSPHPVLTAAVQAIAADAVAIGSLHRDTAEEHLIAELARAHVHGV

SEQ ID NO: 160 - protein, 313 aa, Saccharopolyspora erythraea
VVFVFPGQGAQWEGMARGLLSVPVFAESIAECDAVLSEVAGFSASEVLEQRPDAPSLERVDVVQPVLFSVMVSLARLWGACGVSPSAVIGHSQGEIAAAVVAGVLSLEDGVRVVALRAKALRALAGKGGMVSLAAPGERARALIAPWEDRISVAAVNSPSAVVVSGDPEALAELVARCEDEGVAAETLPVDYASHSRHVEEIRETILADLDGISARRAAIPLYSTLHGERRDGADMGPRYWYDNLRSQVRFDEAVSAAVADGHATFVEMSPHPVLTAAVQAIAADAVAIGSLHRDTAEEHLIAELARAHVHGV

SEQ ID NO: 161 - protein, 313 aa, Saccharopolyspora erythraea
VVFVFPGQGAQWEGMARGLLSVPVFAESIAECDAVLSEVAGFSASEVLEQRPDAPSLERVDVVQPVLFSVMVSLARLWGACGVSPSAVIGHSQGEIAAAVVAGVLSLEDGVRVVALRAKALRALAGKGGMVSLAAPGERARALIAPWEDRISVAAVNSPSAVVVSGDPEALAELVARCEDEGVAAATLPVDYASHSRHVEEIRETILADLDGISARRAAIPLYSTLHGERRDGADMGPRYWYDNLRSQVRFDEAVSAAVADGHATFVEMSPHPVLTAAVQAIAADAVAIGSLHADTAEEHLIAELARAHVHGV

SEQ ID NO: 162 - protein, 313 aa, Saccharopolyspora erythraea
VVFVFPGQGAQWEGMARGLLSVPVFAESIAECDAVLSEVAGFSASEVLEQRPDAPSLERVDVVQPVLFSVMVSLARLWGACGVSPSAVIGHSQGEIAAAVVAGVLSLEDGVRVVALRAKALRALAGKGGMVSLAAPGERARALIAPWEDRISVAAVNSPSAVVVSGDPEALAELVARCEDEGVAAATLPVDYASHSRHVEEIRETILADLDGISARRAAIPLYSTLHGERRDGADMGPRYWYDNLRSQVRFDEAVSAAVADGHATFVEMSPHPVLTAAVQAIAADAVAIGSLHEDTAEEHLIAELARAHVHGV

SEQ ID NO: 163 - protein, 313 aa, Saccharopolyspora erythraea
VVFVFPGQGAQWEGMARGLLSVPVFAESIAECDAVLSEVAGFSASEVLEQRPDAPSLERVDVVQPVLFSVMVSLARLWGACGVSPSAVIGHSQGEIAAAVVAGVLSLEDGVRVVALRAKALRALAGKGGMVSLAAPGERARALIAPWEDRISVAAVNSPSAVVVSGDPEALAELVARCEDEGVAAETLPVDYASHSRHVEEIRETILADLDGISARRAAIPLYSTLHGERRDGADMGPRYWYDNLRSQVRFDEAVSAAVADGHATFVEMSPHPVLTAAVQAIAADAVAIGSLHADTAEEHLIAELARAHVHGV

SEQ ID NO: 164 - protein, 313 aa, Saccharopolyspora erythraea
VVFVFPGQGAQWEGMARGLLSVPVFAESIAECDAVLSEVAGFSASEVLEQRPDAPSLERVDVVQPVLFSVMVSLARLWGACGVSPSAVIGHSQGEIAAAVVAGVLSLEDGVRVVALRAKALRALAGKGGMVSLAAPGERARALIAPWEDRISVAAVNSPSAVVVSGDPEALAELVARCEDEGVAAETLPVDYASHSRHVEEIRETILADLDGISARRAAIPLYSTLHGERRDGADMGPRYWYDNLRSQVRFDEAVSAAVADGHATFVEMSPHPVLTAAVQAIAADAVAIGSLHEDTAEEHLIAELARAHVHGV

SEQ ID NO: 165 - protein, 313 aa, Saccharopolyspora erythraea
VVFVFPGQGAQWEGMARGLLSVPVFAESIAECDAVLSEVAGFSASEVLEQRPDAPSLERVDVVQPVLFSVMVSLARLWGACGVSPSAVIGHSQGEIAAAVVAGVLSLEDGVRVVALRAKALRALAGKGGMVSLAAPGERARALIAPWEDRISVAAVNSPSSVVVSGDPEALAELVARCEDEGVAAATLPVDYASHSRHVEEIRETILADLDGISARRAAIPLYSTLHGERRDGADMGPRYWYDNLRSQVRFDEAVSAAVADGHATFVEMSPHPVLTAAVQAIAADAVAIGSLHRDTAEEHLIAELARAHVHGV